European Patent Application EP 4 623 922 A2, published October 1, 2025. Title: ALTERING MICROBIAL POPULATIONS & MODIFYING MICROBIOTA. Applicant: SNIPR Technologies Ltd. The sequence listing filed with the application follows.

SEQUENCE LISTING (738 sequences)

SEQ ID NO: 1-19 - skipped (19 entries)

SEQ ID NO: 20 - DNA, 10 bp, Streptococcus
  misc_feature 1..10: note = Transcribed Leader Seq 18
  source 1..10: mol_type = other DNA
acgatttgag

SEQ ID NO: 21 - skipped

SEQ ID NO: 22 - DNA, 10 bp, Streptococcus
  misc_feature 1..10: note = Transcribed Leader Seq 20
  source 1..10: mol_type = other DNA
ttcatttgag

SEQ ID NO: 23 - DNA, 10 bp, Streptococcus
  misc_feature 1..10: note = Transcribed Leader Seq 21
  source 1..10: mol_type = other DNA
atcatttgag

SEQ ID NO: 24 - DNA, 11 bp, Streptococcus
  misc_feature 1..11: note = Transcribed Leader Seq 22
  source 1..11: mol_type = other DNA
tttcatttgag

SEQ ID NO: 25 - DNA, 11 bp, Streptococcus
  misc_feature 1..11: note = Transcribed Leader Seq 23
  source 1..11: mol_type = other DNA
aatcatttgag

SEQ ID NO: 26 - DNA, 12 bp, Streptococcus
  misc_feature 1..12: note = Transcribed Leader Seq 24
  source 1..12: mol_type = other DNA
aattcatttgag

SEQ ID NO: 27 - DNA, 12 bp, Streptococcus
  misc_feature 1..12: note = Transcribed Leader Seq 25
  source 1..12: mol_type = other DNA
aaatcatttgag

SEQ ID NO: 28 - DNA, 13 bp, Streptococcus
  misc_feature 1..13: note = Transcribed Leader Seq 26
  source 1..13: mol_type = other DNA
aaattcatttgag

SEQ ID NO: 29 - DNA, 13 bp, Streptococcus
  misc_feature 1..13: note = Transcribed Leader Seq 27
  source 1..13: mol_type = other DNA
aaaatcatttgag

SEQ ID NO: 30 - DNA, 14 bp, Streptococcus
  misc_feature 1..14: note = Transcribed Leader Seq 28
  source 1..14: mol_type = other DNA
aaaattcatttgag

SEQ ID NO: 31-37 - skipped (7 entries)

SEQ ID NO: 38 - DNA, 10 bp, Streptococcus
  misc_feature 1..10: note = Repeat 8
  source 1..10: mol_type = other DNA
gtttttgtac

SEQ ID NO: 39 - DNA, 11 bp, Streptococcus
  misc_feature 1..11: note = Repeat 9
  source 1..11: mol_type = other DNA
gtttttgtact

SEQ ID NO: 40 - DNA, 12 bp, Streptococcus
  misc_feature 1..12: note = Repeat 10
  source 1..12: mol_type = other DNA
gtttttgtactc

SEQ ID NO: 41 - DNA, 13 bp, Streptococcus
  misc_feature 1..13: note = Repeat 11
  source 1..13: mol_type = other DNA
gtttttgtactct

SEQ ID NO: 42 - DNA, 14 bp, Streptococcus
  misc_feature 1..14: note = Repeat 12
  source 1..14: mol_type = other DNA
gtttttgtactctc

SEQ ID NO: 43 - DNA, 15 bp, Streptococcus
  misc_feature 1..15: note = Repeat 13
  source 1..15: mol_type = other DNA
gtttttgtactctca

SEQ ID NO: 44 - DNA, 16 bp, Streptococcus
  misc_feature 1..16: note = Repeat 14
  source 1..16: mol_type = other DNA
gtttttgtactctcaa

SEQ ID NO: 45 - DNA, 63 bp, Streptococcus thermophilus
  misc_feature 1..63: note = CRISPR leader in the CR1SPR1 locus
  source 1..63: mol_type = other DNA
caaggacagttattgattttataatcactatgtgggtataaaaacgtcaaaatttcatttgag

SEQ ID NO: 46 - DNA, 103 bp, Escherichia coli
  misc_feature 1..103: note = CRISPR leader in the CR1SPR1 locus
  source 1..103: mol_type = other DNA
aaacaaagaattagctgatctttaataataaggaaatgttacattaaggttggtgggttgtttttatgggaaaaaatgctttaagaacaaatgtatacttaga

SEQ ID NO: 47 - protein, 1053 aa, Staphylococcus aureus
  REGION 1..1053: note = CRISPR-associated endonuclease Cas9
MKRNYILGLDIGITSVGYGIIDYETRDVIDAGVRLFKEANVENNEGRRSKRGARRLKRRRRHRIQRVKKLLFDYNLLTDHSELSGINPYEARVKGLSQKLSEEEFSAALLHLAKRRGVHNVNEVEEDTGNELSTKEQISRNSKALEEKYVAELQLERLKKDGEVRGSINRFKTSDYVKEAKQLLKVQKAYHQLDQSFIDTYIDLLETRRTYYEGPGEGSPFGWKDIKEWYEMLMGHCTYFPEELRSVKYAYNADLYNALNDLNNLVITRDENEKLEYYEKFQIIENVFKQKKKPTLKQIAKEILVNEEDIKGYRVTSTGKPEFTNLKVYHDIKDITARKEIIENAELLDQIAKILTIYQSSEDIQEELTNLNSELTQEEIEQISNLKGYTGTHNLSLKAINLILDELWHTNDNQIAIFNRLKLVPKKVDLSQQKEIPTTLVDDFILSPVVKRSFIQSIKVINAIIKKYGLPNDIIIELAREKNSKDAQKMINEMQKRNRQTNERIEEIIRTTGKENAKYLIEKIKLHDMQEGKCLYSLEAIPLEDLLNNPFNYEVDHIIPRSVSFDNSFNNKVLVKQEENSKKGNRTPFQYLSSSDSKISYETFKKHILNLAKGKGRISKTKKEYLLEERDINRFSVQKDFINRNLVDTRYATRGLMNLLRSYFRVNNLDVKVKSINGGFTSFLRRKWKFKKERNKGYKHHAEDALIIANADFIFKEWKKLDKAKKVMENQMFEEKQAESMPEIETEQEYKEIFITPHQIKHIKDFKDYKYSHRVDKKPNRELINDTLYSTRKDDKGNTLIVNNLNGLYDKDNDKLKKLINKSPEKLLMYHHDPQTYQKLKLIMEQYGDEKNPLYKYYEETGNYLTKYSKKDNGPVIKKIKYYGNKLNAHLDITDDYPNSRNKVVKLSLKPYRFDVYLDNGVYKFVTVKNLDVIKKENYYEVNSKCYEEAKKLKKISNQAEFIASFYNNDLIKINGELYRVIGVNNDLLNRIEVNMIDITYREYLENMNDKRPPRIIKTIASKTQSIKKYSTDILGNLYEVKSKKHPQIIKKG

SEQ ID NO: 48 - protein, 1368 aa, Streptococcus pyogenes [sequence omitted]

SEQ ID NO: 49 - DNA, 3162 bp, Staphylococcus aureus
  misc_feature 1..3162: note = Staphylococcus aureus subsp. aureus ORFX gene and pseudo SCCmec-SCC-SCCCRISPR element
  source 1..3162: mol_type = other DNA
atgaaaaggaattatatcttaggattagatatcggaattacatcagtgggttatggaattattgattatgaaactagagatgtcatagatgcgggcgtacgtttatttaaagaggctaatgttgaaaataatgaaggacgacgatcaaaaagaggtgccagaaggcttaagaggcgtcgtagacatagaatacaaagagtaaagaaacttttatttgattacaatttgttgacagatcatagtgagctaagtggaatcaatccttacgaggcgcgcgtaaagggattaagtcaaaaattaagtgaagaggaattttctgcggcattgctacatttagcaaagcgtagaggtgtacataatgttaatgaagtggaagaagatacaggtaatgaattatccactaaagaacaaatttcaagaaatagtaaagcgttagaagagaagtatgttgcagaattacagttggaacgtttgaaaaaagacggtgaagtgagaggttcgattaaccgtttcaaaacatctgactatgtaaaagaagcaaagcagttattaaaagtacaaaaagcatatcatcaacttgatcaatcatttatagacacttatattgatttattggaaacaagaagaacatattatgagggaccaggtgaaggtagcccatttggatggaaagatattaaagaatggtatgaaatgttaatgggacattgtacgtatttcccagaagaattacgtagtgtgaaatatgcctataatgctgatttatataatgcgctgaatgatttgaacaacttggttattacacgagatgagaatgagaagctagagtattatgaaaaattccaaattatcgagaatgtctttaaacaaaagaaaaagccgacgcttaaacaaattgcgaaggaaatcttggtgaatgaagaagacatcaaaggctatcgtgtcacaagtacaggtaaaccagaatttacaaacttgaaagtttatcacgatatcaaagatattacagcaagaaaagaaattatcgagaatgcagagctactcgatcaaatagctaaaatattaactatttaccagtcatcagaagatatacaagaagaattaacaaacctaaattcagaattgacacaagaagagattgaacaaatttcaaacttgaaaggttatacaggaactcataacctttcactaaaggcaataaatttaatattagacgaattgtggcatacgaacgataatcaaatagctattttcaatcgtttgaaacttgtacctaaaaaggtagatttaagccaacaaaaagaaattcctactactttagttgatgattttatactgtctccagtagtgaaacgttcatttatacaatctattaaagttattaacgctattattaaaaaatacggtttgccaaatgatattattattgaacttgcgagagaaaagaattctaaagatgcacaaaaaatgattaatgaaatgcagaagagaaatcgtcaaacgaatgaacgtattgaggaaattataagaacgacaggtaaagaaaatgctaaatatttaattgaaaaaattaagctgcacgatatgcaagaagggaaatgtttatactcgttagaagcaatccctctagaagatttacttaataatccattcaattacgaagtagaccatatcattccacgttctgtttctttcgataactctttcaataataaagtgttggtgaaacaagaagaaaatagtaaaaaaggtaatagaacgccatttcaatatttaagttcttcagattctaaaataagttatgagacattcaaaaagcatattttaaatcttgctaaaggcaaaggtagaatctctaagacgaaaaaagaatatttgttagaagaacgagatatcaatcgcttcagtgtccaaaaagattttattaaccgtaacttagtagatacacgctatgcgacaagagggttaatgaacttattaagatcttattttagagtgaataacttagatgtcaaagtgaaatcgattaatggcggattcacaagtttcttaagaaggaaatggaagttcaaaaaagaaagaaataagggctacaaacaccatgctgaagatgcactgattattgcgaacgctgattttattttcaaagaatggaaaaaactagataaagctaaaaaagtgatggaaaatcaaatgtttgaagaaaagcaagctgaaagtatgcctgaaattgagactgagcaagagtataaagaaatttttataacgcctcatcaaattaaacatattaaggattttaaagattataaatattcacatagagttgataaaaagccgaatagagagttaataaatgatacattatattctacgagaaaagatgacaagggtaatacattaatcgttaataacttaaatggtttatacgataaagataatgataaattgaaaaaattaattaataaatcacctgaaaaattattgatgtatcatcatgatccacaaacatatcaaaaattaaaattgatcatggaacaatatggcgatgagaaaaatccgctttataaatattatgaagaaacaggcaattacttaacaaaatatagtaaaaaagataacggaccagtcatcaaaaaaattaaatattatggtaacaagctaaatgcgcatttagatattacggatgattatccaaatagcagaaataaagtagtaaaactttcattaaaaccatatcgctttgatgtttatttagataatggggtatataaatttgtgacagttaaaaatttagatgttatcaaaaaagaaaactactatgaagttaattcaaagtgttatgaagaagcaaaaaaactgaagaaaattagtaatcaagcagaatttatcgcaagtttttacaataatgacttgattaagattaacggagaattatatagagtcataggtgtaaataatgatctacttaacagaattgaagtaaatatgatagacatcacatatagagaatatttagagaacatgaatgataaaagaccacctagaataattaaaacaatagcaagcaaaacacaatctattaaaaagtattctacagatattctaggcaatctttatgaagtgaagagtaaaaagcatcctcaaatcataaagaaaggatga

SEQ ID NO: 50 - DNA, 23 bp, Desulfovibrio desulfuricans
  misc_feature 1..23: note = Desulphovibrio desulphuricans ND132 NC_016803_1
  source 1..23: mol_type = other DNA
cctggcctgccccaagtgcaagg

SEQ ID NO: 51 - DNA, 32 bp, Desulfovibrio desulfuricans
  misc_feature 1..32: note = Desulphovibrio desulphuricans ND132 NC_016803_4
  source 1..32: mol_type = other DNA
gtcgccccccacgcgggggcgtggattgaaac

SEQ ID NO: 52 - DNA, 28 bp, Desulfovibrio desulfuricans
  misc_feature 1..28: note = Desulphovibrio desulphuricans subsp. desulphuricans str. (ATCC 27774) NC_011883_1
  source 1..28: mol_type = other DNA
tggagcgggaaacgggatttgaacccgc

SEQ ID NO: 53 - DNA, 29 bp, Desulfovibrio desulfuricans
  misc_feature 1..29: note = Desulphovibrio desulphuricans subsp. desulphuricans str. (ATCC 27774) NC_011883_2
  source 1..29: mol_type = other DNA
gtgttccccacgggcgtggggatgaaccg

SEQ ID NO: 54 - DNA, 25 bp, Desulfovibrio gigas
  misc_feature 1..25: note = Desulphovibrio gigas DSM 1382 (ATCC 19364) NC_022444_2
  source 1..25: mol_type = other DNA
aacctttctgcaaaaaggtttcccc

SEQ ID NO: 55 - DNA, 23 bp, Desulfovibrio gigas
  misc_feature 1..23: note = Desulphovibrio gigas DSM 1382 (ATCC 19364) NC_022444_3
  source 1..23: mol_type = other DNA
ccgctggatccggctgcagcgcc

SEQ ID NO: 56 - DNA, 28 bp, Desulfovibrio gigas
  misc_feature 1..28: note = Desulphovibrio gigas DSM 1382 (ATCC 19364) NC_022444_4
  source 1..28: mol_type = other DNA
gttcactgccgcataggcagctcagaaa

SEQ ID NO: 57 - DNA, 32 bp, Desulfovibrio gigas
  misc_feature 1..32: note = Desulphovibrio gigas DSM 1382 (ATCC 19364) NC_022444_5
  source 1..32: mol_type = other DNA
cacccgactattgaagtcgggcctcattgaag

SEQ ID NO: 58 - DNA, 36 bp, Desulfovibrio hydrothermalis
  misc_feature 1..36: note = Desulphovibrio hydrothermalis NC_022579_1
  source 1..36: mol_type = other DNA
gtcaaaacccataccgatatggatacctcttttgag

SEQ ID NO: 59 - DNA, 36 bp, Desulfovibrio hydrothermalis; identical to SEQ ID NO: 58
  misc_feature 1..36: note = Desulphovibrio hydrothermalis NC_022579_2
  source 1..36: mol_type = other DNA

SEQ ID NO: 60 - DNA, 36 bp, Desulfovibrio hydrothermalis; identical to SEQ ID NO: 58
  misc_feature 1..36: note = Desulphovibrio hydrothermalis NC_022579_3
  source 1..36: mol_type = other DNA

SEQ ID NO: 61 - DNA, 36 bp, Desulfovibrio hydrothermalis; identical to SEQ ID NO: 58
  misc_feature 1..36: note = Desulphovibrio hydrothermalis NC_022579_4
  source 1..36: mol_type = other DNA

SEQ ID NO: 62 - DNA, 36 bp, Desulfovibrio hydrothermalis
  misc_feature 1..36: note = Desulphovibrio hydrothermalis NC_022579_5
  source 1..36: mol_type = other DNA
ctcaaaagaggtatccatatcggtatgggttttgac

SEQ ID NO: 63 - DNA, 28 bp, Desulfovibrio hydrothermalis
  misc_feature 1..28: note = Desulphovibrio hydrothermalis NC_022579_6
  source 1..28: mol_type = other DNA
gttcactgccggataggcagcttagaaa

SEQ ID NO: 64 - DNA, 32 bp, Desulfovibrio magneticus
  misc_feature 1..32: note = Desulphovibrio magneticus RS-1 NC_012796_1
  source 1..32: mol_type = other DNA
gtcgccccctgcgcgggggcgtggattgaaac

SEQ ID NO: 65 - DNA, 29 bp, Desulfovibrio magneticus
  misc_feature 1..29: note = Desulphovibrio magneticus RS-1 NC_012796_3
  source 1..29: mol_type = other DNA
ttttctgagctgcctatgcggcagtgaac

SEQ ID NO: 66 - DNA, 46 bp, Desulfovibrio vulgaris
  misc_feature 1..46: note = Desulphovibrio vulgaris str. 'Miyazaki F' NC_011769_1
  source 1..46: mol_type = other DNA
catcgacgacgaacccgggcaccgcctgatggtccacgccgtcatg

SEQ ID NO: 67 - DNA, 32 bp, Desulfovibrio vulgaris
  misc_feature 1..32: note = Desulphovibrio vulgaris str. 'Miyazaki F' NC_011769_3
  source 1..32: mol_type = other DNA
gtcgcccctcacgcgggggcgtggatagaaac

SEQ ID NO: 68 - DNA, 32 bp, Desulfovibrio vulgaris
  misc_feature 1..32: note = Desulphovibrio vulgaris subsp. vulgaris DP4 NC_008741_1
  source 1..32: mol_type = other DNA
gtttcaatccacgcccccgcacggggggcgac

SEQ ID NO: 69 - DNA, 28 bp, Desulfurispirillum indicum S5
  misc_feature 1..28: note = Desulphurispirillum indicum S5 NC_014836_1
  source 1..28: mol_type = other DNA
tttctgagctgcctatgcggcagtgaac

SEQ ID NO: 70 - DNA, 36 bp, Desulfurispirillum indicum S5
  misc_feature 1..36: note = Desulphurispirillum indicum S5 NC_014836_2
  source 1..36: mol_type = other DNA
gaccgaagacctgtcggaaacgacggggattgagac

SEQ ID NO: 71 - DNA, 29 bp, Desulfurivibrio alkaliphilus AHT2
  misc_feature 1..29: note = Desulphurivibrio alkaliphilus AHT2 NC_014216_2
  source 1..29: mol_type = other DNA
cggttcatccccgcgagtgcggggaacat

SEQ ID NO: 72 - DNA, 28 bp, Desulfurivibrio alkaliphilus AHT2
  misc_feature 1..28: note = Desulphurivibrio alkaliphilus AHT2 NC_014216_3
  source 1..28: mol_type = other DNA
tttctgagctgcctgtgcggcagtgaac

SEQ ID NO: 73 - DNA, 29 bp, Desulfurobacterium thermolithotrophum DSM 11699
  misc_feature 1..29: note = Desulphurobacterium thermolithotrophum DSM 11699 NC_015185_1
  source 1..29: mol_type = other DNA
gttttatctgaacgtagtgggatataaag

SEQ ID NO: 74 - DNA, 29 bp, Desulfovibrio desulfuricans
  misc_feature 1..29: note = Desulphovibrio desulphuricans G20 NC_007519_1
  source 1..29: mol_type = other DNA
cggttcatccccgcgggtgcggggaacac

SEQ ID NO: 75 - RNA, 28 nt, Phage ICP1
  misc_feature 1..28: note = CR1 and CR2 consensus direct repeat with the partially palindromic sequence forming the predicted stem in the crRNA
  source 1..28: mol_type = other RNA
gttagcagccgcataggctgcttaaata

SEQ ID NO: 76 - DNA, 33 bp, Vibrio cholerae
  misc_feature 1..33: note = V. cholerae PICI-like element
  source 1..33: mol_type = other DNA
aatttaaatagggaagataagcaaagggttgac

SEQ ID NO: 77 - DNA, 31 bp, Vibrio cholerae
  misc_feature 1..31: note = V. cholerae PICI-like element protospacer sequence
  source 1..31: mol_type = other DNA
tttaaatagggaagataagcaaagggttgac

SEQ ID NO: 78 - protein, 11 aa, Vibrio cholerae
  REGION 1..11: note = V. cholerae PICI-like element
NLNREDKQRVD

SEQ ID NO: 79 - DNA, 32 bp, Phage ICP1
  misc_feature 1..32: note = ICP1_ 2011_A CR1 1a
  source 1..32: mol_type = other DNA
cattgcaactatgcaaaatgatgaagctaaaa

SEQ ID NO: 80 - DNA, 32 bp, Phage ICP1
  misc_feature 1..32: note = ICP1_ 2011_A CR1 2a
  source 1..32: mol_type = other DNA
tgttagagtcggtagtatctggatgatcgata

SEQ ID NO: 81 - DNA, 32 bp, Phage ICP1
  misc_feature 1..32: note = ICP1_ 2011_A CR1 3a
  source 1..32: mol_type = other DNA
ttatgtattgaccccgacacgccccccgactg

SEQ ID NO: 82 - DNA, 32 bp, Phage ICP1
  misc_feature 1..32: note = ICP1_ 2011_A CR1 4a
  source 1..32: mol_type = other DNA
ttacagacgacctaactcttcagtaccatgat

SEQ ID NO: 83 - DNA, 32 bp, Phage ICP1
  misc_feature 1..32: note = ICP1_ 2011_A CR1 5a
  source 1..32: mol_type = other DNA
tacataagctgcaacacggtgttcgtttaagt

SEQ ID NO: 84 - DNA, 32 bp, Phage ICP1
  misc_feature 1..32: note = ICP1_ 2011_A CR1 6a
  source 1..32: mol_type = other DNA
aaaatacgcctttttcccttcatcgtttaaag

SEQ ID NO: 85 - DNA, 32 bp, Phage ICP1
  misc_feature 1..32: note = ICP1_ 2011_A CR1 7a
  source 1..32: mol_type = other DNA
accaacaaatcccataaactgataaccacgtt

SEQ ID NO: 86 - DNA, 32 bp, Phage ICP1
  misc_feature 1..32: note = ICP1_ 2011_A CR1 8a
  source 1..32: mol_type = other DNA
gtcaaccctttgcttatcttccctatttaaat

SEQ ID NO: 87 - DNA, 32 bp, Phage ICP1
  misc_feature 1..32: note = ICP1_ 2011_A CR1 9a
  source 1..32: mol_type = other DNA
tgttaaccaccgcttgaaataatcatgatgca

SEQ ID NO: 88 - DNA, 32 bp, Phage ICP1
  misc_feature 1..32: note = ICP1_ 2006_E CR1 1b
  source 1..32: mol_type = other DNA
tgtgtctatactcaaccaatttaagcgccgca

SEQ ID NO: 89 - DNA, 32 bp, Phage ICP1
  misc_feature 1..32: note = ICP1_ 2006_E CR1 2b
  source 1..32: mol_type = other DNA
ctactctccccaatattagccattcctaattc

SEQ ID NO: 90 - DNA, 32 bp, Phage ICP1
  misc_feature 1..32: note = ICP1_ 2006_E CR1 3b
  source 1..32: mol_type = other DNA
gtcaccttaccgtaagacaggcagtaaaatta

SEQ ID NO: 91 - DNA, 32 bp, Phage ICP1
  misc_feature 1..32: note = ICP1_ 2006_E CR1 4b
  source 1..32: mol_type = other DNA
aaactagtggacgtaatgcagtattcacggtt

SEQ ID NO: 92 - DNA, 32 bp, Phage ICP1
  misc_feature 1..32: note = ICP1_ 2006_E CR2 1c
  source 1..32: mol_type = other DNA
atccacactacaaatagaacactcaaccgtga

SEQ ID NO: 93 - DNA, 32 bp, Phage ICP1; identical to SEQ ID NO: 88
  misc_feature 1..32: note = ICP1_ 2005_A CR1 1d
  source 1..32: mol_type = other DNA

SEQ ID NO: 94 - DNA, 32 bp, Phage ICP1; identical to SEQ ID NO: 89
  misc_feature 1..32: note = ICP1_ 2005_A CR1 2d
  source 1..32: mol_type = other DNA

SEQ ID NO: 95 - DNA, 32 bp, Phage ICP1; identical to SEQ ID NO: 91
  misc_feature 1..32: note = ICP1_ 2005_A CR1 3d
  source 1..32: mol_type = other DNA

SEQ ID NO: 96 - DNA, 32 bp, Phage ICP1
  misc_feature 1..32: note = ICP1_ 2005_A CR1 4d
  source 1..32: mol_type = other DNA
ataatcgttttgagtctcaccagcttttaggc

SEQ ID NO: 97 - DNA, 32 bp, Phage ICP1; identical to SEQ ID NO: 92
  misc_feature 1..32: note = ICP1_ 2005_A CR2 1e
  source 1..32: mol_type = other DNA

SEQ ID NO: 98 - DNA, 32 bp, Phage ICP1
  misc_feature 1..32: note = ICP1_ 2005_A CR2 2e
  source 1..32: mol_type = other DNA
tattgattggtctctaaccttgggatgattaa

SEQ ID NO: 99 - DNA, 32 bp, Phage ICP1
  misc_feature 1..32: note = ICP1_ 2005_A CR2 3e
  source 1..32: mol_type = other DNA
ttcacgggtagcaacagggtaataaaccaata

SEQ ID NO: 100 - DNA, 32 bp, Phage ICP1; identical to SEQ ID NO: 79
  misc_feature 1..32: note = ICP1_ 2004_A CR1 1f
  source 1..32: mol_type = other DNA

SEQ ID NO: 101 - DNA, 32 bp, Phage ICP1; identical to SEQ ID NO: 80
  misc_feature 1..32: note = ICP1_ 2004_A CR1 2f
  source 1..32: mol_type = other DNA

SEQ ID NO: 102 - DNA, 32 bp, Phage ICP1
  misc_feature 1..32: note = ICP1_ 2004_A CR1 3f
  source 1..32: mol_type = other DNA
tagaagagtaataggagctactgcaaacttgt

SEQ ID NO: 103 - DNA, 32 bp, Phage ICP1
  misc_feature 1..32: note = ICP1_ 2004_A CR1 4f
  source 1..32: mol_type = other DNA
taactatgtgtggtttatattttgtgtgcaag

SEQ ID NO: 104 - DNA, 32 bp, Phage ICP1
  misc_feature 1..32: note = ICP1_ 2004_A CR1 5f
  source 1..32: mol_type = other DNA
ttttgaaactattgacagaaggttgggaacct

SEQ ID NO: 105 - DNA, 32 bp, Phage ICP1
  misc_feature 1..32: note = ICP1_ 2004_A CR1 6f
  source 1..32: mol_type = other DNA
ttgaggttgaacctcttccggttcctcttctg

SEQ ID NO: 106 - DNA, 32 bp, Phage ICP1
  misc_feature 1..32: note = ICP1_ 2004_A CR2 1g
  source 1..32: mol_type = other DNA
gtgtattgcttgcagtgggttacacacaagaa

SEQ ID NO: 107 - DNA, 47 bp, Bacteroides fragilis
  misc_feature 1..47: note = Bacteriodes Repeat 1
  source 1..47: mol_type = other DNA
gttgtgatttgctttcaaattagtatctttgaaccattggaaacagc

SEQ ID NO: 108 - DNA, 29 bp, Bacteroides fragilis
  misc_feature 1..29: note = Bacteriodes Repeat 2
  source 1..29: mol_type = other DNA
atttcaattccataaggtacaattaatac

SEQ ID NO: 109 - DNA, 32 bp, Bacteroides helcogenes P 36-108
  misc_feature 1..32: note = Bacteriodes Repeat 3
  source 1..32: mol_type = other DNA
gtttcaatccacacacccgtatagggtgtgac

SEQ ID NO: 110 - DNA, 47 bp, Bacteroides sp. CF50
  misc_feature 1..47: note = Bacteriodes Repeat 4
  source 1..47: mol_type = other DNA
actgtttctgatatgtcaaagataaaattttgaaagcaaatcacaac

SEQ ID NO: 111 - DNA, 23 bp, Bacteroides thetaiotaomicron VPI-5482
  misc_feature 1..23: note = Bacteriodes Repeat 5
  source 1..23: mol_type = other DNA
gaaaaaatacagtttcgctctca

SEQ ID NO: 112 - DNA, 32 bp, Prevotella dentalis DSM 3688
  misc_feature 1..32: note = Prevotella Repeat 1
  source 1..32: mol_type = other DNA
gtcgcgtctcacgtaggcgcgtggattgaaac

SEQ ID NO: 113 - DNA, 47 bp, Prevotella denticola F0289
  misc_feature 1..47: note = Prevotella Repeat 2
  source 1..47: mol_type = other DNA
attgtgcttgctactgcaaagatacacattttgaagcaattcacaac

SEQ ID NO: 114 - DNA, 37 bp, Prevotella denticola F0289
  misc_feature 1..37: note = Prevotella Repeat 3
  source 1..37: mol_type = other DNA
ctcaatgagtatcttccattaaaacaaggattaagac

SEQ ID NO: 115 - DNA, 36 bp, Prevotella intermedia 17
  misc_feature 1..36: note = Prevotella Repeat 5
  source 1..36: mol_type = other DNA
gttgtttttaccttgcaaacagcaggcagatacaac

SEQ ID NO: 116 - DNA, 47 bp, Prevotella intermedia 17
  misc_feature 1..47: note = Prevotella Repeat 6
  source 1..47: mol_type = other DNA
gttgtatttgccaatgcaaagatactaattttaaagctaatcacaac

SEQ ID NO: 117 - DNA, 36 bp, Prevotella ruminicola 23
  misc_feature 1..36: note = Prevotella Repeat 7
  source 1..36: mol_type = other DNA
gttgtatatcattcctttcctacatcaaaccacaac

SEQ ID NO: 118 - DNA, 29 bp, Clostridium difficile 630
  misc_feature 1..29: note = C dificile strain 630 repeat
  source 1..29: mol_type = other DNA
atttacataccacttagttaatataaaac

SEQ ID NO: 119 - DNA, 29 bp, Clostridium difficile 630
  misc_feature 1..29: note = C dificile strain 630 repeat 2
  source 1..29: mol_type = other DNA
gttttatattaactaagtggtatgtaaat

SEQ ID NO: 120 - DNA, 112 bp, unidentified
  source 1..112: mol_type = other DNA
  misc_feature 1..112: note = tracrRNA-encoding sequence
ttaaataacgaaaacaccctgccataaaatgacagggtgttgatttcggcatgaagccttatctttgtagcttctgcaagatttaagtaactgtgtaaggcgtcccttacac

SEQ ID NO: 121 - DNA, 30 bp, unidentified
  misc_feature 1..30: note = S1. spacer 1 (DNA Pol lll)
  source 1..30: mol_type = other DNA
tgtcctatgaatcagctccttttctcggcc

SEQ ID NO: 122 - DNA, 30 bp, unidentified
  misc_feature 1..30: note = S2. spacer 2 (tetA)
  source 1..30: mol_type = other DNA
ggctataagataaactacgggcaagtttga

SEQ ID NO: 123 - DNA, 487 bp, unidentified
  misc_feature 1..487: note = pBAV1KTXylR-short1 CRISPR array
  source 1..487: mol_type = other DNA
gcggataacaattactagagaaagaggagaaatactattcttctcctctttaaataacgaaaacaccctgccataaaatgacagggtgttgatttcggcatgaagccttatctttgtagcttctgcaagatttaagtaactgtgtaaggcgtcccttacacttgcatgtatagttattataccagggggacagtgcaatgtcaagaataaactgtagaatgactagtgacttaaatcttgagagtacaaaaacccgttggaatcgtgattaatagtaactgttgttgtacagttacttaaatcttgagagtacaaaaacggccgagaaaaggagctgattcataggacagttgtacagttacttaaatcttgagagtacaaaaactcaaacttgcccgtagtttatcttatagccgttgtacagttacttaaatcttgagagtacaaaaacatttacctcctttgatttaagtgaacaagtttatcc

SEQ ID NO: 124 - DNA, 221 bp, unidentified
  misc_feature 1..221: note = Repeat-spacers sequence
  source 1..221: mol_type = other DNA
ttaaatcttgagagtacaaaaacccgttggaatcgtgattaatagtaactgttgttgtacagttacttaaatcttgagagtacaaaaacggccgagaaaaggagctgattcataggacagttgtacagttacttaaatcttgagagtacaaaaactcaaacttgcccgtagtttatcttatagccgttgtacagttacttaaatcttgagagtacaaaaac

SEQ ID NO: 125 - DNA, 32 bp, Desulfovibrio vulgaris str. Hildenborough; identical to SEQ ID NO: 51
  misc_feature 1..32: note = Desulphovibrio vulgaris subsp. vulgaris str. Hildenborough NC_005863_3
  source 1..32: mol_type = other DNA

SEQ ID NO: 126 - DNA, 32 bp, Desulfobulbus propionicus DSM 2032; identical to SEQ ID NO: 51
  misc_feature 1..32: note = Desulphobulbus propionicus DSM 2032 NC_014972_1
  source 1..32: mol_type = other DNA

SEQ ID NO: 127 - DNA, 25 bp, Desulphurispirillum indicum S5
  misc_feature 1..25: note = Desulphurispirillum indicum S5
  source 1..25: mol_type = other DNA
aacctttctgcaaaaaggtttcccc

SEQ ID NO: 128 - DNA, 28 bp, Desulfovibrio gigas
  misc_feature 1..28: note = Desulphovibrio gigas DSM 1382 (ATCC 19364)
  source 1..28: mol_type = other DNA
tttctgagctgcctatgcggcagtgaac

SEQ ID NO: 129 - DNA, 43 bp, unidentified
  misc_feature 1..43: note = PJ23100 Promoter
  source 1..43: mol_type = other DNA
ttgacggctagctcagtcctaggtacagtgctagctactagag

SEQ ID NO: 130 - DNA, 102 bp, unidentified
  misc_feature 1..102: note = Linker+ Theophylline riboswitch Regulator
  source 1..102: mol_type = other DNA
aagtctagcgaaccgcacttaatacgactcactataggtaccggtgataccagcatcgtcttgatgcccttggcagcaccctgctaaggtaacaacaagatg

SEQ ID NO: 131 - DNA, 4107 bp, Streptococcus pyogenes
  misc_feature 1..4107: note = Cas9 from Streptococcus pyogens
  source 1..4107: mol_type = other DNA
atggataagaaatactcaataggcttagatatcggcacaaatagcgtcggatgggcggtgatcactgatgaatataaggttccgtctaaaaagttcaaggttctgggaaatacagaccgccacagtatcaaaaaaaatcttataggggctcttttatttgacagtggagagacagcggaagcgactcgtctcaaacggacagctcgtagaaggtatacacgtcggaagaatcgtatttgttatctacaggagattttttcaaatgagatggcgaaagtagatgatagtttctttcatcgacttgaagagtcttttttggtggaagaagacaagaagcatgaacgtcatcctatttttggaaatatagtagatgaagttgcttatcatgagaaatatccaactatctatcatctgcgaaaaaaattggtagattctactgataaagcggatttgcgcttaatctatttggccttagcgcatatgattaagtttcgtggtcattttttgattgagggagatttaaatcctgataatagtgatgtggacaaactatttatccagttggtacaaacctacaatcaattatttgaagaaaaccctattaacgcaagtggagtagatgctaaagcgattctttctgcacgattgagtaaatcaagacgattagaaaatctcattgctcagctccccggtgagaagaaaaatggcttatttgggaatctcattgctttgtcattgggtttgacccctaattttaaatcaaattttgatttggcagaagatgctaaattacagctttcaaaagatacttacgatgatgatttagataatttattggcgcaaattggagatcaatatgctgatttgtttttggcagctaagaatttatcagatgctattttactttcagatatcctaagagtaaatactgaaataactaaggctcccctatcagcttcaatgattaaacgctacgatgaacatcatcaagacttgactcttttaaaagctttagttcgacaacaacttccagaaaagtataaagaaatcttttttgatcaatcaaaaaacggatatgcaggttatattgatgggggagctagccaagaagaattttataaatttatcaaaccaattttagaaaaaatggatggtactgaggaattattggtgaaactaaatcgtgaagatttgctgcgcaagcaacggacctttgacaacggctctattccccatcaaattcacttgggtgagctgcatgctattttgagaagacaagaagacttttatccatttttaaaagacaatcgtgagaagattgaaaaaatcttgacttttcgaattccttattatgttggtccattggcgcgtggcaatagtcgttttgcatggatgactcggaagtctgaagaaacaattaccccatggaattttgaagaagttgtcgataaaggtgcttcagctcaatcatttattgaacgcatgacaaactttgataaaaatcttccaaatgaaaaagtactaccaaaacatagtttgctttatgagtattttacggtttataacgaattgacaaaggtcaaatatgttactgaaggaatgcgaaaaccagcatttctttcaggtgaacagaagaaagccattgttgatttactcttcaaaacaaatcgaaaagtaaccgttaagcaattaaaagaagattatttcaaaaaaatagaatgttttgatagtgttgaaatttcaggagttgaagatagatttaatgcttcattaggtacctaccatgatttgctaaaaattattaaagataaagattttttggataatgaagaaaatgaagatatcttagaggatattgttttaacattgaccttatttgaagatagggagatgattgaggaaagacttaaaacatatgctcacctctttgatgataaggtgatgaaacagcttaaacgtcgccgttatactggttggggacgtttgtctcgaaaattgattaatggtattagggataagcaatctggcaaaacaatattagattttttgaaatcagatggttttgccaatcgcaattttatgcagctgatccatgatgatagtttgacatttaaagaagacattcaaaaagcacaagtgtctggacaaggcgatagtttacatgaacatattgcaaatttagctggtagccctgctattaaaaaaggtattttacagactgtaaaagttgttgatgaattggtcaaagtaatggggcggcataagccagaaaatatcgttattgaaatggcacgtgaaaatcagacaactcaaaagggccagaaaaattcgcgagagcgtatgaaacgaatcgaagaaggtatcaaagaattaggaagtcagattcttaaagagcatcctgttgaaaatactcaattgcaaaatgaaaagctctatctctattatctccaaaatggaagagacatgtatgtggaccaagaattagatattaatcgtttaagtgattatgatgtcgatcacattgttccacaaagtttccttaaagacgattcaatagacaataaggtcttaacgcgttctgataaaaatcgtggtaaatcggataacgttccaagtgaagaagtagtcaaaaagatgaaaaactattggagacaacttctaaacgccaagttaatcactcaacgtaagtttgataatttaacgaaagctgaacgtggaggtttgagtgaacttgataaagctggttttatcaaacgccaattggttgaaactcgccaaatcactaagcatgtggcacaaattttggatagtcgcatgaatactaaatacgatgaaaatgataaacttattcgagaggttaaagtgattaccttaaaatctaaattagtttctgacttccgaaaagatttccaattctataaagtacgtgagattaacaattaccatcatgcccatgatgcgtatctaaatgccgtcgttggaactgctttgattaagaaatatccaaaacttgaatcggagtttgtctatggtgattataaagtttatgatgttcgtaaaatgattgctaagtctgagcaagaaataggcaaagcaaccgcaaaatatttcttttactctaatatcatgaacttcttcaaaacagaaattacacttgcaaatggagagattcgcaaacgccctctaatcgaaactaatggggaaactggagaaattgtctgggataaagggcgagattttgccacagtgcgcaaagtattgtccatgccccaagtcaatattgtcaagaaaacagaagtacagacaggcggattctccaaggagtcaattttaccaaaaagaaattcggacaagcttattgctcgtaaaaaagactgggatccaaaaaaatatggtggttttgatagtccaacggtagcttattcagtcctagtggttgctaaggtggaaaaagggaaatcgaagaagttaaaatccgttaaagagttactagggatcacaattatggaaagaagttcctttgaaaaaaatccgattgactttttagaagctaaaggatataaggaagttaaaaaagacttaatcattaaactacctaaatatagtctttttgagttagaaaacggtcgtaaacggatgctggctagtgccggagaattacaaaaaggaaatgagctggctctgccaagcaaatatgtgaattttttatatttagctagtcattatgaaaagttgaagggtagtccagaagataacgaacaaaaacaattgtttgtggagcagcataagcattatttagatgagattattgagcaaatcagtgaattttctaagcgtgttattttagcagatgccaatttagataaagttcttagtgcatataacaaacatagagacaaaccaatacgtgaacaagcagaaaatattattcatttatttacgttgacgaatcttggagctcccgctgcttttaaatattttgatacaacaattgatcgtaaacgatatacgtctacaaaagaagttttagatgccactcttatccatcaatccatcactggtctttatgaaacacgcattgatttgagtcagctaggaggtgactga

SEQ ID NO: 132 - DNA, 1221 bp, Streptococcus pyogenes
  misc_feature 1..1221: note = pSC101 Origin of replication and replicon
  source 1..1221: mol_type = other DNA
gagttatacacagggctgggatctattctttttatctttttttattctttctttattctataaattataaccacttgaatataaacaaaaaaaacacacaaaggtctagcggaatttacagagggtctagcagaatttacaagttttccagcaaaggtctagcagaatttacagatacccacaactcaaaggaaaaggacatgtaattatcattgactagcccatctcaattggtatagtgattaaaatcacctagaccaattgagatgtatgtctgaattagttgttttcaaagcaaatgaactagcgattagtcgctatgacttaacggagcatgaaaccaagctaattttatgctgtgtggcactactcaaccccacgattgaaaaccctacaaggaaagaacggacggtatcgttcacttataaccaatacgctcagatgatgaacatcagtagggaaaatgcttatggtgtattagctaaagcaaccagagagctgatgacgagaactgtggaaatcaggaatcctttggttaaaggctttgagattttccagtggacaaactatgccaagttctcaagcgaaaaattagaattagtttttagtgaagagatattgccttatcttttccagttaaaaaaattcataaaatataatctggaacatgttaagtcttttgaaaacaaatactctatgaggatttatgagtggttattaaaagaactaacacaaaagaaaactcacaaggcaaatatagagattagccttgatgaatttaagttcatgttaatgcttgaaaataactaccatgagtttaaaaggcttaaccaatgggttttgaaaccaataagtaaagatttaaacacttacagcaatatgaaattggtggttgataagcgaggccgcccgactgatacgttgattttccaagttgaactagatagacaaatggatctcgtaaccgaacttgagaacaaccagataaaaatgaatggtgacaaaataccaacaaccattacatcagattcctacctacataacggactaagaaaaacactacacgatgctttaactgcaaaaattcagctcaccagttttgaggcaaaatttttgagtgacatgcaaagtaagtatgatctcaatggttcgttctcatggctcacgcaaaaacaacgaaccacactagagaacatactggctaaatacggaaggatctga

SEQ ID NO: 133 - DNA, 789 bp, unidentified
  misc_feature 1..789: note = aadA Spectinomycin resistance gene
  source 1..789: mol_type = other DNA
atgagggaagcggtgatcgccgaagtatcgactcaactatcagaggtagttggcgtcatcgagcgccatctcgaaccgacgttgctggccgtacatttgtacggctccgcagtggatggcggcctgaagccacacagtgatattgatttgctggttacggtgaccgtaaggcttgatgaaacaacgcggcgagctttgatcaacgaccttttggaaacttcggcttcccctggagagagcgagattctccgcgctgtagaagtcaccattgttgtgcacgacgacatcattccgtggcgttatccagctaagcgcgaactgcaatttggagaatggcagcgcaatgacattcttgcaggtatcttcgagccagccacgatcgacattgatctggctatcttgctgacaaaagcaagagaacatagcgttgccttggtaggtccagcggcggaggaactctttgatccggttcctgaacaggatctatttgaggcgctaaatgaaaccttaacgctatggaactcgccgcccgactgggctggcgatgagcgaaatgtagtgcttacgttgtcccgcatttggtacagcgcagtaaccggcaaaatcgcgccgaaggatgtcgctgccgactgggcaatggagcgcctgccggcccagtatcagcccgtcatacttgaagctagacaggcttatcttggacaagaagaagatcgcttggcctcgcgcgcagatcagttggaagaatttgtccactacgtgaaaggcgagatcaccaaggtagtcggcaaa

SEQ ID NO: 134 - DNA, 1191 bp, unidentified
  misc_feature 1..1191: note = AraC/PBAD Arabinose expression system
  source 1..1191: mol_type = other DNA
ttatgacaacttgacggctacatcattcactttttcttcacaaccggcacggaactcgctcgggctggccccggtgcattttttaaatacccgcgagaaatagagttgatcgtcaaaaccaacattgcgaccgacggtggcgataggcatccgggtggtgctcaaaagcagcttcgcctggctgatacgttggtcctcgcgccagcttaagacgctaatccctaactgctggcggaaaagatgtgacagacgcgacggcgacaagcaaacatgctgtgcgacgctggcgatatcaaaattgctgtctgccaggtgatcgctgatgtactgacaagcctcgcgtacccgattatccatcggtggatggagcgactcgttaatcgcttccatgcgccgcagtaacaattgctcaagcagatttatcgccagcagctccgaatagcgcccttccccttgcccggcgttaatgatttgcccaaacaggtcgctgaaatgcggctggtgcgcttcatccgggcgaaagaaccccgtattggcaaatattgacggccagttaagccattcatgccagtaggcgcgcggacgaaagtaaacccactggtgataccattcgcgagcctccggatgacgaccgtagtgatgaatctctcctggcgggaacagcaaaatatcacccggtcggcaaacaaattctcgtccctgatttttcaccaccccctgaccgcgaatggtgagattgagaatataacctttcattcccagcggtcggtcgataaaaaaatcgagataaccgttggcctcaatcggcgttaaacccgccaccagatgggcattaaacgagtatcccggcagcaggggatcattttgcgcttcagccatacttttcatactcccgccattcagagaagaaaccaattgtccatattgcatcagacattgccgtcactgcgtcttttactggctcttctcgctaaccaaaccggtaaccccgcttattaaaagcattctgtaacaaagcgggaccaaagccatgacaaaaacgcgtaacaaaagtgtctataatcacggcagaaaagtccacattgattatttgcacggcgtcacactttgctatgccatagcatttttatccataagattagcggatcctacctgacgctttttatcgcaactctctactgtttctccata

SEQ ID NO: 135 - DNA, 657 bp, unidentified
  misc_feature 1..657: note = Chloroamphenicol resistance gene
  source 1..657: mol_type = other DNA
atggagaaaaaaatcactggatataccaccgttgatatatcccaatggcatcgtaaagaacattttgaggcatttcagtcagttgctcaatgtacctataaccagaccgttcagctggatattacggcctttttaaagaccgtaaagaaaaataagcacaagttttatccggcctttattcacattcttgcccgcctgatgaatgctcatccggaatttcgtatggcaatgaaagacggtgagctggtgatatgggatagtgttcacccttgttacaccgttttccatgagcaaactgaaacgttttcatcgctctggagtgaataccacgacgatttccggcagtttctacacatatattcgcaagatgtggcgtgttacggtgaaaacctggcctatttccctaaagggtttattgagaatatgtttttcgtctcagccaatccctgggtgagtttcaccagttttgatttaaacgtggccaatatggacaacttcttcgcccccgttttcaccatgggcaaatattatacgcaaggcgacaaggtgctgatgccgctggcgattcaggttcatcatgccgtttgtgatggcttccatgtcggcagaatgcttaatgaattacaacagtactgcgatgagtggcagggcggggcg

SEQ ID NO: 136 - DNA, 718 bp, unidentified
  misc_feature 1..718: note = p15A Origin of replication
  source 1..718: mol_type = other DNA
ttaataagatgatcttcttgagatcgttttggtctgcgcgtaatctcttgctctgaaaacgaaaaaaccgccttgcagggcggtttttcgaaggttctctgagctaccaactctttgaaccgaggtaactggcttggaggagcgcagtcaccaaaacttgtcctttcagtttagccttaaccggcgcatgacttcaagactaactcctctaaatcaattaccagtggctgctgccagtggtgcttttgcatgtctttccgggttggactcaagacgatagttaccggataaggcgcagcggtcggactgaacggggggttcgtgcatacagtccagcttggagcgaactgcctacccggaactgagtgtcaggcgtggaatgagacaaacgcggccataacagcggaatgacaccggtaaaccgaaaggcaggaacaggagagcgcacgagggagccgccagggggaaacgcctggtatctttatagtcctgtcgggtttcgccaccactgatttgagcgtcagatttcgtgatgcttgtcaggggggcggagcctatggaaaaacggctttgccgcggccctctcacttccctgttaagtatcttcctggcatcttccaggaaatctccgccccgttcgtaagccatttccgctcgccgcagtcgaacgaccgagcgtagcgagtcagtgagcgaggaagcggaatatatccctagg

SEQ ID NO: 137 - DNA, 23 bp, unidentified
  misc_feature 1..23: note = rrnA, rrnB, rrnC, rrnD, rrnE, rrnG and rrnH target sequence
  source 1..23: mol_type = other DNA
taggtgaagtccctcgcggatgg

SEQ ID NO: 138 - DNA, 29 bp, Clostridium difficile R20291
  misc_feature 1..29: note = C. difficile Repeat 1
  source 1..29: mol_type = other DNA
gttttatattaactaagtggtatgtaaag

SEQ ID NO: 139 - DNA, 29 bp, Clostridium difficile R20291
  misc_feature 1..29: note = C. difficile Repeat 2
  source 1..29: mol_type = other DNA
gttttatattaactaagtggtatgtaaat

SEQ ID NO: 140 - DNA, 29 bp, Clostridium difficile R20291
  misc_feature 1..29: note = C. difficile Repeat 3
  source 1..29: mol_type = other DNA
gttttatattaactatatggaatgtaaat

SEQ ID NO: 141 - DNA, 29 bp, Clostridium difficile R20291
  misc_feature 1..29: note = C. difficile Repeat 4
  source 1..29: mol_type = other DNA
gttttagattaactatatggaatgtaaat

SEQ ID NO: 142 - DNA, 29 bp, Clostridium difficile R20291
  misc_feature 1..29: note = C. difficile Repeat 5
  source 1..29: mol_type = other DNA
gttttatattaactatatggaatgtaaat

SEQ ID NO: 143 - DNA, 29 bp, Clostridium difficile R20291
  misc_feature 1..29: note = C. difficile Repeat 6
  source 1..29: mol_type = other DNA
gttttatattaactatgtggtatgtaaat

SEQ ID NO: 144 - DNA, 29 bp, Clostridium difficile R20291
  misc_feature 1..29: note = C. difficile Repeat 7
  source 1..29: mol_type = other DNA
gttttatattaactatatggaatgtaaag

SEQ ID NO: 145 - DNA, 29 bp, Clostridium difficile R20291
  misc_feature 1..29: note = C. difficile Repeat 8
  source 1..29: mol_type = other DNA
gttttatattaactaagtggtatgtaaat

SEQ ID NO: 146 - DNA, 29 bp, Clostridium difficile R20291
  misc_feature 1..29: note = C. difficile Repeat 9
  source 1..29: mol_type = other DNA
gtttaaattacactaagttagttataaat

SEQ ID NO: 147 - DNA, 29 bp, Clostridium difficile 630
  misc_feature 1..29: note = C. difficile Repeat 10
  source 1..29: mol_type = other DNA
gttttagattaactatatggaatgtaaat

SEQ ID NO: 148 - DNA, 29 bp, Clostridium difficile 630
  misc_feature 1..29: note = C. difficile Repeat 11
  source 1..29: mol_type = other DNA
gttttagattaactatatggaatgtaaat

SEQ ID NO: 149 - DNA, 29 bp, Clostridium difficile 630
  misc_feature 1..29: note = C. difficile Repeat 12
  source 1..29: mol_type = other DNA
gttttatattaactaagtggtatgtaaag

SEQ ID NO: 150 - DNA, 29 bp, Clostridium difficile 630
  misc_feature 1..29: note = C. difficile Repeat 13
  source 1..29: mol_type = other DNA
gttttatattaactaagtggtatgtaaat

SEQ ID NO: 151 - DNA, 29 bp, Clostridium difficile 630
  misc_feature 1..29: note = C. difficile Repeat 14
  source 1..29: mol_type = other DNA
gttttatattaactatatggaatgtaaat

SEQ ID NO: 152 - DNA, 29 bp, Clostridium difficile 630
  misc_feature 1..29: note = C. difficile Repeat 15
  source 1..29: mol_type = other DNA
gttttatattaactatgtggtatgtaaat

SEQ ID NO: 153 - DNA, 29 bp, Clostridium difficile 630
  misc_feature 1..29: note = C. difficile Repeat 16
  source 1..29: mol_type = other DNA
gttttatatcaactatgtggtatgtaaag

SEQ ID NO: 154 - DNA, 29 bp, Clostridium difficile 630
  misc_feature 1..29: note = C. difficile Repeat 17
  source 1..29: mol_type = other DNA
gttttagattaactatatggaatgtaaat

SEQ ID NO: 155 - DNA, 29 bp, Clostridium difficile 630
  misc_feature 1..29: note = C. difficile Repeat 18
  source 1..29: mol_type = other DNA
gttttatattaactatatggaatgtaaat

SEQ ID NO: 156 - DNA, 29 bp, Clostridium difficile 630
  misc_feature 1..29: note = C. difficile Repeat 19
  source 1..29: mol_type = other DNA
gttttagattaactatatggaatgtaaat

SEQ ID NO: 157 - DNA, 29 bp, Clostridium difficile 630
  misc_feature 1..29: note = C. difficile Repeat 20
  source 1..29: mol_type = other DNA
gttttagattaactatatggaatgtaaat

SEQ ID NO: 158 - DNA, 29 bp, Clostridium difficile 630
  misc_feature 1..29: note = C. difficile Repeat 21
  source 1..29: mol_type = other DNA
gttttagattaactatatggaatgtaaat

SEQ ID NO: 159 - DNA, 29 bp, Clostridium difficile ATCC 45233
  misc_feature 1..29: note = C. difficile Repeat 22
  source 1..29: mol_type = other DNA
gttttatattaactaagtggtatgtaaag

SEQ ID NO: 160 - DNA, 29 bp, Clostridium difficile ATCC 45233
  misc_feature 1..29: note = C. difficile Repeat 23
  source 1..29: mol_type = other DNA
gttttatattaactaagtggtatgtaaat

SEQ ID NO: 161 - DNA, 29 bp, Clostridium difficile ATCC 45233
  misc_feature 1..29: note = C. difficile Repeat 24
  source 1..29: mol_type = other DNA
gttttatattaactatatggaatgtaaat

SEQ ID NO: 162 - DNA, 29 bp, Clostridium difficile ATCC 45233
  misc_feature 1..29: note = C. difficile Repeat 25
  source 1..29: mol_type = other DNA
gttttatattaactaagtggtatgtaaat

SEQ ID NO: 163 - DNA, 29 bp, Clostridium difficile ATCC 45233
  misc_feature 1..29: note = C. difficile Repeat 26
  source 1..29: mol_type = other DNA
gttttagattaactatatggaatgtaaaa

SEQ ID NO: 164 - DNA, 29 bp, Clostridium difficile ATCC 45233
  misc_feature 1..29: note = C. difficile Repeat 27
  source 1..29: mol_type = other DNA
gttttatattaactatatggaatgtaaat

SEQ ID NO: 165 - DNA, 29 bp, Clostridium difficile ATCC 45233
  misc_feature 1..29: note = C. difficile Repeat 28
  source 1..29: mol_type = other DNA
gttttatatcaactatgtggtatgtaaag

SEQ ID NO: 166 - DNA, 29 bp, Clostridium difficile ATCC 45233
  misc_feature 1..29: note = C. difficile Repeat 29
  source 1..29: mol_type = other DNA
gttttatattaactaagtggtatgtaaat

SEQ ID NO: 167 - DNA, 29 bp, Clostridium difficile BI9
  misc_feature 1..29: note = C. difficile Repeat 30
  source 1..29: mol_type = other DNA
gttttatattaactatgtggtatgtaaat

SEQ ID NO: 168 - DNA, 29 bp, Clostridium difficile BI9
  misc_feature 1..29: note = C. difficile Repeat 31
  source 1..29: mol_type = other DNA
gttttagattaactatatggaatgtaaat

SEQ ID NO: 169 - DNA, 29 bp, Clostridium difficile BI9
  misc_feature 1..29: note = C. difficile Repeat 32
  source 1..29: mol_type = other DNA
gttttagattaactatatggaatgtaaat

SEQ ID NO: 170 - DNA, 29 bp, Clostridium difficile BI9
  misc_feature 1..29: note = C. difficile Repeat 33
  source 1..29: mol_type = other DNA
gttttatattaactaagtggtatgtaaat

SEQ ID NO: 171 - DNA, 29 bp, Clostridium difficile BI9
  misc_feature 1..29: note = C. difficile Repeat 34
  source 1..29: mol_type = other DNA
gttttatattaactatatggaatgtaaat

SEQ ID NO: 172 - DNA, 29 bp, Clostridium difficile BI9
  misc_feature 1..29: note = C. difficile Repeat 35
  source 1..29: mol_type = other DNA
gttttatattaactaagtggtatgtaaat

SEQ ID NO: 173 - DNA, 29 bp, Clostridium difficile BI9
  misc_feature 1..29: note = C. difficile Repeat 36
  source 1..29: mol_type = other DNA
gttttagattaactatatggaatgtaaaa

SEQ ID NO: 174 - DNA, 29 bp, Clostridium difficile BI9
  misc_feature 1..29: note = C. difficile Repeat 37
  source 1..29: mol_type = other DNA
gttttatattaactatatggaatgtaaat

SEQ ID NO: 175 - DNA, 29 bp, Clostridium difficile BI9
  misc_feature 1..29: note = C. difficile Repeat 38
  source 1..29: mol_type = other DNA
gttttatattaactaagtggtatgtaaat

SEQ ID NO: 176 - DNA, 29 bp, Clostridium difficile M120
  misc_feature 1..29: note = C. difficile Repeat 39
  source 1..29: mol_type = other DNA
gttttatattaactaagtggtatgtaaag

SEQ ID NO: 177 - DNA, 29 bp, Clostridium difficile M120
  misc_feature 1..29: note = C. difficile Repeat 40
  source 1..29: mol_type = other DNA
gttttatattaactatgtggtatgtaaat

SEQ ID NO: 178 - DNA, 29 bp, Clostridium difficile M120
  misc_feature 1..29: note = C. difficile Repeat 41
  source 1..29: mol_type = other DNA
gttttatattaactatgtggtatgtaaag

SEQ ID NO: 179 - DNA, 29 bp, Clostridium difficile M120
  misc_feature 1..29: note = C. difficile Repeat 42
  source 1..29: mol_type = other DNA
gttttatattaactaagtggtatgtaaat

SEQ ID NO: 180 - DNA, 30 bp, Clostridium difficile M120
  misc_feature 1..30: note = C. difficile Repeat 43
  source 1..30: mol_type = other DNA
gttaaacagtaacatgagatgtatttaaat

SEQ ID NO: 181 - DNA, 29 bp, Clostridium difficile M120
  misc_feature 1..29: note = C. difficile Repeat 44
  source 1..29: mol_type = other DNA
gttttatattaactaagtggtatgtaaag

SEQ ID NO: 182 - DNA, 29 bp, Clostridium difficile CF5
  misc_feature 1..29: note = C. difficile Repeat 45
  source 1..29: mol_type = other DNA
gttttatattaactaagtggtatgtaaat

SEQ ID NO: 183 - DNA, 29 bp, Clostridium difficile CF5
  misc_feature 1..29: note = C. difficile Repeat 46
  source 1..29: mol_type = other DNA
gttttatattaactatatggaatgtaaat

SEQ ID NO: 184 - DNA, 29 bp, Clostridium difficile CF5
  misc_feature 1..29: note = C. difficile Repeat 47
  source 1..29: mol_type = other DNA
gttttagattaactatatggaatgtaaat

SEQ ID NO: 185 - DNA, 29 bp, Clostridium difficile CF5
  misc_feature 1..29: note = C. difficile Repeat 48
  source 1..29: mol_type = other DNA
gttttagattaactatatggaatgtaaat

SEQ ID NO: 186 - DNA, 29 bp, Clostridium difficile CF5
  misc_feature 1..29: note = C. difficile Repeat 49
  source 1..29: mol_type = other DNA
gttttatattaactatgtggtatgtaaat

SEQ ID NO: 187 - DNA, 29 bp, Clostridium difficile CF5
  misc_feature 1..29: note = C. difficile Repeat 50
  source 1..29: mol_type = other DNA
gttttatattaactatatggaatgtaaat

SEQ ID NO: 188 - DNA, 29 bp, Clostridium difficile CD002
  misc_feature 1..29: note = C. difficile Repeat 51
  source 1..29: mol_type = other DNA
gttttagattaactatatggaatgtaaat

SEQ ID NO: 189 - DNA, 29 bp, Clostridium difficile CD002
  misc_feature 1..29: note = C. difficile Repeat 52
  source 1..29: mol_type = other DNA
gttttatattaactaagtggtatgtaaat

SEQ ID NO: 190 - DNA, 29 bp, Clostridium difficile CD002
  misc_feature 1..29: note = C. difficile Repeat 53
  source 1..29: mol_type = other DNA
gttttatattaactatatggaatgtaaat

SEQ ID NO: 191 - DNA, 29 bp, Clostridium difficile CD002
  misc_feature 1..29: note = C. difficile Repeat 54
  source 1..29: mol_type = other DNA
gttttatattaactatgtggtatgtaaat

SEQ ID NO: 192 - DNA, 29 bp, Clostridium difficile CD002
  misc_feature 1..29: note = C. difficile Repeat 55
  source 1..29: mol_type = other DNA
gttttatattaactatatggaatgtaaat

SEQ ID NO: 193 - DNA, 29 bp, Clostridium difficile CD002
  misc_feature 1..29: note = C. difficile Repeat 56
  source 1..29: mol_type = other DNA
gttttatattaactaagtggtatgtaaag

SEQ ID NO: 194 - DNA, 29 bp, Clostridium difficile CD002
  misc_feature 1..29: note = C. difficile Repeat 57
  source 1..29: mol_type = other DNA
gtttaaattacactaagttagttataaat

SEQ ID NO: 195 - DNA, 29 bp, Clostridium difficile CD3
  misc_feature 1..29: note = C. difficile Repeat 58
  source 1..29: mol_type = other DNA
gttttagattaactatatggaatgtaaat

SEQ ID NO: 196 - DNA, 29 bp, Clostridium difficile CD3
  misc_feature 1..29: note = C. difficile Repeat 59
  source 1..29: mol_type = other DNA
gttttagattaactatatggaatgtaaat

SEQ ID NO: 197 - DNA, 29 bp, Clostridium difficile CD3
  misc_feature 1..29: note = C. difficile Repeat 60
  source 1..29: mol_type = other DNA
gttttatattaactaagtggtatgtaaat

SEQ ID NO: 198 - DNA, 29 bp, Clostridium difficile CD3
  misc_feature 1..29: note = C. difficile Repeat 61
  source 1..29: mol_type = other DNA
gttttatattaactatatggaatataaat

SEQ ID NO: 199 - DNA, 29 bp, Clostridium difficile CD3
  misc_feature 1..29: note = C. difficile Repeat 62
  source 1..29: mol_type = other DNA
gttttatattaactaagtggtatgtaaat

SEQ ID NO: 200 - DNA, 29 bp, Clostridium difficile CD3
  misc_feature 1..29: note = C. difficile Repeat 63
  source 1..29: mol_type = other DNA
gttttagattaactatatggaatgtaaat

SEQ ID NO: 201 - DNA, 29 bp, Clostridium difficile CD3
  misc_feature 1..29: note = C. difficile Repeat 64
  source 1..29: mol_type = other DNA
gttttatattaactatatggaatgtaaat

SEQ ID NO: 202 - DNA, 29 bp, Clostridium difficile CD69
  misc_feature 1..29: note = C. difficile Repeat 65
  source 1..29: mol_type = other DNA
gttttagattaactatatggaatgtaaat

SEQ ID NO: 203 - DNA, 29 bp, Clostridium difficile CD69
  misc_feature 1..29: note = C. difficile Repeat 66
  source 1..29: mol_type = other DNA
gttttatattaactatgtggtatgtaaag

SEQ ID NO: 204 - DNA, 29 bp, Clostridium difficile CD69
  misc_feature 1..29: note = C. difficile Repeat 67
  source 1..29: mol_type = other DNA
gttttatattaactatatggaatgtaaag

SEQ ID NO: 205 - DNA, 29 bp, Clostridium difficile CD69
  misc_feature 1..29: note = C. difficile Repeat 68
  source 1..29: mol_type = other DNA
gttttatattaactatgtggtatgtaaat

SEQ ID NO: 206 - DNA, 29 bp, Clostridium difficile CD69
  misc_feature 1..29: note = C. difficile Repeat 69
  source 1..29: mol_type = other DNA
gttttatattaactaagtggtatgtaaat

SEQ ID NO: 207 - DNA, 29 bp, Clostridium difficile CD69
  misc_feature 1..29: note = C. difficile Repeat 70
  source 1..29: mol_type = other DNA
gttttatattaactaagtggtatgtaaag

SEQ ID NO: 208 - DNA, 29 bp, Clostridium difficile CD69
  misc_feature 1..29: note = C. difficile Repeat 71
  source 1..29: mol_type = other DNA
gttttatattaactatatggaatgtaaat

SEQ ID NO: 209 - DNA, 29 bp, Clostridium difficile CD69
  misc_feature 1..29: note = C. difficile Repeat 72
  source 1..29: mol_type = other DNA
atttacattccatatagttaatctaaaac

SEQ ID NO: 210 - DNA, 29 bp, Escherichia coli K-12
  misc_feature 1..29: note = E.coli Repeat 1
  source 1..29: mol_type = other DNA
cggtttatccccgctggcgcggggaactc

SEQ ID NO: 211 - DNA, 28 bp, Escherichia coli K-12
  misc_feature 1..28: note = E.coli Repeat 2
  source 1..28: mol_type = other DNA
ggtttatccccgctggcgcggggaacac

SEQ ID NO: 212 - DNA, 27 bp, Escherichia coli K-12
  misc_feature 1..27: note = E.coli Repeat 3
  source 1..27: mol_type = other DNA
cggtttatccccgctggcgcggggaac

SEQ ID NO: 213 - DNA, 29 bp, Escherichia coli O157:H7
  misc_feature 1..29: note = E.coli Repeat 4
  source 1..29: mol_type = other DNA
cggtttatccccgctggcgcggggaacac

SEQ ID NO: 214 - DNA, 29 bp, Salmonella enterica subsp. enterica serovar Typhimurium
  misc_feature 1..29: note = Salmonella enterica subsp. enterica serovar Typhimurium Repeat Sequence
  source 1..29: mol_type = other DNA
cggtttatccccgctggcgcggggaacac

SEQ ID NO: 215 - DNA, 36 bp, Streptococcus thermophilus
  misc_feature 1..36: note = Streptococcus thermophilus Repeat 1
  source 1..36: mol_type = other DNA
gtttttgtactctcaagatttaagtaactgtacaac

SEQ ID NO: 216 - DNA, 36 bp, Streptococcus thermophilus
  misc_feature 1..36: note = Streptococcus thermophilus Repeat 2
  source 1..36: mol_type = other DNA
gatataaacctaattacctcgagaggggacggaaac

SEQ ID NO: 217 - DNA, 28 bp, Streptococcus thermophilus
  misc_feature 1..28: note = Streptococcus thermophilus Repeat 3
  source 1..28: mol_type = other DNA
ggatcacccccgcgtgtgcgggaaaaac

SEQ ID NO: 218 - DNA, 36 bp, Streptococcus thermophilus
  misc_feature 1..36: note = Streptococcus thermophilus Repeat 4
  source 1..36: mol_type = other DNA
gttttggaaccattcgaaacaacacagctctaaaac

SEQ ID NO: 219 - protein, 280 aa, Clostridium difficile
  REGION 1..280: note = C difficile Spo0A
MGGFLVEKIKIVLADDNKDFCQVLKEYLSNEDDIDILGIAKDGIEALDLVKKTQPDLLILDVIMPHLDGLGVIEKLNTMDIPKMPKIIVLSAVGQDKITQSAINLGADYYIVKPFDFVVFINRIRELVSNRVTQVEPKPRPVQETQMTRSDFVKNVGNIENVGNIETEITNIIHEIGVPAHIKGYLYLREAIKMVIDNVELLGAVTKELYPSIAKKFNTTPSRVERAIRHAIEVAWSRGKVDTINQLFGYTVHNTKGKPTNSEFIAMIADKLRLEHSMVK

SEQ ID NO: 220 - DNA, 861 bp, Clostridium difficile
  misc_feature 1..861: note = C difficile Spo0A
  source 1..861: mol_type = other DNA
ataagaagatgttttttaatggggggatttttagtggaaaaaatcaaaatagttttagcagatgacaataaggatttttgtcaggtattaaaagagtatttgtctaatgaagatgatatcgatatattaggcatagctaaggatggaattgaagcattagacttagtaaaaaagacacaaccggacttattaatactagatgtaataatgccacatctagatggattaggtgtaattgaaaaattgaatactatggatatacctaaaatgccaaaaataatagtactatcagcagtaggtcaagataagataactcaaagcgcaataaatctaggagcagattactacatagtaaagccatttgattttgttgtgtttataaacagaattagagagctagtttctaatagagttacacaagttgagccaaaacctagaccagttcaagagactcaaatgactagaagtgattttgttaagaatgtaggaaatatagagaatgtaggaaatatagagacagaaatcacaaatataatacatgaaataggagtaccagctcatataaaaggatatttatatttaagagaagcaataaaaatggttattgataatgttgagcttttaggtgcagtaacaaaagagttatatccaagtatagctaaaaaattcaatacaacaccaagtagagttgaaagagcaataagacatgcaatagaggttgcatggagtagaggaaaagttgacacaataaatcaattatttggatatacggtacacaatactaaaggaaaaccaactaattcagaatttatagcaatgattgctgataaattaagactagaacatagtatggttaaataa

SEQ ID NO: 221 - protein, 86 aa, Clostridium difficile
  REGION 1..86: note = C difficile spoIIID
MRSHIEERAIVVAKYILEKNTTVRQTAKTFGVSKSTIHKDVTERLKEINPSLAKEVKNVLDKNKSERHIRGGLATKLKYEKEHKKM

SEQ ID NO: 222 - DNA, 261 bp, Clostridium difficile
  misc_feature 1..261: note = C difficile spoIIID
  source 1..261: mol_type = other DNA
ttgagatctcatatagaggaaagggccatagtggtagcaaaatatatacttgaaaaaaacactacagtaagacaaaccgccaagacatttggagtaagtaaaagtacaattcataaggatgttacagaaagattgaaggaaataaatccatcccttgccaaagaagttaaaaatgtgctggacaaaaataaatcagagagacatattagagggggattagcaacgaaattaaaatatgagaaggaacataaaaaaatgtag

SEQ ID NO: 223 - protein, 219 aa, Clostridium difficile
  REGION 1..219: note = C difficile sigK
MAALKSFEKPLTPEEEIEYLTKFKIENDKSAKDTLIERNMRLVAYIAKKYNNSTEDQDDLISIGTIGLIKAIETYNIDKGTRLATYASRCIENEILMNIRSNKKNKTQVSLQDPIGTDKEGNEINTILYMSLLDILGTEANYVLDEVELKVQVGKLYEQLNKILTPREREIVQLRYGLTPYGYKTQREIAQKLDISRSYVSRIEKKALKKLEKELVQES

SEQ ID NO: 224 - DNA, 660 bp, Clostridium difficile
  misc_feature 1..660: note = C difficile sigK
  source 1..660: mol_type = other DNA
ttggcagctcttaaatcttttgaaaaacccttaacccctgaagaagagattgagtatttaactaaatttaaaatagaaaacgataaaagtgcaaaagatacattaattgaaagaaacatgagattagtagcttatatagcaaagaaatataataattcaacggaagatcaggatgatttaatatccataggtacaataggattaattaaagctatagaaacttataacatagataaaggaactcgattagcaacatatgcttctagatgtattgaaaatgagattttaatgaatattagatctaacaaaaaaaataaaactcaagtatctctacaagaccctatcggaacagataaagaaggtaatgaaataaacactattctttatatgagtcttttagatatacttggtacagaggctaactatgttcttgatgaagttgaactaaaagttcaagttggaaaactttacgaacaactaaacaaaattcttactcctagagaaagagaaattgtccagttaagatatgggttaactccttatggctataagacacaaagagaaattgcacaaaaactcgatatatcaaggtcatatgtatctagaatcgaaaaaaaagctcttaaaaaactagaaaaagagcttgttcaagaaagttaa

SEQ ID NO: 225 - protein, 254 aa, Clostridium difficile
  REGION 1..254: note = C difficile sigF
MEVTVAREEKKPLLSHEETLELIEKVQNGDEEAKEILISSNLGLVRSVVSRFLNIGYDREDLFQLGSIGLIKSIYKFDPKFNVKFSTYAVPMILGEIKRYLRDDGMIKVSRSLKQIAIKAKMESEALTKKLGREPSIEELAKAIDVEKEDLVMAMEANFNVEYLQGVIHEEEGSPICLIDKISMKGESEEEKVVDNILLKDILGRLDKRERQIIVLRYFEDMTQSEIGEMLNISQVQVSRIEKKVLSKLKEYIS

SEQ ID NO: 226 - DNA, 765 bp, Clostridium difficile
  misc_feature 1..765: note = C difficile sigF
  source 1..765: mol_type = other DNA
atggaagtaactgttgccagagaagaaaaaaaacctcttcttagtcatgaagagactctagaacttattgaaaaagttcaaaatggagatgaagaggcaaaagaaatattaatatcaagcaatttaggtctagttaggagcgttgtatctagatttttaaatataggatatgatagagaagatttatttcagttaggttctataggcttaataaaatcaatatataaatttgacccaaaatttaatgtaaaattctctacttatgcagtaccaatgattttaggtgaaataaagagatacttaagagatgatggtatgataaaagtatcaaggtcgttaaagcaaatagctataaaggcaaagatggaaagtgaagctttaactaaaaaattaggtagagagccgagtatagaagaattagctaaagcaatagatgtagaaaaagaagatttagtaatggctatggaagctaatttcaatgttgagtatttgcaaggagttattcatgaagaggaaggttctccaatatgccttattgataaaataagcatgaaaggagaaagtgaagaagaaaaagtagtggataacatattgttaaaagacatacttggaagactggataagagagagcgtcaaataatagttctcagatactttgaagacatgactcaaagtgaaataggagagatgctcaatatatcacaagttcaagtatctaggatagagaagaaagtattgtctaagttaaaagaatatatatcgtga

SEQ ID NO: 227 - protein, 220 aa, Clostridium difficile
  REGION 1..220: note = C difficile sigH
MGEIYMLVAKEKSYELVDNCQQDEYNIVLRASEGDKIALEYIITKYRNFVKAKAKSYFLIGADKEDIIQEGMIGLYKAVRDFDGSKTNSFKCFAEICITRQIITAIKTATRQKHIPLNSYVSLNKPIYDEESDRTLLDIIATSIVTDPEELIISKEELKNIESKMNELLSDLELEVLELYLNGKSYQFIADKLKRDVKSIDNALQRVKRKLEKHLENRND

SEQ ID NO: 228 - DNA, 663 bp, Clostridium difficile
  misc_feature 1..663: note = C difficile sigH
  source 1..663: mol_type = other DNA
atgggggagatttacatgttggtagcaaaagaaaaaagttatgagttagtggacaattgtcagcaggatgagtataacattgtattaagagcaagtgaaggggataaaatagcactagagtacattattactaaatacagaaattttgtaaaggcaaaagcaaagtcatattttttaattggagcagataaagaagatataatacaagaaggaatgataggcctttataaggcagttagagattttgatggaagtaagaccaattcatttaaatgttttgcggagatatgtataacaagacaaataataactgctataaaaactgcaacaagacaaaaacatatacctttaaattcatatgtttctttgaataaaccaatatatgatgaagagtcagacagaacacttttagatattatagctacaagtatagtaacagatccagaagagcttataattagtaaagaagagttgaaaaatatagaatcaaaaatgaacgaattgttaagtgacttggaattagaagtactagaattatatttaaatggaaagtcataccagtttatagcggacaagcttaaaagagatgtaaagtcaatagataacgctttacaaagggttaagagaaaattagaaaaacatcttgaaaacagaaatgattaa

SEQ ID NO: 229 - DNA, 258 bp, Bacillus subtilis
  misc_feature 1..258: note = Bacillus subtilis Spo0A-P phosphatase
  source 1..258: mol_type = other DNA
atgggcggttcttctgaacaagaaagattgttggtgtctattgatgaaaaaagaaagttaatgatagatgccgctagaaagcagggatttacagggcatgacacgatcaggcacagtcaggagctggattgtttaataaatgaatatcatcagcttatgcaagaaaacgaacattcccaagggattcaaggccttgtaaagaaattaggcttgtggccccgcagagatgttatgccagcatatgatgcaaataaatag

SEQ ID NO: 230 - protein, 85 aa, Bacillus subtilis
  REGION 1..85: note = Bacillus subtilis Spo0A-P phosphatase
MGGSSEQERLLVSIDEKRKLMIDAARKQGFTGHDTIRHSQELDCLINEYHQLMQENEHSQGIQGLVKKLGLWPRRDVMPAYDANK

SEQ ID NO: 231 - protein, 790 aa, Clostridium difficile
  REGION 1..790: note = C difficile spoIIE
MQRSVAVVKNKTVKPNVIKLISGYIDFTTAAFAVMGFLLSRSIIVDSVAPLGIAFFICASKIDKYKIPVFISTLLGILLSSNDFGNVAKYAVCLTIFMAMNKKLKLSDSIAKVAFIGAIILLPISMGQAFFSNRYVYGLLIAGVEAIIMFISIYVFSYGIGLMANVNNRMSVRTEEAISISLLLTFSIMGIGDISLFGISIRTILSTVLILLTSIVGGATMGASSGVIIGVASILNNMTSAVYMGIYSFSGLISGAFNKINKYFCILGYILSWTIIYLYTSGITSNMMQLRDILLGCLIVLVLPERLFNKIEKLIKSNVASNEIVYDYIMRSKNLTNSRLNSIYKTYDDLADTFDKIREKDKVLDQRDIANVIDMIHNDECKSCSMRRMCWESRFNHTYTMIYNILEKIEEKGELSLNDIPKNFRKECMKPESIVKISNHYYKMFVLDYDWSVKFSESRKLIANQIRSISKSIKSLSQDLEGDIMLDIEKEKNIYEQLERYDITVDKVSYLTKSNSEFEISIEKKTCHDGCMCEDKIVNIISDLVGENMSVRKIGCHCLGGKCKATFVKSQKYKAVTEVSAMSRDGHILCGDNYTYMEINDGKYMMAISDGMGKGKKAYEESSATIDILEKMIDAKIKDEIVIDTINNMLLLKSSEEMFSTLDLGILDLKRGCLETIKMGACSTYIKREDGEVDLISSSSLPVGILSDVKIDRKNVKVKEGDYVIMVSDGIVDAGRNNNLGDNWLIYFLKNIETTNPKEISNLILDRALELQALQIEDDMTVLVTKICTK

SEQ ID NO: 232 - DNA, 2373 bp, Clostridium difficile
  misc_feature 1..2373: note = C difficile spoIIE
  source 1..2373: mol_type = other DNA
atgcaaagaagtgtagcagttgtgaagaataagactgtaaaaccaaatgtcataaaattaataagcggatatattgattttactacggcggcattcgctgtgatgggatttttacttagtaggtctattatagtagactctgtagctcctttaggaattgccttttttatatgtgcatcaaagattgataagtacaagatacctgtattcatatcaacattattaggaatattgttatcatctaatgattttggaaatgtagcaaaatatgctgtgtgccttacaatatttatggctatgaataaaaaattaaaattatcagattcaattgctaaggttgcatttataggtgcaataatactacttccaatctccatgggacaagctttcttttcaaataggtatgtatatggtcttcttatagcaggagtagaagcaataataatgtttatatctatatatgtgttttcttatgggataggtttaatggccaatgtcaacaataggatgtctgtacggacagaagaagccatatcaataagtttactgctaacctttagcataatgggaataggagatatatctctgtttggaatatcaataaggaccattttatcgaccgtattgatattgctgacctcaatagtaggtggagctaccatgggagcatctagtggtgtaattattggtgtagcatccattttaaataatatgacatcagctgtttatatggggatatattctttttcaggattaataagtggagcatttaataaaataaataaatatttctgtatactaggatatattctaagttggacaataatatacctatatacttctggtattacttctaatatgatgcaattaagagatatactattaggttgtttgatagtactagtattgccagagcgattatttaataagattgaaaaattaataaaaagtaatgtggcttcaaatgaaatcgtatacgattatattatgagaagcaaaaacctaactaatagcagattgaacagtatttataaaacttatgatgaccttgcagatacatttgataagataagagaaaaagacaaagtgctagaccaaagagacatagctaatgtaatagatatgattcataatgatgaatgtaaaagttgtagtatgagaagaatgtgctgggagtcaagatttaatcatacatacactatgatatataacattcttgaaaaaattgaggagaaaggggagttaagtctaaacgatatacctaaaaattttagaaaggaatgtatgaaaccagagtcaatagtgaaaatatcaaatcactattacaaaatgtttgtattagattatgattggagtgtgaagttttcagaaagtagaaagttaatagcaaatcagataagaagtatttcaaaatccattaaatccttatctcaagatttagaaggcgacataatgctagatatagaaaaggaaaaaaatatatatgaacagttagaaagatatgatataacagttgataaagtaagttacttaacaaaaagtaacagtgagtttgaaatatcaatagaaaagaaaacttgccatgatggatgtatgtgtgaagataaaattgtaaatataatttcagacctagtaggtgaaaatatgtctgttagaaaaataggatgtcactgtttaggaggtaaatgcaaggcaacattcgttaaatctcaaaaatataaggctgttacagaagtttcagcaatgtcaagggatgggcatatcctttgtggagacaattacacatacatggagataaatgatggtaaatacatgatggctataagtgatggtatgggaaaaggtaaaaaagcatatgaagaatcttctgccactattgatatactggaaaaaatgatagatgcaaaaattaaagatgagatagtcattgatactataaataatatgttgttgttaaaatcttcagaagagatgttttcaactctggatttgggaattttagatttaaaacgaggttgtttagaaactataaagatgggagcgtgttctacttatataaaaagagaggatggagaagttgacttaatatcatcatcatcattacctgtgggtatattatcagatgtaaaaattgatagaaaaaatgtaaaagttaaggaaggagactatgttataatggtttctgatggaattgtagatgcaggaagaaataacaatttaggagacaattggttaatatacttcttaaagaatatagagactacaaatccaaaggaaatttcaaatttaatattggatagagcattagagttacaagcgttacaaatcgaagatgacatgactgttttagttacgaaaatatgtacaaaataa

SEQ ID NO: 233 - protein, 117 aa, Bacillus subtilis
  REGION 1..117: note = Bacillus subtilis spoIIAA
MSLGIDMNVKESVLCIRLTGELDHHTAETLKQKVTQSLEKDDIRHIVLNLEDLSFMDSSGLGVILGRYKQIKQIGGEMVVCAISPAVKRLFDMSGLFKIIRFEQSEQQALLTLGVAS

SEQ ID NO: 234 - DNA, 354 bp, Bacillus subtilis
  misc_feature 1..354: note = Bacillus subtilis spoIIAA
  source 1..354: mol_type = other DNA
atgagccttggaattgacatgaatgtcaaagaatctgtgctttgtattcgattaacaggcgaactcgatcaccatacggctgaaaccctgaagcaaaaagtgactcaatcattggagaaggatgatattcgccatatcgtgctgaacttggaggacctttcctttatggacagctcggggcttggcgttattttaggaagatacaagcaaattaagcaaattggcggagaaatggttgtttgcgctatctctcctgcggtgaagcgattgtttgatatgtcgggtctgtttaaaattatccgatttgaacaatctgaacagcaggcactcctgacactgggggtggcatcatga

SEQ ID NO: 235 - protein, 142 aa, Clostridium difficile
  REGION 1..142: note = C difficile spoIIAB
MNNIMEVKFSAISENESLARVIVASFAAKLDPTVDELVDIKTAVSEAVTNAIIHGYEEDSSKFVFLRCEIEGNTIKIIVEDEGYGIENVEKAMEPLYTSKPELDRSGMGFTVMKSFMDDVEVSSVKDNGTRIEMTKKINVPK

SEQ ID NO: 236 - DNA, 429 bp, Clostridium difficile
  misc_feature 1..429: note = C difficile spoIIAB
  source 1..429: mol_type = other DNA
atgaataatattatggaagttaaattttcggcaatatctgaaaatgaaagtttagcaagagttatagtagcatcctttgcagctaagttagacccaacagtagatgagttagtagatataaaaactgctgtctctgaggctgttacgaatgctataatacatggatatgaagaagacagttctaagtttgttttcttaagatgtgagatagaaggaaatactataaagattatagttgaagatgaagggtatggaatagaaaatgtggagaaggcaatggaaccactttatacatcaaaaccagaacttgatagatcaggaatgggattcacagtaatgaaaagctttatggacgatgtagaggtaagttctgtaaaagataatgggactagaattgaaatgactaaaaaaataaatgtgcctaaataa

SEQ ID NO: 237 - protein, 281 aa, Clostridium difficile
  REGION 1..281: note = C difficile spoIIGA
MVYIEYYVIENLVINYIIISCTSILTKRYNPKKNKLLGASLGGAYSVAYLYPSMNILFTVPFKIIIMSIITLISFRSKSKKDYVHVALVFYLVNIFISGSTYFIIYFTGISHLKISFLIACTYVSCELLKYIYKDLKMLKYIKELTKTININLLEKSFCCKALVDSGNLLKDPISQSDVIIVKSSVLEGFIPEKLLNINYEDINMKKAQEIIGSLDDKTSGRVRIIPYKHAGSNKTSIIIGLKADYIEVDEQKIGNIILGISNFNDREYGAIMNPNILPGF

SEQ ID NO: 238 - DNA, 846 bp, Clostridium difficile
  misc_feature 1..846: note = C difficile spoIIGA
  source 1..846: mol_type = other DNA
atggtgtatattgagtactatgttatagaaaacctagtaataaattatattattataagttgtacttctattcttactaaaagatataatcctaaaaaaaataagttattgggggctagtttaggaggtgcctattctgttgcttatttgtatccatcaatgaatatactatttactgtaccatttaaaataataatcatgagtataataactttaatttcatttagaagtaagagcaaaaaagattatgttcatgtagcgttagttttttatctagtaaacatttttatttctggaagcacttattttataatttattttacaggaataagtcacttaaaaatatctttcttaattgcatgtacttatgtgagttgtgaattattaaaatacatttataaagatttgaaaatgcttaagtacattaaggagcttacaaagactataaatataaacttactagaaaaaagtttttgctgtaaagctttagtagatagtggtaatttgttaaaagacccaataagtcaaagtgatgtaataatagttaagtctagtgtgttagaaggatttattccagaaaaactattaaatattaattatgaagatataaatatgaagaaagcacaagaaattataggaagtttagatgataaaacttcaggtagagttagaataataccttataaacatgctggaagtaataagacaagcataataataggcttaaaagctgactatatagaagtagatgagcaaaagataggaaatataatacttggtatttcaaattttaatgatagagaatatggagcaataatgaatccaaatatattgcctggattttag

SEQ ID NO: 239 - protein, 240 aa, Clostridium difficile
  REGION 1..240: note = C difficile sigE
MLRLKERIISFITMLGIKLKIIKPKGIYYMGGANILPPPLKPEEEMELLQKLETDESVKSILIERNLRLVVYISRKFENTGIDVEDLISIGTIGLIKAVNTFKLNKNIKLATYASRCIENEILMYLRKNNKKKTEVSFDEPLNIDLDGNELLLSDVLGTENDEIYKIIEEEIDRDLLVMALDRLSDREKQIMELRFGLIDKGIEKTQKEVAGMLGISQSYISRLEKKIISRLQKEMKKFV

SEQ ID NO: 240 - DNA, 723 bp, Clostridium difficile
  misc_feature 1..723: note = C difficile sigE
  source 1..723: mol_type = other DNA
atgttacgattgaaagaaagaataataagctttattactatgttaggtattaaattaaaaataataaagccaaagggaatatactatatgggaggggcaaatatacttcctcctccattgaaaccagaagaagaaatggagcttttacaaaagctagaaacagatgaaagtgtaaagtcaattttaatagaaagaaatcttagattagtagtctacatatcgagaaaatttgaaaatacaggtatagatgtagaagatttgatttcaataggaactataggtttgataaaagcagttaatacttttaaactgaataaaaatataaaattggcaacttatgcttcgagatgtatagaaaatgaaatattaatgtacttaagaaaaaataataaaaagaaaacagaagtatcatttgatgaacctttaaatatagatttagatggaaacgaacttttattatctgatgtattgggtacagaaaatgatgaaatatacaaaataattgaagaagaaatagatagagatttgttggttatggcacttgacagattaagtgacagagaaaagcaaattatggaattaagatttggtcttattgataaaggtattgaaaaaacacaaaaagaagttgctggaatgcttggaatatcacagtcctacatatctagacttgaaaagaaaataatctcaaggttgcaaaaagaaatgaaaaaatttgtataa

SEQ ID NO: 241 - protein, 219 aa, Clostridium difficile
  REGION 1..219: note = C difficile spoIIR
MRKIKIRLGLLILSLISVISIMTIVINGEVKKVDNISKDYKDKLIRFHVIANSNTDEDQELKLKVRDEVIKYLQPKLQNSKSIKESEAIIKKEYSSLEEISKNIILKNGYNYSVKVGIQYSNFPTKQYSNIVLPAGEYKALKIIIGKGEGKNWWCVMFPPLCFVDESNGVIDKSTDDKLKEVLTDKEYKLIKQDTPKKTSRVKIKFKVLEVVKDLEKKF

SEQ ID NO: 242 - DNA, 660 bp, Clostridium difficile
  misc_feature 1..660: note = C difficile spoIIR
  source 1..660: mol_type = other DNA
atgagaaaaattaagattagattgggactattaatattaagtcttatatcagtcatatcaataatgacaatagtaataaatggtgaggtaaaaaaagtagacaatatatcaaaagattataaagataaattaataagatttcatgttatagcaaacagcaatacagatgaagaccaagaacttaaactaaaagttagagatgaagtaataaaatatttacagccaaagcttcaaaattcaaaaagtataaaagaaagtgaagctattataaaaaaggaatatagtagtctggaagaaataagtaaaaatattattcttaaaaatggatataattacagtgtaaaggtaggtatacaatatagcaatttccctactaaacaatattctaatatagttcttccagctggtgaatataaagcattaaagattattattgggaaaggtgaaggaaaaaactggtggtgtgttatgttccctccactatgttttgttgatgaatctaatggagtgatagataaatctacagatgataagttgaaggaagttttaactgataaagaatataagttaataaaacaagatacaccaaaaaaaacaagtagagtaaaaattaagtttaaagtacttgaagtagtcaaggatttagagaaaaaattttaa

SEQ ID NO: 243 - protein, 257 aa, Clostridium difficile
  REGION 1..257: note = C difficile sigG
MQVNKVEICGVNTSELPVLKNKQMKELLLQIKNGDEEARQQFVRGNLRLVLSVIKKFNNRGENIDDLFQIGCIGLIKAIDNFDLSQNVRFSTYAVPMIIGEIRRYLRDNNPIRVSRSLKDIAYKALQVRERLIRTNSKEPTVSEIAKELELEVESVVMALDAIQDPISLFDPVYQDNGDAIFVMDQVQDKKDTDENWLQEISLKEAIKKLNSREKLVLDLRFYKGRTQIEVADEIGISQAQVSRIEKNALKNMRKYV

SEQ ID NO: 244 - DNA, 774 bp, Clostridium difficile
  misc_feature 1..774: note = C difficile sigG
  source 1..774: mol_type = other DNA
atgcaagttaataaggttgaaatatgtggtgttaatacatcagaacttccagttcttaaaaataagcaaatgaaggaacttttattacaaataaaaaatggtgatgaagaagccagacaacagtttgtaagagggaatttaagattagtcttgagtgtaataaaaaagtttaacaacagaggagaaaatatagacgatttatttcaaataggttgtattggtcttataaaagcgatagataactttgatttaagccaaaatgtaaggttttcaacttatgctgttcctatgattataggagaaattagaaggtatctaagagacaataacccaattagagtaagtaggtcattaaaagatatagcatataaggcactacaagttagagaaagattaattagaacaaattctaaagaacctacagtatcagaaatagcaaaggaattagaattagaagtagaatcagttgtaatggcacttgatgccatacaagacccaatatctctgtttgacccagtatatcaagacaatggagatgcaatattcgttatggatcaggttcaagataaaaaagatactgatgaaaattggttgcaagaaatatcacttaaagaagctattaagaaattaaatagtagagaaaagttggtattagatttaaggttttacaaaggaagaactcagatagaagttgctgatgaaatcggtatatctcaagcacaagtatcaagaattgaaaaaaatgctttaaaaaatatgagaaaatatgtataa

SEQ ID NO: 245 - protein, 218 aa, Bacillus subtilis
  REGION 1..218: note = B subtilis SpoIIIA
MLKKQTVWLLTMLSLVVVLSVYYIMSPESKNAVQMQSEKSASDSGEVATEKAPAKQDTKEKSGTETEKGKEDGTKGTKDSSADKETSAEASEKGTVVTETADDDLFTTYRLDLEDARSKEREELNAIVSSDDATAKEKSEAYDKMTALSEVEGTEKQLETLIKTQGYEDALVNAEGDKINITVKSDKHSKSKATAIIDLVAKEIKTMKDVAVTFEPSK

SEQ ID NO: 246 - DNA, 657 bp, Bacillus subtilis
  misc_feature 1..657: note = B subtilis SpoIIIA
  source 1..657: mol_type = other DNA
atgcttaaaaaacaaaccgtttggctattaacaatgctcagtcttgtcgtggtgttaagcgtctactatatcatgtcgccggaaagcaaaaacgccgtgcagatgcaaagtgaaaaaagcgcgtctgacagcggagaggtcgcaactgaaaaagcgcctgccaagcaagacacgaaggaaaaaagcggtacagaaactgaaaaaggaaaagaagatggaacaaagggaacgaaagattcatcagcagacaaggaaacatccgctgaagccagtgaaaaaggaactgttgttacggaaacagccgatgatgatttgtttacaacgtaccgtcttgatttagaagatgccagaagcaaagaaagagaagagctgaatgccattgtgtcaagcgatgatgcaacagccaaggagaaaagcgaagcatacgataaaatgacggctctcagtgaagtggaaggaacagaaaaacagctggaaacgctgattaaaacacaaggttacgaggatgcgcttgttaatgctgaaggagataaaatcaatattacagtcaaatcagacaaacactctaaatcgaaggcgacagccattatagaccttgtggcaaaagaaatcaaaacaatgaaagatgtcgctgtcacatttgaaccctctaaataa

SEQ ID NO: 247 - protein, 354 aa, Clostridium difficile
  REGION 1..354: note = C dificile spoIID
MKNPLVVLLGFVTCSVLVPSLITLVSYKNVELTEKPESPVSINKTIKKSDIEDKGNKEEKNTVNYETVNKKAPIINVYNHITGKTEKMDMENYLCGVLAGEMSSEFDIEALKAQSVAARTYVVYKQEHGKSSKHKNAVVCTDYKHCQEYKSYDTLKKLNGEEWIKNKYSKIQEAVRGTKGQIITYNDKAILPLYFSTSSGKTENSEEVFSAKYPYLKSVESPYDKYSPKFASTLKISNTDFVKSLRRAYSTIVIDVNNLSKQVSITKRSDAGTVEKIKLGNKELTGKDIRTVFKLNSANFDIKFGEGYIDFVVKGYGHGVGMSQWGAEGMAEEGYKYYDILSHYYTDTKIKDIY

SEQ ID NO: 248 - DNA, 1065 bp, Clostridium difficile
  misc_feature 1..1065: note = C dificile spoIID
  source 1..1065: mol_type = other DNA
atgaagaacccattggttgttttgttaggatttgtgacttgctctgtgttagttccatcacttataactttagtttcttataaaaatgtagaattaactgaaaaaccagagagcccagtatctataaacaaaactattaaaaaaagtgatattgaagacaaaggtaataaagaagaaaaaaatacagtgaactatgaaactgtaaataaaaaagcaccaattatcaatgtatataatcatataacagggaaaaccgaaaagatggacatggagaactatttatgtggagtactagctggtgagatgtcttcagagtttgatatagaagctttaaaagctcaatctgtagcagctagaacatatgtagtatataaacaagaacatggtaaatctagtaaacataaaaatgcagtagtatgtactgattataaacattgtcaagaatataagagttatgatactcttaaaaaattaaatggtgaagaatggattaagaataaatattccaaaatccaagaagcagttagaggaactaaaggtcaaataataacttataatgataaggcgatacttcctctttatttttctacatcttcaggaaaaacagaaaatagtgaagaagtattttctgcaaaatatccttatttaaagtctgtggaaagtccttatgataagtattcccctaaatttgcgtcaacacttaaaataagtaacacagattttgttaaaagtcttagaagggcatatagcactattgtgatagatgtgaataatttaagtaaacaagtttcaataactaaaagaagtgatgccggaactgtagaaaaaataaaattaggaaataaagaattgactggaaaagacattagaactgtttttaaattgaactctgcaaactttgacataaaatttggagaaggatacatagatttcgtggtaaaaggatatggtcatggtgttggtatgagccagtggggagcagaaggaatggcagaagagggctataaatattatgatatattatcacattactacacagatacaaaaataaaagatatatactaa

SEQ ID NO: 249 - protein, 283 aa, Bacillus subtilis
  REGION 1..283: note = B subtilis SpoIIQ
MREEEKKTSQVKKLQQFFRKRWVFPAIYLVSAAVILTAVLWYQSVSNDEVKDQLADNGGNSAYDNNDDAVEVGKSMENVAMPVVDSENVSVVKKFYETDAAKEEKEAALVTYNNTYSLSKGIDLAEKDGKDFDVSASLSGTVVKAEKDPVLGYVVEVEHADGLSTVYQSLSEVSVEQGDKVKQNQVIGKSGKNLYSEDSGNHVHFEIRKDGVAMNPLNFMDKPVSSIEKAATQETEESIQQSSEKKDGSTEKGTEEKSGEKKDDSTDKSGSKESSTTEDTEQS

SEQ ID NO: 250 - DNA, 852 bp, Bacillus subtilis
  misc_feature 1..852: note = B subtilis SpoIIQ
  source 1..852: mol_type = other DNA
atgagagaggaagaaaagaaaacttctcaagtcaaaaaacttcagcagttttttcgtaaacgctgggtgttccctgcaatttacttagtcagtgcggccgtcattttaacagctgtcctttggtatcaatcagtatcaaatgatgaggtaaaggatcagttggctgataacggcggaaactccgcatatgacaacaacgacgatgcagttgaagtaggaaagtcaatggaaaatgtcgcaatgccggttgttgattctgaaaacgtttctgttgtgaaaaagttctatgaaaccgatgccgcaaaagaagagaaagaagcagcactcgttacctataataacacgtacagcctaagcaaaggaattgacttagctgagaaagacggaaaagatttcgatgtctctgcttctctgagcggtacggttgttaaagctgaaaaagatccagtgctgggatatgttgtggaagtagaacatgccgacggtttatcgactgtgtatcaatctctttccgaagtaagcgtagagcaaggtgacaaagtaaaacaaaatcaagtgatcggaaaatctggcaagaacctttacagtgaagacagcggaaaccacgtgcactttgaaatccgtaaagatggggttgcaatgaatccgttaaactttatggacaaaccagtttcttctattgaaaaagctgccacccaagaaacagaagaatccattcagcaatcttccgagaaaaaggacggatcaactgaaaaaggaacagaagaaaaatccggtgagaaaaaggatgattcaactgacaaatctggttctaaagaaagcagcacaacagaagacactgaacagtcttaa

SEQ ID NO: 251 - protein, 335 aa, Clostridium difficile
  REGION 1..335: note = C difficile SpoIVB
MQLKNFHFKNNTLSKKTNLAKSKFTIVLTFLFLLYFFSNNLIYAQNLQKNEPEYLIPIGNVLQIDAELKNIIVRNPGEASPFRLGDAIVKVNNAEVDGYSDFANTLNALPEEKQVSILLNRGGQLITMKTTKHILEKISFNNLLSGFATLTYINPDTSEFGAVGHPISVGNARKIPIKTGSISTTKHLNIEKSYKGSVGCINAKRENIIGSFTENTDFGIRGQINNFDISKLKKYKVASLDEVKLGKAQIILQDNFNKCKKYNIEIIDIENQKHPESKSFKIKITDKKLLAQTGGIVQGMSGTPIVQDNKIIGAVSHAIENDPAVGYGVFIKWML

SEQ ID NO: 252 - DNA, 1008 bp, Clostridium difficile
  misc_feature 1..1008: note = C difficile SpoIVB
  source 1..1008: mol_type = other DNA
atgcaacttaaaaattttcattttaaaaataatactttaagtaaaaaaaccaacttagctaagtcaaaatttacaattgttttaacatttttatttttattatattttttctcaaataatttaatttatgcacaaaatttacaaaaaaatgaacctgaatatttaataccaattggaaacgtacttcaaattgacgcagaattaaaaaatatcatagttagaaatcctggagaagcatctccatttagattgggtgatgctatagtaaaggtaaataatgctgaagttgatggatatagtgactttgccaataccttaaatgctttaccagaagaaaaacaagtatctattttattaaatagaggtggacaacttataacaatgaaaactaccaaacacatattagaaaaaattagttttaacaatttactttctggatttgctactttaacgtatatcaatccagatacatcagagtttggagctgtaggtcatccaataagtgttggtaatgcaagaaaaatacctattaaaacaggttcaatttctacaactaagcaccttaatatagaaaaatcttataaaggtagtgttggatgtataaatgcaaaacgagaaaatattattggtagctttacagaaaatactgattttggaataagaggtcaaattaataactttgatatttccaagttaaaaaaatataaagtagcatctttagatgaagttaaattaggaaaagctcaaataattttacaagataactttaataagtgtaaaaaatataatattgaaattatagatatagaaaaccaaaaacatccagaaagtaaaagttttaaaattaaaattacagataaaaagcttttagctcaaactggtggtattgtacaaggtatgagtggtactccaatagttcaagataataaaataatcggagcagtgtcacatgcaattgaaaacgacccagctgtaggttatggtgtatttattaaatggatgttgtaa

SEQ ID NO: 253 - protein, 480 aa, Bacillus subtilis
  REGION 1..480: note = B subtilis CtpB
MNQKIMAVIAAGSMLFGGAGVYAGINLLEMDKPQTAAVPATAQADSERDKAMDKIEKAYELISNEYVEKVDREKLLEGAIQGMLSTLNDPYSVYMDKQTAKQFSDSLDSSFEGIGAEVGMEDGKIIIVSPFKKSPAEKAGLKPNDEIISINGESMAGKDLNHAVLKIRGKKGSSVSMKIQRPGTKKQLSFRIKRAEIPLETVFASEKKVQGHSVGYIAISTFSEHTAEDFAKALRELEKKEIEGLVIDVRGNPGGYLQSVEEILKHFVTKDQPYIQIAERNGDKKRYFSTLTHKKAYPVNVITDKGSASASEILAGALKEAGHYDVVGDTSFGKGTVQQAVPMGDGSNIKLTLYKWLTPNGNWIHKKGIEPTIAIKQPDYFSAGPLQLKEPLKVDMNNEDVKHAQVLLKGLSFDPGREDGYFSKDMKKAVMAFQDQNKLNKTGVIDTRTAETLNQQIEKKKSDEKNDLQLQTALKSLFVN

SEQ ID NO: 254 - DNA, 1443 bp, Bacillus subtilis
  misc_feature 1..1443: note = B subtilis CtpB
  source 1..1443: mol_type = other DNA
atgaatcaaaaaataatggctgtgatagcagcagggagcatgctgttcggaggcgccggtgtatatgcgggaatcaacctgcttgagatggataagccccagactgcagcagttcccgcgacggcacaagctgactctgaacgggataaagctatggacaaaatcgaaaaagcgtatgagttaatttcgaatgagtacgtagaaaaagtagatagagaaaagctgctcgagggagccatccagggaatgctgtctacgctaaatgatccttattctgtttacatggacaagcagacagctaagcaattttctgattctcttgattcctcatttgaaggcatcggggctgaggttggaatggaagacggcaaaattattattgtttctccattcaagaaatcgccagcggaaaaagccgggttgaagcctaatgatgaaattatcagcatcaatggagaatcgatggccggcaaggatttaaaccacgctgtgttaaaaataagaggaaaaaaagggtccagcgtttcaatgaagattcagcggcctggaacgaagaagcagttgtcattccggatcaagagagctgagattccgctcgaaacggtttttgcatcagagaaaaaagtacaggggcattctgtcggatatattgccatctctactttttctgagcacaccgcagaggattttgcaaaagcgctgagggagcttgagaaaaaagaaatagaaggacttgtcattgatgtacgcggcaacccgggtggatatcttcaaagtgtggaagaaattcttaagcatttcgttacaaaggatcagccgtatattcagattgctgaacgcaatggagataaaaaacgttatttttcaacattgacccataaaaaagcgtaccctgtcaatgtgattacggataaaggaagtgcctctgcatcagaaattcttgccggcgcattaaaggaagctggccattatgatgttgtaggcgatacgtcttttggaaagggaacggttcaacaggctgtgccaatgggggacggcagcaacatcaaattaacgctttacaagtggctgacgccaaatggaaactggattcataagaaaggaattgaaccgaccattgcgattaagcagcccgattatttttccgccgggcccttacagctgaaagagccgcttaaagtggacatgaacaatgaagacgtcaagcatgcgcaggtattgttaaaaggtctcagctttgatccgggacgtgaggatggctatttcagcaaagacatgaaaaaagcggttatggcttttcaggatcaaaacaagctgaataaaaccggtgtgatcgacactcgcactgcagagacattaaatcagcagatagaaaagaaaaaatcagatgaaaaaaatgatttgcagcttcaaacagcattgaaatcattatttgtcaattaa

SEQ ID NO: 255 - protein, 2710 aa, Clostridium difficile
  REGION 1..2710: note = C difficile Toxin A
MSLISKEELIKLAYSIRPRENEYKTILTNLDEYNKLTTNNNENKYLQLKKLNESIDVFMNKYKTSSRNRALSNLKKDILKEVILIKNSNTSPVEKNLHFVWIGGEVSDIALEYIKQWADINAEYNIKLWYDSEAFLVNTLKKAIVESSTTEALQLLEEEIQNPQFDNMKFYKKRMEFIYDRQKRFINYYKSQINKPTVPTIDDIIKSHLVSEYNRDETVLESYRTNSLRKINSNHGIDIRANSLFTEQELLNIYSQELLNRGNLAAASDIVRLLALKNFGGVYLDVDMLPGIHSDLFKTISRPSSIGLDRWEMIKLEAIMKYKKYINNYTSENFDKLDQQLKDNFKLIIESKSEKSEIFSKLENLNVSDLEIKIAFALGSVINQALISKQGSYLTNLVIEQVKNRYQFLNQHLNPAIESDNNFTDTTKIFHDSLFNSATAENSMFLTKIAPYLQVGFMPEARSTISLSGPGAYASAYYDFINLQENTIEKTLKASDLIEFKFPENNLSQLTEQEINSLWSFDQASAKYQFEKYVRDYTGGSLSEDNGVDFNKNTALDKNYLLNNKIPSNNVEEAGSKNYVHYIIQLQGDDISYEATCNLFSKNPKNSIIIQRNMNESAKSYFLSDDGESILELNKYRIPERLKNKEKVKVTFIGHGKDEFNTSEFARLSVDSLSNEISSFLDTIKLDISPKNVEVNLLGCNMFSYDFNVEETYPGKLLLSIMDKITSTLPDVNKNSITIGANQYEVRINSEGRKELLAHSGKWINKEEAIMSDLSSKEYIFFDSIDNKLKAKSKNIPGLASISEDIKTLLLDASVSPDTKFILNNLKLNIESSIGDYIYYEKLEPVKNIIHNSIDDLIDEFNLLENVSDELYELKKLNNLDEKYLISFEDISKNNSTYSVRFINKSNGESVYVETEKEIFSKYSEHITKEISTIKNSIITDVNGNLLDNIQLDHTSQVNTLNAAFFIQSLIDYSSNKDVLNDLSTSVKVQLYAQLFSTGLNTIYDSIQLVNLISNAVNDTINVLPTITEGIPIVSTILDGINLGAAIKELLDEHDPLLKKELEAKVGVLAINMSLSIAATVASIVGIGAEVTIFLLPIAGISAGIPSLVNNELILHDKATSVVNYFNHLSESKKYGPLKTEDDKILVPIDDLVISEIDFNNNSIKLGTCNILAMEGGSGHTVTGNIDHFFSSPSISSHIPSLSIYSAIGIETENLDFSKKIMMLPNAPSRVFWWETGAVPGLRSLENDGTRLLDSIRDLYPGKFYWRFYAFFDYAITTLKPVYEDTNIKIKLDKDTRNFIMPTITTNEIRNKLSYSFDGAGGTYSLLLSSYPISTNINLSKDDLWIFNIDNEVREISIENGTIKKGKLIKDVLSKIDINKNKLIIGNQTIDFSGDIDNKDRYIFLTCELDDKISLIIEINLVAKSYSLLLSGDKNYLISNLSNTIEKINTLGLDSKNIAYNYTDESNNKYFGAISKTSQKSIIHYKKDSKNILEFYNDSTLEFNSKDFIAEDINVFMKDDINTITGKYYVDNNTDKSIDFSISLVSKNQVKVNGLYLNESVYSSYLDFVKNSDGHHNTSNFMNLFLDNISFWKLFGFENINFVIDKYFTLVGKTNLGYVEFICDNNKNIDIYFGEWKTSSSKSTIFSGNGRNVVVEPIYNPDTGEDISTSLDFSYEPLYGIDRYINKVLIAPDLYTSLININTNYYSNEYYPEIIVLNPNTFHKKVNINLDSSSFEYKWSTEGSDFILVRYLEESNKKILQKIRIKGILSNTQSFNKMSIDFKDIKKLSLGYIMSNFKSFNSENELDRDHLGFKIIDNKTYYYDEDSKLVKGLININNSLFYFDPIEFNLVTGWQTINGKKYYFDINTGAALTSYKIINGKHFYFNNDGVMQLGVFKGPDGFEYFAPANTQNNNIEGQAIVYQSKFLTLNGKKYYFDNNSKAVTGWRIINNEKYYFNPNNAIAAVGLQVIDNNKYYFNPDTAIISKGWQTVNGSRYYFDTDTAIAFNGYKTIDGKHFYFDSDCVVKIGVFSTSNGFEYFAPANTYNNNIEGQAIVYQSKFLTLNGKKYYFDNNSKAVTGLQTIDSKKYYFNTNTAEAATGWQTIDGKKYYFNTNTAEAATGWQTIDGKKYYFNTNTAIASTGYTIINGKHFYFNTDGIMQIGVFKGPNGFEYFAPANTDANNIEGQAILYQNEFLTLNGKKYYFGSDSKAVTGWRIINNKKYYFNPNNAIAAIHLCTINNDKYYFSYDGILQNGYITIERNNFYFDANNESKMVTGVFKGPNGFEYFAPANTHNNNIEGQAIVYQNKFLTLNGKKYYFDNDSKAVTGWQTIDGKKYYFNLNTAEAATGWQTIDGKKYYFNLNTAEAATGWQTIDGKKYYFNTNTFIASTGYTSINGKHFYFNTDGIMQIGVFKGPNGFEYFAPANTDANNIEGQAILYQNKFLTLNGKKYYFGSDSKAVTGLRTIDGKKYYFNTNTAVAVTGWQTINGKKYYFNTNTSIASTGYTIISGKHFYFNTDGIMQIGVFKGPDGFEYFAPANTDANNIEGQAIRYQNRFLYLHDNIYYFGNNSKAATGWVTIDGNRYYFEPNTAMGANGYKTIDNKNFYFRNGLPQIGVFKGSNGFEYFAPANTDANNIEGQAIRYQNRFLHLLGKIYYFGNNSKAVTGWQTINGKVYYFMPDTAMAAAGGLFEIDGVIYFFGVDGVKAPGIYG

SEQ ID NO: 256 - DNA, 8407 bp, Clostridium difficile
  misc_feature 1..8407: note = C difficile Toxin A
  misc_feature 8372: note = n = unknown or any nucleotide
  source 1..8407: mol_type = other DNA
ataaaaaatcaatattaatttatttttaaaaaatagaaaggagtgtataagatttattttcaaagtttaaaaacaagaaaatcaatttaaatttcagaaggaataaatgtggttatagaagtggatttattatcaaaaataataatactaggaggtttttatgtctttaatatctaaagaagagttaataaaactcgcatatagcattagaccaagagaaaatgagtataaaactatactaactaatttagacgaatataataagttaactacaaacaataatgaaaataaatatttacaattaaaaaaactaaatgaatcaattgatgtttttatgaataaatataaaacttcaagcagaaatagagcactctctaatctaaaaaaagatatattaaaagaagtaattcttattaaaaattccaatacaagccctgtagaaaaaaatttacattttgtatggataggtggagaagtcagtgatattgctcttgaatacataaaacaatgggctgatattaatgcagaatataatattaaactgtggtatgatagtgaagcattcttagtaaatacactaaaaaaggctatagttgaatcttctaccactgaagcattacagctactagaggaagagattcaaaatcctcaatttgataatatgaaattttacaaaaaaaggatggaatttatatatgatagacaaaaaaggtttataaattattataaatctcaaatcaataaacctacagtacctacaatagatgatattataaagtctcatctagtatctgaatataatagagatgaaactgtattagaatcatatagaacaaattctttgagaaaaataaatagtaatcatgggatagatatcagggctaatagtttgtttacagaacaagagttattaaatatttatagtcaggagttgttaaatcgtggaaatttagctgcagcatctgacatagtaagattattagccctaaaaaattttggcggagtatatttagatgttgatatgcttccaggtattcactctgatttatttaaaacaatatctagacctagctctattggactagaccgttgggaaatgataaaattagaggctattatgaagtataaaaaatatataaataattatacatcagaaaactttgataaacttgatcaacaattaaaagataattttaaactcattatagaaagtaaaagtgaaaaatctgagatattttctaaattagaaaatttaaatgtatctgatcttgaaattaaaatagctttcgctttaggcagtgttataaatcaagccttgatatcaaaacaaggttcatatcttactaacctagtaatagaacaagtaaaaaatagatatcaatttttaaaccaacaccttaacccagccatagagtctgataataacttcacagatactactaaaatttttcatgattcattatttaattcagctaccgcagaaaactctatgtttttaacaaaaatagcaccatacttacaagtaggttttatgccagaagctcgctccacaataagtttaagtggtccaggagcttatgcgtcagcttactatgatttcataaatttacaagaaaatactatagaaaaaactttaaaagcatcagatttaatagaatttaaattcccagaaaataatctatctcaattgacagaacaagaaataaatagtctatggagctttgatcaagcaagtgcaaaatatcaatttgagaaatatgtaagagattatactggtggatctctttctgaagacaatggggtagactttaataaaaatactgccctcgacaaaaactatttattaaataataaaattccatcaaacaatgtagaagaagctggaagtaaaaattatgttcattatatcatacagttacaaggagatgatataagttatgaagcaacatgcaatttattttctaaaaatcctaaaaatagtattattatacaacgaaatatgaatgaaagtgcaaaaagctactttttaagtgatgatggagaatctattttagaattaaataaatataggatacctgaaagattaaaaaataaggaaaaagtaaaagtaacctttattggacatggtaaagatgaattcaacacaagcgaatttgctagattaagtgtagattcactttccaatgagataagttcatttttagataccataaaattagatatatcacctaaaaatgtagaagtaaacttacttggatgtaatatgtttagttatgattttaatgttgaagaaacttatcctgggaagttgctattaagtattatggacaaaattacttccactttacctgatgtaaataaaaattctattactataggagcaaatcaatatgaagtaagaattaatagtgagggaagaaaagaacttctggctcactcaggtaaatggataaataaagaagaagctattatgagcgatttatctagtaaagaatacattttttttgattctatagataataagctaaaagcaaagtccaagaatattccaggattagcatcaatatcagaagatataaaaacattattacttgatgcaagtgttagtcctgatacaaaatttattttaaataatcttaagcttaatattgaatcttctattggggattacatttattatgaaaaattagagcctgttaaaaatataattcacaattctatagatgatttaatagatgagttcaatctacttgaaaatgtatctgatgaattatatgaattaaaaaaattaaataatctagatgagaagtatttaatatcttttgaagatatctcaaaaaataattcaacttactctgtaagatttattaacaaaagtaatggtgagtcagtttatgtagaaacagaaaaagaaattttttcaaaatatagcgaacatattacaaaagaaataagtactataaagaatagtataattacagatgttaatggtaatttattggataatatacagttagatcatacttctcaagttaatacattaaacgcagcattctttattcaatcattaatagattatagtagcaataaagatgtactgaatgatttaagtacctcagttaaggttcaactttatgctcaactatttagtacaggtttaaatactatatatgactctatccaattagtaaatttaatatcaaatgcagtaaatgatactataaatgtactacctacaataacagaggggatacctattgtatctactatattagacggaataaacttaggtgcagcaattaaggaattactagacgaacatgacccattactaaaaaaagaattagaagctaaggtgggtgttttagcaataaatatgtcattatctatagctgcaactgtagcttcaattgttggaataggtgctgaagttactattttcttattacctatagctggtatatctgcaggaataccttcattagttaataatgaattaatattgcatgataaggcaacttcagtggtaaactattttaatcatttgtctgaatctaaaaaatatggccctcttaaaacagaagatgataaaattttagttcctattgatgatttagtaatatcagaaatagattttaataataattcgataaaactaggaacatgtaatatattagcaatggaggggggatcaggacacacagtgactggtaatatagatcactttttctcatctccatctataagttctcatattccttcattatcaatttattctgcaataggtatagaaacagaaaatctagatttttcaaaaaaaataatgatgttacctaatgctccttcaagagtgttttggtgggaaactggagcagttccaggtttaagatcattggaaaatgacggaactagattacttgattcaataagagatttatacccaggtaaattttactggagattctatgcttttttcgattatgcaataactacattaaaaccagtttatgaagacactaatattaaaattaaactagataaagatactagaaacttcataatgccaactataactactaacgaaattagaaacaaattatcttattcatttgatggagcaggaggaacttactctttattattatcttcatatccaatatcaacgaatataaatttatctaaagatgatttatggatatttaatattgataatgaagtaagagaaatatctatagaaaatggtactattaaaaaaggaaagttaataaaagatgttttaagtaaaattgatataaataaaaataaacttattataggcaatcaaacaatagatttttcaggcgatatagataataaagatagatatatattcttgacttgtgagttagatgataaaattagtttaataatagaaataaatcttgttgcaaaatcttatagtttgttattgtctggggataaaaattatttgatatccaatttatctaatactattgagaaaatcaatactttaggcctagatagtaaaaatatagcgtacaattacactgatgaatctaataataaatattttggagctatatctaaaacaagtcaaaaaagcataatacattataaaaaagacagtaaaaatatattagaattttataatgacagtacattagaatttaacagtaaagattttattgctgaagatataaatgtatttatgaaagatgatattaatactataacaggaaaatactatgttgataataatactgataaaagtatagatttctctatttctttagttagtaaaaatcaagtaaaagtaaatggattatatttaaatgaatccgtatactcatcttaccttgattttgtgaaaaattcagatggacaccataatacttctaattttatgaatttatttttggacaatataagtttctggaaattgtttgggtttgaaaatataaattttgtaatcgataaatactttacccttgttggtaaaactaatcttggatatgtagaatttatttgtgacaataataaaaatatagatatatattttggtgaatggaaaacatcgtcatctaaaagcactatatttagcggaaatggtagaaatgttgtagtagagcctatatataatcctgatacgggtgaagatatatctacttcactagatttttcctatgaacctctctatggaatagatagatatataaataaagtattgatagcacctgatttatatacaagtttaataaatattaataccaattattattcaaatgagtactaccctgagattatagttcttaacccaaatacattccacaaaaaagtaaatataaatttagatagttcttcttttgagtataaatggtctacagaaggaagtgactttattttagttagatacttagaagaaagtaataaaaaaatattacaaaaaataagaatcaaaggtatcttatctaatactcaatcatttaataaaatgagtatagattttaaagatattaaaaaactatcattaggatatataatgagtaattttaaatcatttaattctgaaaatgaattagatagagatcatttaggatttaaaataatagataataaaacttattactatgatgaagatagtaaattagttaaaggattaatcaatataaataattcattattctattttgatcctatagaatttaacttagtaactggatggcaaactatcaatggtaaaaaatattattttgatataaatactggagcagctttaactagttataaaattattaatggtaaacacttttattttaataatgatggtgtgatgcagttgggagtatttaaaggacctgatggatttgaatattttgcacctgccaatactcaaaataataacatagaaggtcaggctatagtttatcaaagtaaattcttaactttgaatggcaaaaaatattattttgataataactcaaaagcagtcactggatggagaattattaacaatgagaaatattactttaatcctaataatgctattgctgcagtcggattgcaagtaattgacaataataagtattatttcaatcctgacactgctatcatctcaaaaggttggcagactgttaatggtagtagatactactttgatactgataccgctattgcctttaatggttataaaactattgatggtaaacacttttattttgatagtgattgtgtagtgaaaataggtgtgtttagtacctctaatggatttgaatattttgcacctgctaatacttataataataacatagaaggtcaggctatagtttatcaaagtaaattcttaactttgaatggtaaaaaatattactttgataataactcaaaagcagttaccggatggcaaactattgatagtaaaaaatattactttaatactaacactgctgaagcagctactggatggcaaactattgatggtaaaaaatattactttaatactaacactgctgaagcagctactggatggcaaactattgatggtaaaaaatattactttaatactaacactgctatagcttcaactggttatacaattattaatggtaaacatttttattttaatactgatggtattatgcagataggagtgtttaaaggacctaatggatttgaatattttgcacctgctaatacggatgctaacaacatagaaggtcaagctatactttaccaaaatgaattcttaactttgaatggtaaaaaatattactttggtagtgactcaaaagcagttactggatggagaattattaacaataagaaatattactttaatcctaataatgctattgctgcaattcatctatgcactataaataatgacaagtattactttagttatgatggaattcttcaaaatggatatattactattgaaagaaataatttctattttgatgctaataatgaatctaaaatggtaacaggagtatttaaaggacctaatggatttgagtattttgcacctgctaatactcacaataataacatagaaggtcaggctatagtttaccagaacaaattcttaactttgaatggcaaaaaatattattttgataatgactcaaaagcagttactggatggcaaaccattgatggtaaaaaatattactttaatcttaacactgctgaagcagctactggatggcaaactattgatggtaaaaaatattactttaatcttaacactgctgaagcagctactggatggcaaactattgatggtaaaaaatattactttaatactaacactttcatagcctcaactggttatacaagtattaatggtaaacatttttattttaatactgatggtattatgcagataggagtgtttaaaggacctaatggatttgaatactttgcacctgctaatacggatgctaacaacatagaaggtcaagctatactttaccaaaataaattcttaactttgaatggtaaaaaatattactttggtagtgactcaaaagcagttaccggactgcgaactattgatggtaaaaaatattactttaatactaacactgctgttgcagttactggatggcaaactattaatggtaaaaaatactactttaatactaacacttctatagcttcaactggttatacaattattagtggtaaacatttttattttaatactgatggtattatgcagataggagtgtttaaaggacctgatggatttgaatactttgcacctgctaatacagatgctaacaatatagaaggtcaagctatacgttatcaaaatagattcctatatttacatgacaatatatattattttggtaataattcaaaagcggctactggttgggtaactattgatggtaatagatattacttcgagcctaatacagctatgggtgcgaatggttataaaactattgataataaaaatttttactttagaaatggtttacctcagataggagtgtttaaagggtctaatggatttgaatactttgcacctgctaatacggatgctaacaatatagaaggtcaagctatacgttatcaaaatagattcctacatttacttggaaaaatatattactttggtaataattcaaaagcagttactggatggcaaactattaatggtaaagtatattactttatgcctgatactgctatggctgcagctggtggacttttcgagattgatggtgttatatatttctttggtgttgatggagtaaaagcccctgggatatatggctaaaatatatgtttgataaaaaattattcctgtgctactaagaaattatttttatataataaatattgagatttaattaaantcatgtgttattgtaatacatgacttttagttaaa

SEQ ID NO: 257 - protein, 2366 aa, Clostridium difficile
  REGION 1..2366: note = C difficile Toxin B
MSLVNRKQLEKMANVRFRTQEDEYVAILDALEEYHNMSENTVVEKYLKLKDINSLTDIYIDTYKKSGRNKALKKFKEYLVTEVLELKNNNLTPVEKNLHFVWIGGQINDTAINYINQWKDVNSDYNVNVFYDSNAFLINTLKKTVVESAINDTLESFRENLNDPRFDYNKFFRKRMEIIYDKQKNFINYYKAQREENPELIIDDIVKTYLSNEYSKEIDELNTYIEESLNKITQNSGNDVRNFEEFKNGESFNLYEQELVERWNLAAASDILRISALKEIGGMYLDVDMLPGIQPDLFESIEKPSSVTVDFWEMTKLEAIMKYKEYIPEYTSEHFDMLDEEVQSSFESVLASKSDKSEIFSSLGDMEASPLEVKIAFNSKGIINQGLISVKDSYCSNLIVKQIENRYKILNNSLNPAISEDNDFNTTTNTFIDSIMAEANADNGRFMMELGKYLRVGFFPDVKTTINLSGPEAYAAAYQDLLMFKEGSMNIHLIEADLRNFEISKTNISQSTEQEMASLWSFDDARAKAQFEEYKRNYFEGSLGEDDNLDFSQNIVVDKEYLLEKISSLARSSERGYIHYIVQLQGDKISYEAACNLFAKTPYDSVLFQKNIEDSEIAYYYNPGDGEIQEIDKYKIPSIISDRPKIKLTFIGHGKDEFNTDIFAGFDVDSLSTEIEAAIDLAKEDISPKSIEINLLGCNMFSYSINVEETYPGKLLLKVKDKISELMPSISQDSIIVSANQYEVRINSEGRRELLDHSGEWINKEESIIKDISSKEYISFNPKENKITVKSKNLPELSTLLQEIRNNSNSSDIELEEKVMLTECEINVISNIDTQIVEERIEEAKNLTSDSINYIKDEFKLIESISDALCDLKQQNELEDSHFISFEDISETDEGFSIRFINKETGESIFVETEKTIFSEYANHITEEISKIKGTIFDTVNGKLVKKVNLDTTHEVNTLNAAFFIQSLIEYNSSKESLSNLSVAMKVQVYAQLFSTGLNTITDAAKVVELVSTALDETIDLLPTLSEGLPIIATIIDGVSLGAAIKELSETSDPLLRQEIEAKIGIMAVNLTTATTAIITSSLGIASGFSILLVPLAGISAGIPSLVNNELVLRDKATKVVDYFKHVSLVETEGVFTLLDDKIMMPQDDLVISEIDFNNNSIVLGKCEIWRMEGGSGHTVTDDIDHFFSAPSITYREPHLSIYDVLEVQKEELDLSKDLMVLPNAPNRVFAWETGWTPGLRSLENDGTKLLDRIRDNYEGEFYWRYFAFIADALITTLKPRYEDTNIRINLDSNTRSFIVPIITTEYIREKLSYSFYGSGGTYALSLSQYNMGINIELSESDVWIIDVDNVVRDVTIESDKIKKGDLIEGILSTLSIEENKIILNSHEINFSGEVNGSNGFVSLTFSILEGINAIIEVDLLSKSYKLLISGELKILMLNSNHIQQKIDYIGFNSELQKNIPYSFVDSEGKENGFINGSTKEGLFVSELPDVVLISKVYMDDSKPSFGYYSNNLKDVKVITKDNVNILTGYYLKDDIKISLSLTLQDEKTIKLNSVHLDESGVAEILKFMNRKGNTNTSDSLMSFLESMNIKSIFVNFLQSNIKFILDANFIISGTTSIGQFEFICDENDNIQPYFIKFNTLETNYTLYVGNRQNMIVEPNYDLDDSGDISSTVINFSQKYLYGIDSCVNKVVISPNIYTDEINITPVYETNNTYPEVIVLDANYINEKINVNINDLSIRYVWSNDGNDFILMSTSEENKVSQVKIRFVNVFKDKTLANKLSFNFSDKQDVPVSEIILSFTPSYYEDGLIGYDLGLVSLYNEKFYINNFGMMVSGLIYINDSLYYFKPPVNNLITGFVTVGDDKYYFNPINGGAASIGETIIDDKNYYFNQSGVLQTGVFSTEDGFKYFAPANTLDENLEGEAIDFTGKLIIDENIYYFDDNYRGAVEWKELDGEMHYFSPETGKAFKGLNQIGDYKYYFNSDGVMQKGFVSINDNKHYFDDSGVMKVGYTEIDGKHFYFAENGEMQIGVFNTEDGFKYFAHHNEDLGNEEGEEISYSGILNFNNKIYYFDDSFTAVVGWKDLEDGSKYYFDEDTAEAYIGLSLINDGQYYFNDDGIMQVGFVTINDKVFYFSDSGIIESGVQNIDDNYFYIDDNGIVQIGVFDTSDGYKYFAPANTVNDNIYGQAVEYSGLVRVGEDVYYFGETYTIETGWIYDMENESDKYYFNPETKKACKGINLIDDIKYYFDEKGIMRTGLISFENNNYYFNENGEMQFGYINIEDKMFYFGEDGVMQIGVFNTPDGFKYFAHQNTLDENFEGESINYTGWLDLDEKRYYFTDEYIAATGSVIIDGEEYYFDPDTAQLVISE

SEQ ID NO: 258 - DNA, 7692 bp, Clostridium difficile
  misc_feature 1..7692: note = C difficile Toxin B
  source 1..7692: mol_type = other DNA
tctagacaagctgttaataaggctaaaaatagagcatttaaaaaaataaaaaaagactatgaaaattattttaacttgtaattaatgagcttaaagagatatttataatagaaatcaaattttagaattaactttattgtaaaatcaataacttaatctaagaatatcttaatttttatattttatatagaacaaagtttacatatttatttcagacaacgtctttattcaatcgaagagcaaattaatcaactgagtgtcttaaatttaaaatgttaggaagtgaatgtatatgaaaacctaagtagatattagtatattttataaatagaaaggaggatatataaaagagttttagcatttagatgtaaaaatattatagtaaaggagaaaattttatgagtttagttaatagaaaacagttagaaaaaatggcaaatgtaagatttcgtactcaagaagatgaatatgttgcaatattggatgctttagaagaatatcataatatgtcagagaatactgtagtcgaaaaatatttaaaattaaaagatataaatagtttaacagatatttatatagatacatataaaaaatctggtagaaataaagccttaaaaaaatttaaggaatatctagttacagaagtattagagctaaagaataataatttaactccagttgagaaaaatttacattttgtttggattggaggtcaaataaatgacactgctattaattatataaatcaatggaaagatgtaaatagtgattataatgttaatgttttttatgatagtaatgcatttttgataaacacattgaaaaaaactgtagtagaatcagcaataaatgatacacttgaatcatttagagaaaacttaaatgaccctagatttgactataataaattcttcagaaaacgtatggaaataatttatgataaacagaaaaatttcataaactactataaagctcaaagagaagaaaatcctgaacttataattgatgatattgtaaagacatatctttcaaatgagtattcaaaggagatagatgaacttaatacctatattgaagaatccttaaataaaattacacagaatagtggaaatgatgttagaaactttgaagaatttaaaaatggagagtcattcaacttatatgaacaagagttggtagaaaggtggaatttagctgctgcttctgacatattaagaatatctgcattaaaagaaattggtggtatgtatttagatgttgatatgttaccaggaatacaaccagacttatttgagtctatagagaaacctagttcagtaacagtggatttttgggaaatgacaaagttagaagctataatgaaatacaaagaatatataccagaatatacctcagaacattttgacatgttagacgaagaagttcaaagtagttttgaatctgttctagcttctaagtcagataaatcagaaatattctcatcacttggtgatatggaggcatcaccactagaagttaaaattgcatttaatagtaagggtattataaatcaagggctaatttctgtgaaagactcatattgtagcaatttaatagtaaaacaaatcgagaatagatataaaatattgaataatagtttaaatccagctattagcgaggataatgattttaatactacaacgaatacctttattgatagtataatggctgaagctaatgcagataatggtagatttatgatggaactaggaaagtatttaagagttggtttcttcccagatgttaaaactactattaacttaagtggccctgaagcatatgcggcagcttatcaagatttattaatgtttaaagaaggcagtatgaatatccatttgatagaagctgatttaagaaactttgaaatctctaaaactaatatttctcaatcaactgaacaagaaatggctagcttatggtcatttgacgatgcaagagctaaagctcaatttgaagaatataaaaggaattattttgaaggttctcttggtgaagatgataatcttgatttttctcaaaatatagtagttgacaaggagtatcttttagaaaaaatatcttcattagcaagaagttcagagagaggatatatacactatattgttcagttacaaggagataaaattagttatgaagcagcatgtaacttatttgcaaagactccttatgatagtgtactgtttcagaaaaatatagaagattcagaaattgcatattattataatcctggagatggtgaaatacaagaaatagacaagtataaaattccaagtataatttctgatagacctaagattaaattaacatttattggtcatggtaaagatgaatttaatactgatatatttgcaggttttgatgtagattcattatccacagaaatagaagcagcaatagatttagctaaagaggatatttctcctaagtcaatagaaataaatttattaggatgtaatatgtttagctactctatcaacgtagaggagacttatcctggaaaattattacttaaagttaaagataaaatatcagaattaatgccatctataagtcaagactctattatagtaagtgcaaatcaatatgaagttagaataaatagtgaaggaagaagagaattattggatcattctggtgaatggataaataaagaagaaagtattataaaggatatttcatcaaaagaatatatatcatttaatcctaaagaaaataaaattacagtaaaatctaaaaatttacctgagctatctacattattacaagaaattagaaataattctaattcaagtgatattgaactagaagaaaaagtaatgttaacagaatgtgagataaatgttatttcaaatatagatacgcaaattgttgaggaaaggattgaagaagctaagaatttaacttctgactctattaattatataaaagatgaatttaaactaatagaatctatttctgatgcactatgtgacttaaaacaacagaatgaattagaagattctcattttatatcttttgaggacatatcagagactgatgagggatttagtataagatttattaataaagaaactggagaatctatatttgtagaaactgaaaaaacaatattctctgaatatgctaatcatataactgaagagatttctaagataaaaggtactatatttgatactgtaaatggtaagttagtaaaaaaagtaaatttagatactacacacgaagtaaatactttaaatgctgcattttttatacaatcattaatagaatataatagttctaaagaatctcttagtaatttaagtgtagcaatgaaagtccaagtttacgctcaattatttagtactggtttaaatactattacagatgcagccaaagttgttgaattagtatcaactgcattagatgaaactatagacttacttcctacattatctgaaggattacctataattgcaactattatagatggtgtaagtttaggtgcagcaatcaaagagctaagtgaaacgagtgacccattattaagacaagaaatagaagctaagataggtataatggcagtaaatttaacaacagctacaactgcaatcattacttcatctttggggatagctagtggatttagtatacttttagttcctttagcaggaatttcagcaggtataccaagcttagtaaacaatgaacttgtacttcgagataaggcaacaaaggttgtagattattttaaacatgtttcattagttgaaactgaaggagtatttactttattagatgataaaataatgatgccacaagatgatttagtgatatcagaaatagattttaataataattcaatagttttaggtaaatgtgaaatctggagaatggaaggtggttcaggtcatactgtaactgatgatatagatcacttcttttcagcaccatcaataacatatagagagccacacttatctatatatgacgtattggaagtacaaaaagaagaacttgatttgtcaaaagatttaatggtattacctaatgctccaaatagagtatttgcttgggaaacaggatggacaccaggtttaagaagcttagaaaatgatggcacaaaactgttagaccgtataagagataactatgaaggtgagttttattggagatattttgcttttatagctgatgctttaataacaacattaaaaccaagatatgaagatactaatataagaataaatttagatagtaatactagaagttttatagttccaataataactacagaatatataagagaaaaattatcatattctttctatggttcaggaggaacttatgcattgtctctttctcaatataatatgggtataaatatagaattaagtgaaagtgatgtttggattatagatgttgataatgttgtgagagatgtaactatagaatctgataaaattaaaaaaggtgatttaatagaaggtattttatctacactaagtattgaagagaataaaattatcttaaatagccatgagattaatttttctggtgaggtaaatggaagtaatggatttgtttctttaacattttcaattttagaaggaataaatgcaattatagaagttgatttattatctaaatcatataaattacttatttctggcgaattaaaaatattgatgttaaattcaaatcatattcaacagaaaatagattatataggattcaatagcgaattacagaaaaatataccatatagctttgtagatagtgaaggaaaagagaatggttttattaatggttcaacaaaagaaggtttatttgtatctgaattacctgatgtagttcttataagtaaggtttatatggatgatagtaagccttcatttggatattatagtaataatttgaaagatgtcaaagttataactaaagataatgttaatatattaacaggttattatcttaaggatgatataaaaatctctctttctttgactctacaagatgaaaaaactataaagttaaatagtgtgcatttagatgaaagtggagtagctgagattttgaagttcatgaatagaaaaggtaatacaaatacttcagattctttaatgagctttttagaaagtatgaatataaaaagtattttcgttaatttcttacaatctaatattaagtttatattagatgctaattttataataagtggtactacttctattggccaatttgagtttatttgtgatgaaaatgataatatacaaccatatttcattaagtttaatacactagaaactaattatactttatatgtaggaaatagacaaaatatgatagtggaaccaaattatgatttagatgattctggagatatatcttcaactgttatcaatttctctcaaaagtatctttatggaatagacagttgtgttaataaagttgtaatttcaccaaatatttatacagatgaaataaatataacgcctgtatatgaaacaaataatacttatccagaagttattgtattagatgcaaattatataaatgaaaaaataaatgttaatatcaatgatctatctatacgatatgtatggagtaatgatggtaatgattttattcttatgtcaactagtgaagaaaataaggtgtcacaagttaaaataagattcgttaatgtttttaaagataagactttggcaaataagctatcttttaactttagtgataaacaagatgtacctgtaagtgaaataatcttatcatttacaccttcatattatgaggatggattgattggctatgatttgggtctagtttctttatataatgagaaattttatattaataactttggaatgatggtatctggattaatatatattaatgattcattatattattttaaaccaccagtaaataatttgataactggatttgtgactgtaggcgatgataaatactactttaatccaattaatggtggagctgcttcaattggagagacaataattgatgacaaaaattattatttcaaccaaagtggagtgttacaaacaggtgtatttagtacagaagatggatttaaatattttgccccagctaatacacttgatgaaaacctagaaggagaagcaattgattttactggaaaattaattattgacgaaaatatttattattttgatgataattatagaggagctgtagaatggaaagaattagatggtgaaatgcactattttagcccagaaacaggtaaagcttttaaaggtctaaatcaaataggtgattataaatactatttcaattctgatggagttatgcaaaaaggatttgttagtataaatgataataaacactattttgatgattctggtgttatgaaagtaggttacactgaaatagatggcaagcatttctactttgctgaaaacggagaaatgcaaataggagtatttaatacagaagatggatttaaatattttgctcatcataatgaagatttaggaaatgaagaaggtgaagaaatctcatattctggtatattaaatttcaataataaaatttactattttgatgattcatttacagctgtagttggatggaaagatttagaggatggttcaaagtattattttgatgaagatacagcagaagcatatataggtttgtcattaataaatgatggtcaatattattttaatgatgatggaattatgcaagttggatttgtcactataaatgataaagtcttctacttctctgactctggaattatagaatctggagtacaaaacatagatgacaattatttctatatagatgataatggtatagttcaaattggtgtatttgatacttcagatggatataaatattttgcacctgctaatactgtaaatgataatatttacggacaagcagttgaatatagtggtttagttagagttggggaagatgtatattattttggagaaacatatacaattgagactggatggatatatgatatggaaaatgaaagtgataaatattatttcaatccagaaactaaaaaagcatgcaaaggtattaatttaattgatgatataaaatattattttgatgagaagggcataatgagaacgggtcttatatcatttgaaaataataattattactttaatgagaatggtgaaatgcaatttggttatataaatatagaagataagatgttctattttggtgaagatggtgtcatgcagattggagtatttaatacaccagatggatttaaatactttgcacatcaaaatactttggatgagaattttgagggagaatcaataaactatactggttggttagatttagatgaaaagagatattattttacagatgaatatattgcagcaactggttcagttattattgatggtgaggagtattattttgatcctgatacagctcaattagtgattagtgaatagataaaaatatgttaaatatatcctcttatacttaaatatataaaaataaacaaaatgatacactacataaagtgttctatctaatatgaagatttaccaataaaaaggtggactatgatgaatgcacagtagttcacctttttatattactaatggtaacaaaatatttttttatataaacctaggaggcgtt

SEQ ID NO: 259 - DNA, 26039 bp, Clostridium difficile
  misc_feature 1..26039: note = >ENA|X92982|X92982.1 C.difficile cdu2, cdu1, tcdD, tcdB, tcdE, tcdA, tcdC, cdd1, cdd2, cdd3, and cdd4 genes
  source 1..26039: mol_type = other DNA
agctagtcttggtgtattgttagcaggattttttaatttgccaattgaattagttgcagccgttggctatgctagtgtctttggtagtgctacaaatactttttttgcacctgtatttataggggcagaagtttttggatacagctatttaccttatttctttgtagtatgcgctatttcatatatatttaatatggataaatctatttattcactacaaaaaatttcaacaaaacaataaataaaacaacataatgtatgattagaagagaaagaatattagagaaaggatagggtaggaatatgttgacaagtttagctttgatttttttattaggaatggcctcgggaggtatttttaagaggataaagttacctaacttattgggaatgttacttacaggaattatattaggtccatatgttttaaatttgattgataattcaatactagatatttcttctgaccttagaaagattgcattgattattatattaacaagggctggattatctttagatataaacgatttgaagaaagtgggaagacctgctgtacttatgtgctttattccagctacttttgaaattatcggaatgatagttttagcaccaaagttactaggcgtttctatattggaagcagcagtcatgggtgcagtagtaggagcagtttctcctgcaattattgtacctaaaatgcttaaattaatggaagaaggttatggtacagaaaaaagtattccacagatgcttttagcaggaacttctatagacgatattttcgtaattgtgatgtttacagtattcacaggattggcacaaggaaatagtatatcagctattagttttttacaaattccagtatcaattatattaggtgtaatagctggagcagtgattggaatctgtttagcagtattttttaagaaggttcatatgagagattctgctaaaggggtgttgcttttaagtatctcatttttaatgataagtttagaaactgctttagagggtattgtgccattttctggattattagcagttatgagtattgggattttccttcagataaaatatcgtgtagttgcaagaagattgtctataaagtattcaaaactatgggttggcgctgaaattctcttgtttgttttggtaggggcaacagtagatataagttatgcatttaaagcaggaattggagctgtaattttaatatttggagttcttttattccgtatgtaggagtattcttctgccttattaagacaaatttgacaataaaggaaagattgttctgtatgattggctatattccaaaggctacagtacaggcagcaataggaggtgtaccacttgcaatggggatggcatctggacaacttattttgacgttagcagttctcgctatacttataactgcacctcttggagcttttggaattgatgtaacttataaaaaattattaacttctgtaaaaggcgagagtaagtaaaaataaagattattttaactggtaagttatattttggaaaaggattatactattgaatacaatataaaaaaatcatttgggagattaagaaggtagaagttaagaacagattttaaggtatgttatgattattagaattgattttgtgaaattattattgtaatatttaattatatagataaagaagcggagtgataactatgtgtttaaaaaaattatcaaaattagagttagttattatgaaatttatttggaatttagatataaaaaccaattcatatgagattattgattatatgaaagaagaacataatttaccagaaaaagtagctttaaaaactttatcaaaactatcaaagaaaaaattcttatatgttcaagaaacaggcaagtgtatgtattatacagttgcaataaaagaaaaggcatatttagagtttatatcaagaaatgtgcaaaatcttttgaagaataattttataaggaatttattagtatcatttcacgaagaggagctaacagaggaaaagataaagtcgttagaaaactgggtagtaaattgggaagaagcttatgtataaatgttattatttttattacaatttagataattttggttttgtaagctctgcaactatttttagatggttgcagagtttatttttattttttattcccttaagcaatacttaaaagtaaacgcatttatatttactaacttcaattacttctaatacttaaattactttttaaaaatattttgatatgtcatctctatagtaatctagaacttgtttctattctttatataaagtttttatgaatgatatatataatattcgttcatttgattaaaaataacaaaatattaaataattctactctgatagtttgttaaaaaaataataaaaaatattaataaacaaaaaaaaaattatcttaagagaggagaatgttataatataaaaaggtttctagatttcataaaagatactattttagtcttgaaaatatttagtttgaaaagattttaatttaatgattgattaagttaaaaatgtgtatgtaataaattttattttatttattgactaaattataaagtttacataattatttaataattatgtaattgttacttgaaaattgatctattttaaaatctagttataacttcaaaaaagactgaaaattaagaaaaaagaaatataaatataaaaatatgtcatatagattttttttattttactttaataaaatgatttgtttttacaatactttattaatataaagtttattgctaaaatactttatttattagaaaaagattactaattaattattaaaattaatgtattcataatgcatattttcatataaaatttaatttatttgccgattatataattataattactgatttaattccaatgttgttcaaaattttcaaataaagcatcattataaatataagagagggtgattttatgcaaaagtctttttatgaattaattgttttagcaagaaataactcagtagatgatttgcaagaaattttatttatgtttaagccattagtaaaaaaacttagtagagttttacattatgaagagggagaaacagatttaataatattttttattgaattaataaaaaatattaaattaagtagcttttcagaaaaaagcgatgctattatagtcaaatatattcataaatcattactgaataagacttttgagttgtctagaagatattctaaaatgaagtttaattttgtagaatttgatgaaaatatcttaaatatgaaaaataattatcaaagtaagtctgtttttgaggaagatatttgttttttcgaatatattttgaaagaattatctggtattcaaagaaaagttattttttataaatatttaaaaggatattctgatagagaaatatcagtgaaattaaaaatatctagacaagctgttaataaggctaaaaatagagcatttaaaaaaataaaaaaagactatgaaaattattttaacttgtaattaatgagcttaaagagatatttataatagaaatcaaattttagaattaactttattgtaaaatcaataacttaatctaagaatatcttaatttttatattttatatagaacaaagtttacatatttatttcagacaacgtctttattcaatcgaagagcaaattaatcaactgagtgtcttaaatttaaaatgttaggaagtgaatgtatatgaaaacctaagtagatattagtatattttataaatagaaaggaggatatataaaagagttttagcatttagatgtaaaaatattatagtaaaggagaaaattttatgagtttagttaatagaaaacagttagaaaaaatggcaaatgtaagatttcgtactcaagaagatgaatatgttgcaatattggatgctttagaagaatatcataatatgtcagagaatactgtagtcgaaaaatatttaaaattaaaagatataaatagtttaacagatatttatatagatacatataaaaaatctggtagaaataaagccttaaaaaaatttaaggaatatctagttacagaagtattagagctaaagaataataatttaactccagttgagaaaaatttacattttgtttggattggaggtcaaataaatgacactgctattaattatataaatcaatggaaagatgtaaatagtgattataatgttaatgttttttatgatagtaatgcatttttgataaacacattgaaaaaaactgtagtagaatcagcaataaatgatacacttgaatcatttagagaaaacttaaatgaccctagatttgactataataaattcttcagaaaacgtatggaaataatttatgataaacagaaaaatttcataaactactataaagctcaaagagaagaaaatcctgaacttataattgatgatattgtaaagacatatctttcaaatgagtattcaaaggagatagatgaacttaatacctatattgaagaatccttaaataaaattacacagaatagtggaaatgatgttagaaactttgaagaatttaaaaatggagagtcattcaacttatatgaacaagagttggtagaaaggtggaatttagctgctgcttctgacatattaagaatatctgcattaaaagaaattggtggtatgtatttagatgttgatatgttaccaggaatacaaccagacttatttgagtctatagagaaacctagttcagtaacagtggatttttgggaaatgacaaagttagaagctataatgaaatacaaagaatatataccagaatatacctcagaacattttgacatgttagacgaagaagttcaaagtagttttgaatctgttctagcttctaagtcagataaatcagaaatattctcatcacttggtgatatggaggcatcaccactagaagttaaaattgcatttaatagtaagggtattataaatcaagggctaatttctgtgaaagactcatattgtagcaatttaatagtaaaacaaatcgagaatagatataaaatattgaataatagtttaaatccagctattagcgaggataatgattttaatactacaacgaatacctttattgatagtataatggctgaagctaatgcagataatggtagatttatgatggaactaggaaagtatttaagagttggtttcttcccagatgttaaaactactattaacttaagtggccctgaagcatatgcggcagcttatcaagatttattaatgtttaaagaaggcagtatgaatatccatttgatagaagctgatttaagaaactttgaaatctctaaaactaatatttctcaatcaactgaacaagaaatggctagcttatggtcatttgacgatgcaagagctaaagctcaatttgaagaatataaaaggaattattttgaaggttctcttggtgaagatgataatcttgatttttctcaaaatatagtagttgacaaggagtatcttttagaaaaaatatcttcattagcaagaagttcagagagaggatatatacactatattgttcagttacaaggagataaaattagttatgaagcagcatgtaacttatttgcaaagactccttatgatagtgtactgtttcagaaaaatatagaagattcagaaattgcatattattataatcctggagatggtgaaatacaagaaatagacaagtataaaattccaagtataatttctgatagacctaagattaaattaacatttattggtcatggtaaagatgaatttaatactgatatatttgcaggttttgatgtagattcattatccacagaaatagaagcagcaatagatttagctaaagaggatatttctcctaagtcaatagaaataaatttattaggatgtaatatgtttagctactctatcaacgtagaggagacttatcctggaaaattattacttaaagttaaagataaaatatcagaattaatgccatctataagtcaagactctattatagtaagtgcaaatcaatatgaagttagaataaatagtgaaggaagaagagaattattggatcattctggtgaatggataaataaagaagaaagtattataaaggatatttcatcaaaagaatatatatcatttaatcctaaagaaaataaaattacagtaaaatctaaaaatttacctgagctatctacattattacaagaaattagaaataattctaattcaagtgatattgaactagaagaaaaagtaatgttaacagaatgtgagataaatgttatttcaaatatagatacgcaaattgttgaggaaaggattgaagaagctaagaatttaacttctgactctattaattatataaaagatgaatttaaactaatagaatctatttctgatgcactatgtgacttaaaacaacagaatgaattagaagattctcattttatatcttttgaggacatatcagagactgatgagggatttagtataagatttattaataaagaaactggagaatctatatttgtagaaactgaaaaaacaatattctctgaatatgctaatcatataactgaagagatttctaagataaaaggtactatatttgatactgtaaatggtaagttagtaaaaaaagtaaatttagatactacacacgaagtaaatactttaaatgctgcattttttatacaatcattaatagaatataatagttctaaagaatctcttagtaatttaagtgtagcaatgaaagtccaagtttacgctcaattatttagtactggtttaaatactattacagatgcagccaaagttgttgaattagtatcaactgcattagatgaaactatagacttacttcctacattatctgaaggattacctataattgcaactattatagatggtgtaagtttaggtgcagcaatcaaagagctaagtgaaacgagtgacccattattaagacaagaaatagaagctaagataggtataatggcagtaaatttaacaacagctacaactgcaatcattacttcatctttggggatagctagtggatttagtatacttttagttcctttagcaggaatttcagcaggtataccaagcttagtaaacaatgaacttgtacttcgagataaggcaacaaaggttgtagattattttaaacatgtttcattagttgaaactgaaggagtatttactttattagatgataaaataatgatgccacaagatgatttagtgatatcagaaatagattttaataataattcaatagttttaggtaaatgtgaaatctggagaatggaaggtggttcaggtcatactgtaactgatgatatagatcacttcttttcagcaccatcaataacatatagagagccacacttatctatatatgacgtattggaagtacaaaaagaagaacttgatttgtcaaaagatttaatggtattacctaatgctccaaatagagtatttgcttgggaaacaggatggacaccaggtttaagaagcttagaaaatgatggcacaaaactgttagaccgtataagagataactatgaaggtgagttttattggagatattttgcttttatagctgatgctttaataacaacattaaaaccaagatatgaagatactaatataagaataaatttagatagtaatactagaagttttatagttccaataataactacagaatatataagagaaaaattatcatattctttctatggttcaggaggaacttatgcattgtctctttctcaatataatatgggtataaatatagaattaagtgaaagtgatgtttggattatagatgttgataatgttgtgagagatgtaactatagaatctgataaaattaaaaaaggtgatttaatagaaggtattttatctacactaagtattgaagagaataaaattatcttaaatagccatgagattaatttttctggtgaggtaaatggaagtaatggatttgtttctttaacattttcaattttagaaggaataaatgcaattatagaagttgatttattatctaaatcatataaattacttatttctggcgaattaaaaatattgatgttaaattcaaatcatattcaacagaaaatagattatataggattcaatagcgaattacagaaaaatataccatatagctttgtagatagtgaaggaaaagagaatggttttattaatggttcaacaaaagaaggtttatttgtatctgaattacctgatgtagttcttataagtaaggtttatatggatgatagtaagccttcatttggatattatagtaataatttgaaagatgtcaaagttataactaaagataatgttaatatattaacaggttattatcttaaggatgatataaaaatctctctttctttgactctacaagatgaaaaaactataaagttaaatagtgtgcatttagatgaaagtggagtagctgagattttgaagttcatgaatagaaaaggtaatacaaatacttcagattctttaatgagctttttagaaagtatgaatataaaaagtattttcgttaatttcttacaatctaatattaagtttatattagatgctaattttataataagtggtactacttctattggccaatttgagtttatttgtgatgaaaatgataatatacaaccatatttcattaagtttaatacactagaaactaattatactttatatgtaggaaatagacaaaatatgatagtggaaccaaattatgatttagatgattctggagatatatcttcaactgttatcaatttctctcaaaagtatctttatggaatagacagttgtgttaataaagttgtaatttcaccaaatatttatacagatgaaataaatataacgcctgtatatgaaacaaataatacttatccagaagttattgtattagatgcaaattatataaatgaaaaaataaatgttaatatcaatgatctatctatacgatatgtatggagtaatgatggtaatgattttattcttatgtcaactagtgaagaaaataaggtgtcacaagttaaaataagattcgttaatgtttttaaagataagactttggcaaataagctatcttttaactttagtgataaacaagatgtacctgtaagtgaaataatcttatcatttacaccttcatattatgaggatggattgattggctatgatttgggtctagtttctttatataatgagaaattttatattaataactttggaatgatggtatctggattaatatatattaatgattcattatattattttaaaccaccagtaaataatttgataactggatttgtgactgtaggcgatgataaatactactttaatccaattaatggtggagctgcttcaattggagagacaataattgatgacaaaaattattatttcaaccaaagtggagtgttacaaacaggtgtatttagtacagaagatggatttaaatattttgccccagctaatacacttgatgaaaacctagaaggagaagcaattgattttactggaaaattaattattgacgaaaatatttattattttgatgataattatagaggagctgtagaatggaaagaattagatggtgaaatgcactattttagcccagaaacaggtaaagcttttaaaggtctaaatcaaataggtgattataaatactatttcaattctgatggagttatgcaaaaaggatttgttagtataaatgataataaacactattttgatgattctggtgttatgaaagtaggttacactgaaatagatggcaagcatttctactttgctgaaaacggagaaatgcaaataggagtatttaatacagaagatggatttaaatattttgctcatcataatgaagatttaggaaatgaagaaggtgaagaaatctcatattctggtatattaaatttcaataataaaatttactattttgatgattcatttacagctgtagttggatggaaagatttagaggatggttcaaagtattattttgatgaagatacagcagaagcatatataggtttgtcattaataaatgatggtcaatattattttaatgatgatggaattatgcaagttggatttgtcactataaatgataaagtcttctacttctctgactctggaattatagaatctggagtacaaaacatagatgacaattatttctatatagatgataatggtatagttcaaattggtgtatttgatacttcagatggatataaatattttgcacctgctaatactgtaaatgataatatttacggacaagcagttgaatatagtggtttagttagagttggggaagatgtatattattttggagaaacatatacaattgagactggatggatatatgatatggaaaatgaaagtgataaatattatttcaatccagaaactaaaaaagcatgcaaaggtattaatttaattgatgatataaaatattattttgatgagaagggcataatgagaacgggtcttatatcatttgaaaataataattattactttaatgagaatggtgaaatgcaatttggttatataaatatagaagataagatgttctattttggtgaagatggtgtcatgcagattggagtatttaatacaccagatggatttaaatactttgcacatcaaaatactttggatgagaattttgagggagaatcaataaactatactggttggttagatttagatgaaaagagatattattttacagatgaatatattgcagcaactggttcagttattattgatggtgaggagtattattttgatcctgatacagctcaattagtgattagtgaatagataaaaatatgttaaatatatcctcttatacttaaatatataaaaataaacaaaatgatacactacataaagtgttctatctaatatgaagatttaccaataaaaaggtggactatgatgaatgcacagtagttcacctttttatatttctaatggtaacaaaatatttttttatataaacctaggaggcgttatgaatatgacaatatcttttttatcagagcatatatttataaagttagtaattttaactatatcatttgatacattattaggatgtttaagtgcaataaaaagtcgtaaatttaattctagttttggaatagatggaggaatcagaaaagtagcaatgatagcatgtatattttttttatcagtagttgacattcttacaaagtttaactttttatttatgttaccacaagattgtatcaattttttaagactaaaacatcttggaatatctgaatttttctctattttatttattttatatgaaagtgtaagtatattaaaaaatatgtgcttatgtggattaccagtacctaagagattaaaggaaaaaatagcaattttactagatgcaatgacagatgaaatgaatgctaaggatgaaaagtaagtaatggtagatataataaagatattaacaaataaaaagtgttatccaaataagaatagctgaaagttatcataattcatgaaactaataatgaaaacgagggagcagatgccaagagacacacaagtattaaatacatataatttcgaagcaagtgttcattactatatagatgacaaggtagtatatcaaacattggttcacaaagatggtgcatggtcagttggtaaaatctattaagctacattagttacagatatcacaaactataatagttaaacatagaaatatgtgtaaattgtgatggaaattattcaaaaacacaaaaatacgtgatgaaggacaaaatgatatagaaaataagtatcaaaccttaataaatgatttaattgatagtttaaaagttataggaaaaatatataaagaaataaaaacattaaaaaaatataagatatgtttacaaattactatcagacaatctccttatctaatagaagagtcaattaactaattgagtatctttaaattgaaatgttaggaagtgatttaaatatgaaaacttaaattataaaaaatcaatattaatttatttttaaaaaatagaaaggagtgtataagatttattttcaaagtttaaaaacaagaaaatcaatttaaatttcagaaggaataaatgtggttatagaagtggatttattatcaaaaataataatactaggaggtttttatgtctttaatatctaaagaagagttaataaaactcgcatatagcattagaccaagagaaaatgagtataaaactatactaactaatttagacgaatataataagttaactacaaacaataatgaaaataaatatttgcaattaaaaaaactaaatgaatcaattgatgtttttatgaataaatataaaacttcaagcagaaatagagcactctctaatctaaaaaaagatatattaaaagaagtaattcttattaaaaattccaatacaagccctgtagaaaaaaatttacattttgtatggataggtggagaagtcagtgatattgctcttgaatacataaaacaatgggctgatattaatgcagaatataatattaaactgtggtatgatagtgaagcattcttagtaaatacactaaaaaaggctatagttgaatcttctaccactgaagcattacagctactagaggaagagattcaaaatcctcaatttgataatatgaaattttacaaaaaaaggatggaatttatatatgatagacaaaaaaggtttataaattattataaatctcaaatcaataaacctacagtacctacaatagatgatattataaagtctcatctagtatctgaatataatagagatgaaactgtattagaatcatatagaacaaattctttgagaaaaataaatagtaatcatgggatagatatcagggctaatagtttgtttacagaacaagagttattaaatatttatagtcaggagttgttaaatcgtggaaatttagctgcagcatctgacatagtaagattattagccctaaaaaattttggcggagtatatttagatgttgatatgcttccaggtattcactctgatttatttaaaacaatatctagacctagctctattggactagaccgttgggaaatgataaaattagaggctattatgaagtataaaaaatatataaataattatacatcagaaaactttgataaacttgatcaacaattaaaagataattttaaactcattatagaaagtaaaagtgaaaaatctgagatattttctaaattagaaaatttaaatgtatctgatcttgaaattaaaatagctttcgctttaggcagtgttataaatcaagccttgatatcaaaacaaggttcatatcttactaacctagtaatagaacaagtaaaaaatagatatcaatttttaaaccaacaccttaacccagccatagagtctgataataacttcacagatactactaaaatttttcatgattcattatttaattcagctaccgcagaaaactctatgtttttaacaaaaatagcaccatacttacaagtaggttttatgccagaagctcgctccacaataagtttaagtggtccaggagcttatgcgtcagcttactatgatttcataaatttacaagaaaatactatagaaaaaactttaaaagcatcagatttaatagaatttaaattcccagaaaataatctatctcaattgacagaacaagaaataaatagtctatggagctttgatcaagcaagtgcaaaatatcaatttgagaaatatgtaagagattatactggtggatctctttctgaagacaatggggtagactttaataaaaatactgccctcgacaaaaactatttattaaataataaaattccatcaaacaatgtagaagaagctggaagtaaaaattatgttcattatatcatacagttacaaggagatgatataagttatgaagcaacatgcaatttattttctaaaaatcctaaaaatagtattattatacaacgaaatatgaatgaaagtgcaaaaagctactttttaagtgatgatggagaatctattttagaattaaataaatataggatacctgaaagattaaaaaataaggaaaaagtaaaagtaacctttattggacatggtaaagatgaattcaacacaagcgaatttgctagattaagtgtagattcactttccaatgagataagttcatttttagataccataaaattagatatatcacctaaaaatgtagaagtaaacttacttggatgtaatatgtttagttatgattttaatgttgaagaaacttatcctgggaagttgctattaagtattatggacaaaattacttccactttacctgatgtaaataaaaattctattactataggagcaaatcaatatgaagtaagaattaatagtgagggaagaaaagaacttctggctcactcaggtaaatggataaataaagaagaagctattatgagcgatttatctagtaaagaatacattttttttgattctatagataataagctaaaagcaaagtccaagaatattccaggattagcatcaatatcagaagatataaaaacattattacttgatgcaagtgttagtcctgatacaaaatttattttaaataatcttaagcttaatattgaatcttctattggggattacatttattatgaaaaattagagcctgttaaaaatataattcacaattctatagatgatttaatagatgagttcaatctacttgaaaatgtatctgatgaattatatgaattaaaaaaattaaataatctagatgagaagtatttaatatcttttgaagatatctcaaaaaataattcaacttactctgtaagatttattaacaaaagtaatggtgagtcagtttatgtagaaacagaaaaagaaattttttcaaaatatagcgaacatattacaaaagaaataagtactataaagaatagtataattacagatgttaatggtaatttattggataatatacagttagatcatacttctcaagttaatacattaaacgcagcattctttattcaatcattaatagattatagtagcaataaagatgtactgaatgatttaagtacctcagttaaggttcaactttatgctcaactatttagtacaggtttaaatactatatatgactctatccaattagtaaatttaatatcaaatgcagtaaatgatactataaatgtactacctacaataacagaggggatacctattgtatctactatattagacggaataaacttaggtgcagcaattaaggaattactagacgaacatgacccattactaaaaaaagaattagaagctaaggtgggtgttttagcaataaatatgtcattatctatagctgcaactgtagcttcaattgttggaataggtgctgaagttactattttcttattacctatagctggtatatctgcaggaataccttcattagttaataatgaattaatattgcatgataaggcaacttcagtggtaaactattttaatcatttgtctgaatctaaaaaatatggccctcttaaaacagaagatgataaaattttagttcctattgatgatttagtaatatcagaaatagattttaataataattcgataaaactaggaacatgtaatatattagcaatggaggggggatcaggacacacagtgactggtaatatagatcactttttctcatctccatctataagttctcatattccttcattatcaatttattctgcaataggtatagaaacagaaaatctagatttttcaaaaaaaataatgatgttacctaatgctccttcaagagtgttttggtgggaaactggagcagttccaggtttaagatcattggaaaatgacggaactagattacttgattcaataagagatttatacccaggtaaattttactggagattctatgcttttttcgattatgcaataactacattaaaaccagtttatgaagacactaatattaaaattaaactagataaagatactagaaacttcataatgccaactataactactaacgaaattagaaacaaattatcttattcatttgatggagcaggaggaacttactctttattattatcttcatatccaatatcaacgaatataaatttatctaaagatgatttatggatatttaatattgataatgaagtaagagaaatatctatagaaaatggtactattaaaaaaggaaagttaataaaagatgttttaagtaaaattgatataaataaaaataaacttattataggcaatcaaacaatagatttttcaggcgatatagataataaagatagatatatattcttgacttgtgagttagatgataaaattagtttaataatagaaataaatcttgttgcaaaatcttatagtttgttattgtctggggataaaaattatttgatatccaatttatctaatactattgagaaaatcaatactttaggcctagatagtaaaaatatagcgtacaattacactgatgaatctaataataaatattttggagctatatctaaaacaagtcaaaaaagcataatacattataaaaaagacagtaaaaatatattagaattttataatgacagtacattagaatttaacagtaaagattttattgctgaagatataaatgtatttatgaaagatgatattaatactataacaggaaaatactatgttgataataatactgataaaagtatagatttctctatttctttagttagtaaaaatcaagtaaaagtaaatggattatatttaaatgaatccgtatactcatcttaccttgattttgtgaaaaattcagatggacaccataatacttctaattttatgaatttatttttggacaatataagtttctggaaattgtttgggtttgaaaatataaattttgtaatcgataaatactttacccttgttggtaaaactaatcttggatatgtagaatttatttgtgacaataataaaaatatagatatatattttggtgaatggaaaacatcgtcatctaaaagcactatatttagcggaaatggtagaaatgttgtagtagagcctatatataatcctgatacgggtgaagatatatctacttcactagatttttcctatgaacctctctatggaatagatagatatataaataaagtattgatagcacctgatttatatacaagtttaataaatattaataccaattattattcaaatgagtactaccctgagattatagttcttaacccaaatacattccacaaaaaagtaaatataaatttagatagttcttcttttgagtataaatggtctacagaaggaagtgactttattttagttagatacttagaagaaagtaataaaaaaatattacaaaaaataagaatcaaaggtatcttatctaatactcaatcatttaataaaatgagtatagattttaaagatattaaaaaactatcattaggatatataatgagtaattttaaatcatttaattctgaaaatgaattagatagagatcatttaggatttaaaataatagataataaaacttattactatgatgaagatagtaaattagttaaaggattaatcaatataaataattcattattctattttgatcctatagaatttaacttagtaactggatggcaaactatcaatggtaaaaaatattattttgatataaatactggagcagctttaactagttataaaattattaatggtaaacacttttattttaataatgatggtgtgatgcagttgggagtatttaaaggacctgatggatttgaatattttgcacctgccaatactcaaaataataacatagaaggtcaggctatagtttatcaaagtaaattcttaactttgaatggcaaaaaatattattttgataataactcaaaagcagtcactggatggagaattattaacaatgagaaatattactttaatcctaataatgctattgctgcagtcggattgcaagtaattgacaataataagtattatttcaatcctgacactgctatcatctcaaaaggttggcagactgttaatggtagtagatactactttgatactgataccgctattgcctttaatggttataaaactattgatggtaaacacttttattttgatagtgattgtgtagtgaaaataggtgtgtttagtacctctaatggatttgaatattttgcacctgctaatacttataataataacatagaaggtcaggctatagtttatcaaagtaaattcttaactttgaatggtaaaaaatattactttgataataactcaaaagcagttaccggattgcaaactattgatagtaaaaaatattactttaatactaacactgctgaagcagctactggatggcaaactattgatggtaaaaaatattactttaatactaacactgctgaagcagctactggatggcaaactattgatggtaaaaaatattactttaatactaacactgctatagcttcaactggttatacaattattaatggtaaacatttttattttaatactgatggtattatgcagataggagtgtttaaaggacctaatggatttgaatattttgcacctgctaatacggatgctaacaacatagaaggtcaagctatactttaccaaaatgaattcttaactttgaatggtaaaaaatattactttggtagtgactcaaaagcagttactggatggagaattattaacaataagaaatattactttaatcctaataatgctattgctgcaattcatctatgcactataaataatgacaagtattactttagttatgatggaattcttcaaaatggatatattactattgaaagaaataatttctattttgatgctaataatgaatctaaaatggtaacaggagtatttaaaggacctaatggatttgagtattttgcacctgctaatactcacaataataacatagaaggtcaggctatagtttaccagaacaaattcttaactttgaatggcaaaaaatattattttgataatgactcaaaagcagttactggatggcaaaccattgatggtaaaaaatattactttaatcttaacactgctgaagcagctactggatggcaaactattgatggtaaaaaatattactttaatcttaacactgctgaagcagctactggatggcaaactattgatggtaaaaaatattactttaatactaacactttcatagcctcaactggttatacaagtattaatggtaaacatttttattttaatactgatggtattatgcagataggagtgtttaaaggacctaatggatttgaatactttgcacctgctaatacggatgctaacaacatagaaggtcaagctatactttaccaaaataaattcttaactttgaatggtaaaaaatattactttggtagtgactcaaaagcagttaccggactgcgaactattgatggtaaaaaatattactttaatactaacactgctgttgcagttactggatggcaaactattaatggtaaaaaatactactttaatactaacacttctatagcttcaactggttatacaattattagtggtaaacatttttattttaatactgatggtattatgcagataggagtgtttaaaggacctgatggatttgaatactttgcacctgctaatacagatgctaacaatatagaaggtcaagctatacgttatcaaaatagattcctatatttacatgacaatatatattattttggtaataattcaaaagcggctactggttgggtaactattgatggtaatagatattacttcgagcctaatacagctatgggtgcgaatggttataaaactattgataataaaaatttttactttagaaatggtttacctcagataggagtgtttaaagggtctaatggatttgaatactttgcacctgctaatacggatgctaacaatatagaaggtcaagctatacgttatcaaaatagattcctacatttacttggaaaaatatattactttggtaataattcaaaagcagttactggatggcaaactattaatggtaaagtatattactttatgcctgatactgctatggctgcagctggtggacttttcgagattgatggtgttatatatttctttggtgttgatggagtaaaagcccctgggatatatggctaaaatatatgtttgataaaaaattattcctgtgctactaagaaattatttttatataataaatattgagatttaattaaaagtcatgtgttattgtaatacatgacttttagttaaaatttttctatcatttaataatctattattcttgactattttataataaaattcatatatggaaatattaatactaaataattaatagttgataaaaaatagataatatgctaaaagcaaaaactaatttagagccttgtaactgtttatttgcaattataaaaacatctttaaacatattgactataatataaaatattaactataatacaaaacaatattaattaattttctctacagctatccctggtatagttatatttccacccatagttgattcataagttatagttccagcacttatacctcttatagttatgtaatcatcctctaatactcttgaaggagttattgattttttataactacatagtacaaccttatcataatttccagacacagctaatcttatttgcacctcatcaccatcttcaataacttgaataaccttaccttcaaatttaccttttgtactataatcatcaggtgttctagctaattggtcataagtaataccagtatcatatcctttcttctcctcttcttcttttttgcgttgttcttcagcctttttagcttcttcagcttttttagcttcttcagctttacgttgattttcagcttcaatagctttcttttcgtcgtctttcattttgaaccatggttcagcatcagacaatttgctatttaaagtttctatttctgttttttgagaatctataactgatgtttggttagaaatgacctcctcatggtcttcagaacaagctggtgaggatatattgccaaaaaacacgcctaaaataaatgccagtagagcaataccctttgtgctcttaaagaatttaattattttcttagagcttccttttccttcattactaaattcgttaccctcattttttttagaaaacataatacaatctcccttttattagatatattttattttaaaagttaaaaacttaaaataactagttgactaaaaattatatattcatattttcctaaaatatatttcccctaagcataattttacaaaataaagtaagaagattcaatatattttgaaaaaataagataaaaatgtcagattataatataattttcttgaaggtgaattttatatattaaattaaacataaagtattttatttgtataaaactatattatgatgtaattaagtgactcagtgatttagaggtggtaaaatatatatatatgaaagagcataaataaattgatataataaaaaattaaatattaaatattaactataataaaaaaatatctggtaataggtataatataaaaagaatataccagaaagaaggtgaagtatgggagaactacaaaaaattccaggggtagggaaagcaacagaaaaatctttaatcatgttaggatatacaactattaaatcacttaaagatgcaaacccagcacaaatgtatgaaaaggaatgtttaatgcgtggacagcacatagacagatgtcagttatatgtatacagatgtgcagtatattttgcatcaactgaaaatccagaaccagaaaaattaaagtggtggtattggaaagattaaaaaatcaaaaaagttagacataaaaaagagttgaatatccgttttaaataataaaaactaatactcaactcttttttagtcgtaaattttatgtaaatctatttgtatggctaaatatacccatcaataaatgtataaatataccaatcaacaaatgactaaacatactacctaacaaaggattaaataaattacttaacaaagcattctaaaacaattaattagaaactgtttcttcaagccattttctacattgctcaatatttaccatagggtcaaaaccttggtcttttcccttatttaaaagcatatcacaagggaaagtatcacattcaccacaatgattaagttccttactttcacagcaagttttaaccttacattctccaccccaaaatggtttttccatagttgggcaaccagtgcaatttacttgttctttttttgtacaactgtcacaacagacaccacatcttgattcaaacatgttcaaacatcctttccattatttaaaaatattataaaatgattttagatgaatacaaaagtgcaaatagttgattttaggtcatctaaatgttaaacataaagttattagtactggtaaatttataaaaactattccaaaaatctttttgaatatttcaaaacacaataaattacttcaaatccctttgaatatattttacagcattatagattgctttaaatctctttgaatattctacaagactatagattagtttaaatctctttgagtattctacaagactatagattagtttaaatccctttgaatatttcaaaacaccatagattactttaaattcctttgaatattctataacactataaattacttttaacttttatataaccataaagtttttatctggcactttaaatggagttttatatcaaatttgccttccatcgaataaccaaacttaatttaattacacattccaagagtcaaatattcattcaatatatttgataattctatgttatagctataattaaatatagattattaaagttaaatatttatttaatatattgaatgattttttacctatatttaattaagtttcattatataatataaaaattgtttttgcattaagttttaatataatacataataattttaaataataatattattatatattttttaattttaggagtatatctattatatagcgagtagataaaacatataaaattcaaataaaagatatatatttttaaattaaaatggatatagatttcaactaaaaagaatataaatttcaaacccaaaaatatctagcatttaccattaagaaataacatcattctttctaaaatttctattggcaatttcagaaaatactatagtagtaataaatgcaacacatattgtaactatagtgtcattaacatttaaagcagattgctttataacccccatacgactacctaacatagaataagggaaaaatataccaacagcaggttttgctactattaatcccataccaaatagagaaaggcaaagactaataccaataggagttgcaaaacttctaatctttatagacatgtataattgtatagaagctattgaaatagaaataatccaacctttagcaatccaaccagtcaattctttaggtacactaccagaaaaaccaaacatatttcctgcaactatataaaagataacaaagaaaacttgtgtaatagctgtaagtattgaaactactgtaagtttagataaaaagatattttttaaattaactggcagtgtcattacattattccaattatgattcatatgttcaagcctacaaatatatgcacaaaagattgcgattaagataggaaagaaaaattccccataaaaaagactaacttgagtccataagctgtaccattcttttttgagtatgccttgatttagataaaaattaccagaaccaatcaacacacttataagtggcaaagctagtaatacataccatataaaagaattttttaactttagaatttctcccaaaactgacttccttaacatttaaatccctcctatacttctttttttaataaatgatttcttccaatataataaattagcattccaattaagaaaactaaaatcgtaatagaaaaattcatatcaattctatagacagatgaacctaaaacattatcataagcataacttaaaggtgataactctaggtaataagaccatataaacaatctacgaataccttgataaaacaaacctgatgtcaaacctataaaactaccaatcatgccaaatgtaattgcaatcatttgatttggaattacagttgcaatccataggtgtagtgcaatgatagcaatacttacaagaattgttcctaatgtgtattttaaaagtaaagatacagaaattgactcaataacccctctaaaatgtccaaacaacacaatagataacacttgcatcaatacaggtatagataccaaaatagcagaacataaaaatttagataaataaatagtatttaaagatgtcacagaagattttaaaagcttccatgtatctcctttatgttctatatcgcttatacgtgatgtaattattgatattaagataggaaagaatagaccatttaaacttgcaaaactcataagcatataggaatattcaaatccacctaacatatctggattacgtgtaatagccctatttgaatttacgatacaccacattatttcaacagctacaaataaaaaggtcatcagaataatcttctttcttttaagtttataaaattctagaccaaggtatttcattataaagtcaccgccttaccagtaattctaagaatatatcttccaagctttttttatgttcttctattctaaatacatctatatttgaatggacaagcataccatttattttagcgacatctgagtcttttaaattttcaatagtcaagtacccatcttgtataagtgacatatatcctttagtatttaatagtttttgtgcagatacaacattcttagttttgatagcaatctgactttgacctctattatgaagttcttttatgctatcttgaaaaaccagttcgccatgatttattattcctattgatgtggcaatttggtcaatttcacttaaaagatggctagagattagaacagtcatcccgtatttttctggtagagattttattaattctctaatttcctcaatccctgctgggtcgagtccatttgtaggttcatcaagtattaataatttgggaaacttcattattgccatagcaatgccaagacgttgcttcatacctaaagaatattgactaacttttttatttttttgattttctaaccttacaatttttaatgcttcatttacattttttttaggtaaatctaagagtctttgcattatggtcatgttttcaagccctgtaagatgaccatagtatgatggagattctatcaaagaacctatatcttttaaaattgatattctatttttttcatttaactctttacctaaaatattaatatttccttgtgtgggtttagcaagtccaagaagcattttaagagtggtagattttccagctccattaggacccaaaaaaccatatacagctccttgtggaactcttaggtctatatcctttactctaaatattttattgtattcctttgaaagtctttgtgttctaattatcatttccatatgtttcatccccttttttaatctgtgcttattgattcttttaacttatatcagtataataacttggttacatttcaattagctgaaatttaccttacaataaccttaaaagtctatttaggcaaagttgtgaaaatgggtatatggtatac

SEQ ID NO: 260 - DNA, 5106 bp, Clostridium difficile
  misc_feature 1..5106: note = C difficile toxins B & A and utxA genes
  source 1..5106: mol_type = other DNA
agctgatgctttaataacaacattaaaaccaagatatgaagatactaatataagaataaatttagatagtaatactagaagttttatagttccaataataactacagaatatataagagaaaaattatcatattctttctatggttcaggaggaacttatgcattgtctctttctcaatataatatgggtataaatatagaattaagtgaaagtgatgtttggattatagatgttgataatgttgtgagagatgtaactatagaatctgataaaattaaaaaaggtgatttaatagaaggtattttatctacactaagtattgaagagaataaaattatcttaaatagccatgagattaatttttctggtgaggtaaatggaagtaatggatttgtttctttaacattttcaattttagaaggaataaatgcaattatagaagttgatttattatctaaatcatataaattacttatttctggcgaattaaaaatattgatgttaaattcaaatcatattcaacagaaaatagattatataggattcaatagcgaattacagaaaaatataccatatagctttgtagatagtgaaggaaaagagaatggttttattaatggttcaacaaaagaaggtttatttgtatctgaattacctgatgtagttcttataagtaaggtttatatggatgatagtaagccttcatttggatattatagtaataatttgaaagatgtcaaagttataactaaagataatgttaatatattaacaggttattatcttaaggatgatataaaaatctctctttctttgactctacaagatgaaaaaactataaagttaaatagtgtgcatttagatgaaagtggagtagctgagattttgaagttcatgaatagaaaaggtaatacaaatacttcagattctttaatgagctttttagaaagtatgaatataaaaagtattttcgttaatttcttacaatctaatattaagtttatattagatgctaattttataataagtggtactacttctattggccaatttgagtttatttgtgatgaaaatgataatatacaaccatatttcattaagtttaatacactagaaactaattatactttatatgtaggaaatagacaaaatatgatagtggaaccaaattatgatttagatgattctggagatatatcttcaactgttatcaatttctctcaaaagtatctttatggaatagacagttgtgttaataaagttgtaatttcaccaaatatttatacagatgaaataaatataacgcctgtatatgaaacaaataatacttatccagaagttattgtattagatgcaaattatataaatgaaaaaataaatgttaatatcaatgatctatctatacgatatgtatggagtaatgatggtaatgattttattcttatgtcaactagtgaagaaaataaggtgtcacaagttaaaataagattcgttaatgtttttaaagataagactttggcaaataagctatcttttaactttagtgataaacaagatgtacctgtaagtgaaataatcttatcatttacaccttcatattatgaggatggattgattggctatgatttgggtctagtttctttatataatgagaaattttatattaataactttggaatgatggtatctggattaatatatattaatgattcattatattattttaaaccaccagtaaataatttgataactggatttgtgactgtaggcgatgataaatactactttaatccaattaatggtggagctgcttcaattggagagacaataattgatgacaaaaattattatttcaaccaaagtggagtgttacaaacaggtgtatttagtacagaagatggatttaaatattttgccccagctaatacacttgatgaaaacctagaaggagaagcaattgattttactggaaaattaattattgacgaaaatatttattattttgatgataattatagaggagctgtagaatggaaagaattagatggtgaaatgcactattttagcccagaaacaggtaaagcttttaaaggtctaaatcaaataggtgattataaatactatttcaattctgatggagttatgcaaaaaggatttgttagtataaatgataataaacactattttgatgattctggtgttatgaaagtaggttacactgaaatagatggcaagcatttctactttgctgaaaacggagaaatgcaaataggagtatttaatacagaagatggatttaaatattttgctcatcataatgaagatttaggaaatgaagaaggtgaagaaatctcatattctggtatattaaatttcaataataaaatttactattttgatgattcatttacagctgtagttggatggaaagatttagaggatggttcaaagtattattttgatgaagatacagcagaagcatatataggtttgtcattaataaatgatggtcaatattattttaatgatgatggaattatgcaagttggatttgtcactataaatgataaagtcttctacttctctgactctggaattatagaatctggagtacaaaacatagatgacaattatttctatatagatgataatggtatagttcaaattggtgtatttgatacttcagatggatataaatattttgcacctgctaatactgtaaatgataatatttacggacaagcagttgaatatagtggtttagttagagttggggaagatgtatattattttggagaaacatatacaattgagactggatggatatatgatatggaaaatgaaagtgataaatattatttcaatccagaaactaaaaaagcatgcaaaggtattaatttaattgatgatataaaatattattttgatgagaagggcataatgagaacgggtcttatatcatttgaaaataataattattactttaatgagaatggtgaaatgcaatttggttatataaatatagaagataagatgttctattttggtgaagatggtgtcatgcagattggagtatttaatacaccagatggatttaaatactttgcacatcaaaatactttggatgagaattttgagggagaatcaataaactatactggttggttagatttagatgaaaagagatattattttacagatgaatatattgcagcaactggttcagttattattgatggtgaggagtattattttgatcctgatacagctcaattagtgattagtgaatagataaaaatatgttaaatatatcctcttatacttaaatatataaaaataaacaaaatgatacactacataaagtgttctatctaatatgaagatttaccaataaaaaggtggactatgatgaatgcacagtagttcacctttttatatttctaatggtaacaaaatatttttttatataaacctaggaggcgttatgaatatgacaatatcttttttatcagagcatatatttataaagttagtaatttctaactatatcatttgatacattattaggatgtttaagtgcaataaaaagtcgtaaatttaattctagttttggaatagatggaggaatcagaaaagtagcaatgatagcatgtatattttttttatcagtagttgacattcttacaaagtttaactttttatttatgttaccacaagattgtatcaattttttaagactaaaacatcttggaatatctgaatttttctctattttatttattttatatgaaagtgtaagtatattaaaaaatatgtgcttatgtggattaccagtacctaagagattaaaggaaaaaatagcaattttactagatgcaatgacagatgaaatgaatgctaaggatgaaaagtaagtaatggtagatataataaagatattaacaaataaaaagtgttatccaaataagaatagctgaaagttatcataattcatgaaactaataatgaaaacgagggagcagatgccaagagacacacaagtattaaatacatataatttcgaagcaagtgttcattactatatagatgacaaggtagtatatcaaacattggttcacaaagatggtgcatggtcagttggtaaaatctattaagctacattagttacagatatcacaaactataatagttaaacatagaaatatgtgtaaattgtgatggaaattattcaaaaacacaaaaatacgtgatgaaggacaaaatgatatagaaaataagtatcaaaccttaataaatgatttaattgatagtttaaaagttataggaaaaatatataaagaaataaaaacattaaaaaaatataagatatgtttacaaattactatcagacaatctccttatctaatagaagagtcaattaactaattgagtatctttaaattgaaatgttaggaagtgatttaaatatgaaaacttaaattataaaaaatcaatattaatttatttttaaaaaatagaaaggagtgtataagatttattttcaaagtttaaaaacaagaaaatcaatttaaatttcagaaggaataaatgtggttatagaagtggatttattatcaaaaataataatactaggaggtttttatgtctttaatatctaaagaagagttaataaaactcgcatatagcattagaccaagagaaaatgagtataaaactatactaactaatttagacgaatataataagttaactacaaacaataatgaaaataaatatttgcaattaaaaaaactaaatgaatcaattgatgtttttatgaataaatataaaacttcaagcagaaatagagcactctctaatctaaaaaaagatatattaaaagaagtaattcttattaaaaattccaatacaagccctgtagaaaaaaatttacattttgtatggataggtggagaagtcagtgatattgctcttgaatacataaaacaatgggctgatattaatgcagaatataatattaaactgtggtatgatagtgaagcattcttagtaaatacactaaaaaaggctatagttgaatcttctaccactgaagcattacagct

SEQ ID NO: 261 - protein, 899 aa, Escherichia coli
  REGION 1..899: note = Escherichia coli Cas3
MRKYPLSLLKDKNIVTFFDFWGKTRRGEKEGGDGYHLLCWHSLDVAAMGYLMVKRNCFGLADYFRQLGISDKEQAAQFFAWLLCWHDIGKFARSFQQLYLAPELKIPEGSRKNYEKISHSTLGYWLWNYYLSECEELLPSSSLSSRKLTRVIEMWMSITTGHHGRPPDRIDELDNFLPEDKAAARDFLLEIKALFPLIEIPTFWDDDEGVELLKQLSWYISATVVLADWTGSSTRFFPRVAHPMDIKDYWQKTLVQAQNALTVFPPKAETAPFTGINTLFPFIEHPTPLQQKVLDLDISQPGPQLFILEDVTGAGKTEAALILAHRLMAARKAQGLFFGLPTMATANAMYDRLVKTWLAFYSPESRPSLVLAHSARTLMDRFNESLWSGDLVGSEEPDEQTFSQGCAAWFANSNKKALLAEIGVGTLDQAMMAVMPFKHNNLRLLGLSNKILLADEIHACDAYMSCILEGLIERQARGGNSVILLSATLSQQQRDKLVAAFARGTEGQQEAPFLEKDDYPWLTHVTKSDVNSHRVATRKDVERSVSVGWLHSEQESIARIESAVSQGKCIAWIRNSVDDAIKVHRQLLARGVIPASSLSLFHSRFAFSDRQRIEMETLARFGKEDGSQRAGKVLICTQVLEQSVDCDLDEMISDLAPVDLLIQRAGRLQRHIRDINGQLKRDGKDERSPPELLILAPVWDDAPGDEWFGSAMRNSAYVYPDHGRIWLTQRVLREQGAIQMPHAARLLIESVYGEDVVMPEGFARSEQEQVGKYYCDRAMAKKFVLNFKPGYAANINDYLPEKLSTRLAEESVSLWLATCIAGVVKPYATGAHAWEMSVVRVRRSWWKKHRDEFSLLEGEAFRQWCIEQRQDPEMANVILVTDDESCGYSAREGLIGKVD

SEQ ID NO: 262 - DNA, 2700 bp, Escherichia coli
  misc_feature 1..2700: note = Escherichia coli Cas3 nucleotide sequence
  source 1..2700: mol_type = other DNA
atgcgtaaatatcctttaagtttactgaaggataaaaatattgtgactttctttgatttctggggaaaaacccgacgtggcgagaaagagggtggcgacggctatcaccttctttgctggcattcgctggatgtggccgcaatgggctatttaatggttaaaagaaattgcttcgggctggctgattactttcgtcaattagggatttctgacaaggaacaggcggctcaatttttcgcttggttgctgtgctggcacgatattggaaaatttgcccgctcttttcagcaactttacctggcccctgaactcaagattccggaaggttccagaaagaattacgaaaagatctctcattcaacgctgggttactggctgtggaattattatttaagtgaatgtgaggagttgcttccttcatcttcactctcttctcgtaaacttacacgtgtaatagagatgtggatgtccataactaccgggcatcatggtcgaccacctgaccgtattgatgagctggataattttctgcctgaagacaaagctgccgcgcgagattttctccttgaaatcaaggcactgtttccgctcatagagattcccacattctgggatgatgacgagggcgttgaacttttaaaacaactttcctggtatatctctgcaacagtcgtactcgcagactggacgggttcgtcaacgcgattttttccacgcgtcgcacacccaatggatattaaagattactggcagaaaactttagttcaggctcaaaacgccttaaccgtctttcctccaaaagcagaaaccgcacctttcaccggaattaatacgctgtttccttttattgagcacccgacaccattacagcaaaaggtactggatctggatatcagccagccagggccacagttatttattctggaagacgtgactggcgcaggtaaaacagaagcggcgcttatcctggcgcacaggttgatggctgcgaggaaagcacagggtttgttttttggcctgccaacaatggcaacggccaatgccatgtacgatcggctggtcaaaacctggcttgctttctattcgccagagtcccgccccagcttggtgctggcacacagtgcccgcacattaatggaccgcttcaatgaatcactctggtccggtgatttagtcgggtcagaagaaccggatgaacaaacattcagtcagggatgtgcggcctggtttgccaacagtaacaagaaggcgctactggctgaaattggcgtcggcacgctggatcaggcgatgatggcagtgatgccgtttaaacataataatctgcggcttctggggttgagtaacaaaatcctgctggctgatgagatccatgcctgtgatgcttacatgtcgtgcattcttgaagggctgatcgagcggcaggcgcgtggcggaaacagcgtcattttgctttctgctacgttatcccaacagcagcgcgacaaactcgtcgccgcctttgcgcgtggcacagagggccagcaagaagctccgttccttgaaaaggatgattacccctggctgacgcatgtcacgaaatccgatgtgaactcacaccgggtagcgacgcgcaaagacgttgagcgtagcgtcagcgtgggttggcttcatagtgaacaagagagtattgcgcgtatcgaatcggcggtaagtcagggaaaatgcatcgcctggatccggaattctgtcgatgacgctattaaggttcatcgtcagctgcttgcccgcggcgtcattcccgcttccagcctttcactctttcatagccgctttgcttttagcgatcgccagcgaattgaaatggagacgctggcacgctttggtaaagaagacggttcacagcgtgccggaaaagtcctcatttgtactcaggtcttagagcagagcgttgattgtgacctggacgaaatgatctccgacctggcccctgttgatttgctgattcagcgagcggggcgattacagcggcatatccgcgatattaatggtcagttaaagcgtgacggaaaagacgagcgttcccctcctgaattgctgattctggcccccgtctgggacgacgctcctggtgacgaatggttcggcagtgccatgcgtaacagtgcatatgtctatcccgatcatggacgaatctggctgacgcagcgtgtactgcgtgagcaaggcgctattcaaatgccacacgcagcccgccttcttattgaatcagtctacggtgaggacgtggtaatgccggaaggatttgcccgcagcgagcaggagcaagtgggcaaatattactgcgatcgcgcaatggctaaaaagtttgtcctgaacttcaagcctggctatgccgccaatatcaacgattaccttccggaaaagctgtcgacacgtctggctgaggaatctgtttccctgtggctggctacctgtattgccggtgtggtgaagccttatgccaccggtgctcacgcatgggaaatgagcgttgtcagagtgcgtcgaagctggtggaaaaaacatcgggatgagttttctttactggaaggggaagcgttcaggcagtggtgcattgaacagcggcaagatccggaaatggcaaacgtgattttagtcactgatgacgaaagttgcgggtattcggccagggagggattgattggcaaggttgattga

SEQ ID NO: 263 - protein, 888 aa, Escherichia coli
  REGION 1..888: note = Escherichia coli Cas3
MEPFKYICHYWGKSSKSLTKGNDIHLLIYHCLDVAAVADCWWDQSVVLQNTFCRNEMLSKQRVKAWLLFFIALHDIGKFDIRFQYKSAESWLKLNPATPSLNGPSTQMCRKFNHGAAGLYWFNQDSLSEQSLGDFFSFFDAAPHPYESWFPWVEAVTGHHGFILHSQDQDKSRWEMPASLASYAAQDKQAREEWISVLEALFLTPAGLSINDIPPDCSSLLAGFCSLADWLGSWTTTNTFLFNEDAPSDINALRTYFQDRQQDASRVLELSGLVSNKRCYEGVHALLDNGYQPRQLQVLVDALPVAPGLTVIEAPTGSGKTETALAYAWKLIDQQIADSVIFALPTQATANAMLTRMEASASHLFSSPNLILAHGNSRFNHLFQSIKSRAITEQGQEEAWVQCCQWLSQSNKKVFLGQIGVCTIDQVLISVLPVKHRFIRGLGIGRSVLIVDEVHAYDTYMNGLLEAVLKAQADVGGSVILLSATLPMKQKQKLLDTYGLHTDPVENNSAYPLINWRGVNGAQRFDLLAHPEQLPPRFSIQPEPICLADMLPDLTMLERMIAAANAGAQVCLICNLVDVAQVCYQRLKELNNTQVDIDLFHARFTLNDRREKENRVISNFGKNGKRNVGRILVATQVVEQSLDVDFDWLITQHCPADLLFQRLGRLHRHHRKYRPAGFEIPVATILLPDGEGYGRHEHIYSNVRVMWRTQQHIEELNGASLFFPDAYRQWLDSIYDDAEMDEPEWVGNGMDKFESAECEKRFKARKVLQWAEEYSLQDNDETILAVTRDGEMSLPLLPYVQTSSGKQLLDGQVYEDLSHEQQYEALALNRVNVPFTWKRSFSEVVDEDGLLWLEGKQNLDGWVWQGNSIVITYTGDEGMTRVIPANPK

SEQ ID NO: 264 - DNA, 2667 bp, Escherichia coli
  misc_feature 1..2667: note = Escherichia coli Cas3 Nucleotide sequence
  source 1..2667: mol_type = other DNA
atggaaccttttaaatatatatgccattactggggaaaatcctcaaaaagcttgacgaaaggaaatgatattcatctgttaatttatcattgccttgatgttgctgctgttgcagattgctggtgggatcaatcagtcgtactgcaaaatactttttgccgaaatgaaatgctatcaaaacagagggtgaaggcctggctgttatttttcattgctcttcatgatattggaaagtttgatatacgattccaatataaatcagcagaaagttggctgaaattaaatcctgcaacgccatcacttaatggtccatcaacacaaatgtgccgtaaatttaatcatggtgcagccggtctgtattggtttaaccaggattcactttcagagcaatctctcggggattttttcagtttttttgatgccgctcctcatccttatgagtcctggtttccatgggtagaggccgttacaggacatcatggttttatattacattcccaggatcaagataagtcgcgttgggaaatgccagcttctctggcatcttatgctgcgcaagataaacaggctcgtgaggagtggatatctgtactggaagcattatttttaacgccagcggggttatctataaacgatataccacctgattgttcatcactgttagcaggtttttgctcgcttgctgactggttaggctcctggactacaacgaatacctttctgtttaatgaggatgcgccttccgacataaatgctctgagaacgtatttccaggaccgacagcaggatgcgagccgggtattggagttgagtggacttgtatcaaataagcgatgttatgaaggtgttcatgcactactggacaatggctatcaacccagacaattacaggtgttagttgatgctcttccagtagctcccgggctgacggtaatagaggcacctacaggctccggtaaaacggaaacagcgctggcctatgcttggaaacttattgatcaacaaattgcggatagtgttatttttgccctcccaacacaagctaccgcgaatgctatgcttacgagaatggaagcgagcgcgagccacttattttcatccccaaatcttattcttgctcatggcaattcacggtttaaccacctctttcaatcaataaaatcacgcgcgattactgaacaggggcaagaagaagcgtgggttcagtgttgtcagtggttgtcacaaagcaataagaaagtgtttcttgggcaaatcggcgtttgcacgattgatcaggtgttgatatcggtattgccagttaaacaccgctttatccgtggtttgggaattggtcgaagtgttttaattgttgatgaagttcatgcttacgacacctatatgaacggcttgctggaggcagtgctcaaggctcaggctgatgtgggagggagtgttattcttctttccgcaaccctaccaatgaaacaaaaacagaaacttctggatacttatggtctgcatacagatccagtggaaaataactccgcatatccactcattaactggcgaggtgtgaatggtgcgcaacgttttgatctgctagctcatccagaacaactcccgccccgcttttcgattcagccagaacctatttgtttagctgacatgttacctgaccttacgatgttagagcgaatgatcgcagcggcaaacgcgggtgcacaggtctgtcttatttgcaatttggttgacgttgcacaagtatgctaccaacggctaaaggagctaaataacacgcaagtagatatagatttgtttcatgcgcgctttacgctgaacgatcgtcgtgaaaaagagaatcgagttattagcaatttcggcaaaaatgggaagcgaaatgttggacggatacttgtcgcaacccaggtcgtggaacaatcactcgacgttgattttgattggttaattactcagcattgtcctgcagatttgcttttccaacgattgggccgtttacatcgccatcatcgcaaatatcgtcccgctggttttgagattcctgttgccaccattttgctgcctgatggcgagggttacggacgacatgagcatatttatagcaacgttagagtcatgtggcggacgcagcaacatattgaggagcttaatggagcatccttatttttccctgatgcttaccggcaatggctggatagcatttacgatgatgcggaaatggatgagccagaatgggtcggcaatggcatggataaatttgaaagcgccgagtgtgaaaaaaggttcaaggctcgcaaggtcctgcagtgggctgaagaatatagcttgcaggataacgatgaaaccattcttgcggtaacgagggatggggaaatgagcctgccattattgccttatgtacaaacgtcttcaggtaaacaactgctcgatggccaggtctacgaggacctaagtcatgaacagcagtatgaggcgcttgcacttaatcgcgtcaatgtacccttcacctggaaacgtagtttttctgaagtagtagatgaagatgggttactttggctggaagggaaacagaatctggatggatgggtctggcagggtaacagtattgttattacctatacaggggatgaagggatgaccagagtcatccctgcaaatcccaaataa

SEQ ID NO: 265 - protein, 926 aa, Streptococcus thermophilus
  REGION 1..926: note = Streptococcus thermophilus Cas3
MKHINDYFWAKKTEENSRLLWLPLTQHLEDTKNIAGLLWEHWLSEGQKVLIENSINVKSNIENQGKRLAQFLGAVHDIGKATPAFQTQKGYANSVDLDIQLLEKLERAGFSGISSLQLASPKKSHHSIAGQYLLSHYGVDEDIATIIGGHHGRPVDDLDGLNSQKSYPSNYYQDEKKDSLVYQKWKSNQEAFLNWALTETGFNSVSQLPKIKQPAQVILSGLLIMSDWIASNEHFFPLLSLDETDVKNKSQRIETGFKKWKKSNLWQPETFVDLVTLYQERFGFSPRNFQLILSQTIEKTTNPGIVILEAPMGIGKTEAALAVSEQLSSKKGCSGLFFGLPTQATSNGIFKRIEQWTENIKGNNSDHFSIQLVHGKAALNTDFIELLKGNTINMDDSENGSIFVNEWFSGRKTSALDDFVVGTVDQFLMVALKQKHLALRHLGFSKKVIVIDEVHAYDAYMSQYLLEAIRWMGAYGVPVIILSATLPAQQREKLIKSYMAGMGVKWRDIENIDQIKIDAYPLITYNDGPDIHQVKMFEKQEQKNIYIHRLPEEQLFDIVKEGLDNGGVVGIIVNTVRKSQELARNFSDIFGDDMVDLLHSNFIATERIRKEKDLLQEIGKKAIRPPKKIIIGTQVLEQSLDIDFDVLISDLAPMDLLIQRIGRLHRHKIKRPQKHEVARFYVLGTFEEFDFDEGTRLVYGDYLLARTQYFLPDKIRLPDDISPLVQKVYNSDLTITFPKPELHKKYLDAKIEHDDKIKNKETKAKSYRIANPVLKKSRVRTNSLIGWLKNLHPNDSEEKAYAQVRDIEDTVEVIALKKISDGYGLFIENKDISQNITDPIIAKKVAQNTLRLPMSLSKAYNIDQTINELERYNNSHLSQWQNSSWLKGSLGIIFDKNNEFILNGFKLLYDEKYGVTIERLDKNESV

SEQ ID NO: 266 - DNA, 2781 bp, Streptococcus thermophilus
  misc_feature 1..2781: note = Streptococcus thermophilus Cas3
  source 1..2781: mol_type = other DNA
atgaaacatattaatgattatttttgggctaagaaaacagaggaaaatagtagacttctttggttaccattaactcaacacttagaagacacgaaaaatattgcaggcctcttatgggaacattggttaagtgaaggacaaaaggtattaattgaaaattctattaatgttaaatcaaatattgaaaaccaagggaaaagattggcacaattcctaggagctgttcatgatatcggtaaagcaacaccagcttttcagacgcaaaaaggttatgcaaattcagtagatttggatattcaattgttagaaaaattggaacgcgcaggtttttctggcattagttctctccaactagcctcccccaaaaagagtcatcatagcattgcaggtcaatatttgttatcccattatggcgtggacgaagatattgcaacaattattggtggacaccatggacgaccagttgatgatttagacggtttaaattctcaaaaaagctatccctccaattattaccaggatgaaaagaaagatagtctcgtttatcagaaatggaagtcaaatcaagaagcttttttaaactgggctttaacagaaacagggtttaattctgtgtctcagcttccaaaaatcaaacagcctgctcaagttattctatcaggtttactcataatgtctgactggattgctagtaatgagcatttttttcctttgttaagtttggatgaaactgatgtgaaaaacaagagtcaacgtattgaaactgggtttaaaaagtggaaaaaatctaacttgtggcaacctgaaactttcgttgaccttgttactctttatcaggaaagatttggatttagtccacgaaattttcagctgatactctcacaaacaatcgaaaagacgactaatcctgggatagtgatactggaagcgccaatgggaatcgggaaaacagaggcggctctagcggtatcagagcagttatctagtaaaaaaggatgtagtggattgttttttggattgcccacacaagcaacctccaatggaatttttaagaggattgaacagtggacagagaatataaagggtaacaattctgatcatttttccattcagctggttcatggaaaagcagccttaaatacggattttattgagttacttaaaggaaatacaattaatatggacgactcggaaaacggcagtatttttgtcaatgagtggttttctgggagaaaaacttcagcattagatgattttgtagttgggacggtcgaccaatttttaatggtggctttaaaacaaaaacatttggccttacgtcatttaggatttagtaaaaaagttatcgttattgatgaagtccacgcttatgatgcttatatgagccaatatttgttggaagctatcagatggatgggagcttatggtgttcctgtaattattttatcagcaactttacctgcccaacaaagagaaaaactcataaaaagctatatggctggaatgggagtgaaatggcgagatattgaaaatatagatcagataaaaatagacgcataccctttaatcacttataatgacgggcctgacattcatcaagttaaaatgttcgaaaagcaagaacaaaaaaatatctacattcatcgtttaccagaagaacagttatttgatattgtaaaagaaggtcttgacaatggtggagtagttgggataattgtcaatacggtgagaaaatctcaagaattggcaagaaatttttcagatatttttggagatgatatggtagatttgcttcattctaatttcatagcaactgaaagaatccgaaaagaaaaggatttattgcaagaaattgggaaaaaagcaatacgtccaccaaagaaaatcattattggtacacaggtgcttgaacagtcgttagatattgattttgatgtactgataagcgacttagcgcctatggatttactcattcaacgtatcggacgactacatcgtcacaaaatcaaaaggccccaaaagcacgaagtagcaagattttatgttttaggaacatttgaagagtttgattttgatgaaggaacgcgtttggtttatggggactacctattagctagaactcagtactttttaccagataaaatacgacttcctgatgatatttcaccgctagtccaaaaggtttataattcagacctaacaattacgtttccaaagccagaacttcataaaaaatatttggatgctaaaatagaacatgatgataagattaaaaataaagaaacaaaggcaaagtcataccgtattgctaatcctgtcttaaaaaaatcgagagttcgaactaacagtttgattggttggttaaagaacctccatccaaatgatagtgaagaaaaagcatatgctcaagttcgagatattgaagatacagttgaagtgattgcattaaaaaaaatatctgatgggtatggtttgttcatagaaaataaagatatatctcagaacattactgatcctataattgcaaaaaaggtagcacaaaatactttacgacttccgatgagtttatccaaagcctataatattgatcaaacgattaatgagcttgaaagatataacaatagccacttaagtcaatggcaaaactcatcatggttaaagggatctcttgggattatttttgataaaaacaatgagtttatactgaatggatttaaactattatatgatgaaaaatatggtgttaccatagaaaggttggataagaatgagtcggtttaa

SEQ ID NO: 267 - protein, 887 aa, Salmonella enterica subsp. enterica serovar Typhimurium str. LT2
  REGION 1..887: note = Salmonella enterica subsp. enterica serovar Typhimurium LT2 Cas 3
MSIYHYWGKSRRGETDGGDDYHLLCWHSLDVAAVGYWMVINNIYFIDHYLKKLGIQDKEQAAQFFAWILCWHDIGKFAHSFQQLYRHEALNIFNEPTRHYEKIAHTTLGYMLWNSWLSECPELFPPSSLSVRKSKRVMALWMPVTTGHHGRPPEAIQELDHFRQQDKDAARDFLLRIKALFPLITLPEAWDEDEGIDQFQQLSWFISAAVVLADWTGSASRYFPRTAEKMPVDTYWQQALAKAQTAITLFPSAANVSAFTGIETLFPFIQHPTPLQQKALELDINVDGAQLFILEDVTGAGKTEAALILAHRLMAAGKAQGLYFGLPTMATANAMFERMANTWLALYQPDSRPSLILAHSARRLMDRFNQSIWSVTLSGTEEPDEAQPYSQGCAAWFADSNKKALLAEVGVGTLDQAMMAVMPFKHNNLRLLGLSNKILLADEIHACDAWMSRILEGLIERQASNGNATILLSATLSQQQRDKLVAAFSRGVRRSVQAPLLGHDDYPWLTQVTQTELISQRVDTRKEVERCVDIGWLHSEEACLERIGEAVEKGNCIAWIRNSVDDAIRIYRQLQLSKVVVTENLLLFHSRFAFYDRQRIESQTLNLFGKQSGAQRAGKVIIATQVIEQSLDIDCDEMISDLAPVDLLIQRAGRLQRHIRDRNGLVKKSGQDERETPVLRILAPEWDDAPRENWLSSAMRNSAYVYPDHGRMWLTQRILREQGTIRMPQSARLLIESVYGEDVNMPVGFAKTEQLQEGKFYCDRAFAGQMLLNFAPGYCAEISDSLPEKMSTRLAEESVTLWLAKIVDSVVTPYASGEHAWEMSVLRVRQSWWNKHKDEFEKLDGEPLRKWCAQQHQDKDFATVIVVTDFAACGYSANEGLIGMMGE

SEQ ID NO: 268 - DNA, 2664 bp, Salmonella enterica subsp. enterica serovar Typhimurium str. LT2
  misc_feature 1..2664: note = Salmonella enterica subsp. enterica serovar Typhimurium LT2 Cas 3 nucleotide sequence
  source 1..2664: mol_type = other DNA
gtgtcgatatatcactattggggaaagtctcgacgaggagaaactgacggcggtgatgattaccatttgctttgctggcattctttagatgttgcggctgtgggttactggatggtgataaataatatttattttattgaccactatctaaaaaaattaggcatccaggataaggagcaggcggcgcaattttttgcctggattttatgttggcatgatattggaaagtttgctcattccttccagcaactataccgtcatgaggctttaaatatctttaatgagcctacacggcattatgaaaaaatcgcgcataccacgctgggatacatgttgtggaactcctggctaagtgaatgccctgaattgtttcctccttcttcgctttcagttcgtaaaagtaagcgcgttatggcgctttggatgccagtcactacaggtcatcatggacgccctccagaggcaatccaggagctggaccattttcgccagcaggataaagacgcggcaagagattttcttctgagaataaaagcgctctttcctttaattactttgcctgaagcctgggatgaagatgagggtatcgaccaatttcagcaactttcctggtttatttccgctgcggttgtactggctgactggactggttctgccagccgttattttccgcgtactgcggaaaaaatgcctgttgatacctactggcagcaagctctcgctaaagcacaaactgccatcacgctatttccctcagcggcgaatgtgtctgcctttacgggcatagaaacgcttttcccttttattcagcatcccacaccgttacaacaaaaggcgcttgagctggatatcaacgtggatggcgcccaactctttattcttgaagatgtcaccggggccggaaaaacagaggcggcgctcatattagctcatcgactgatggcggcaggtaaagcgcagggactctattttggactgccgacaatggcgacagccaacgcgatgtttgaacgtatggcgaacacctggctggcgctgtatcagccggactcccgtcccagcctgattctggcgcatagcgcgcgtcgcttaatggatcgtttcaatcagtcaatatggtcggtcactctttctggtacggaagaacccgatgaagcgcagccttatagtcagggatgcgccgcctggtttgccgacagcaataaaaaagcgttgttggcggaggttggcgtaggcacgttggatcaggcgatgatggcggtaatgccatttaaacataacaacctgcggttactgggtcttagcaacaagatcttactggctgatgagatccatgcctgtgatgcctggatgtcccgaatacttgaaggtttgatcgaacggcaggccagtaatggcaacgccactattctgttatctgcgacgctatcgcagcagcagcgagataagctggtggcggcattttcccgtggggtgaggcgtagtgtgcaggcgccgttgctaggccatgacgattatccctggctgactcaggtcacacaaacagagctgatttctcagcgggttgatacacgcaaagaggttgagcgttgcgtagatattggctggctacatagtgaagaggcgtgtcttgaacgtataggtgaagcagtggaaaaaggaaactgtatcgcctggatacgtaactccgttgatgatgcgattcgtatctatcgccagcttcaactgagtaaggtcgtcgtcacggaaaaccttttactcttccatagtcgctttgctttttacgatcgtcagcggattgagtcacagacgctgaatctctttggcaaacagagcggcgcgcaacgtgccggtaaggtcattatcgccacgcaggtcatcgaacaaagtctggatattgactgcgatgagatgatctctgatttagcgccggtggatttattaattcagcgggccggtcgactacagcgtcatattcgcgatcgtaacggtctggtgaaaaagagtgggcaggatgagcgagagacgccagtgctgcgcattcttgctccggagtgggatgacgcgccgcgagagaactggttatccagcgccatgcgtaacagcgcctatgtctatcccgatcatgggcgcatgtggctgacacagcgcatattacgtgagcaggggacgattcggatgccgcaatctgcccgattgttgattgagtcggtctacggcgaggatgtcaacatgccggttggatttgcaaaaaccgagcaattgcaggaaggcaaattttattgcgaccgggcatttgccggccagatgctgcttaactttgcgccgggctactgtgctgaaattagcgattctttaccggagaaaatgtcaacgcggctggcggaagagtctgtcacgctgtggctggcgaaaatcgtggatagcgtcgtaaccccttatgccagcggtgaacacgcctgggagatgagcgtgctgcgagtacgtcagagctggtggaataaacataaagacgagtttgaaaaattagacggcgaacccttgcgtaagtggtgtgcgcaacagcatcaggataaggattttgccacggtgattgtggtgacggactttgccgcttgtggttattcggcgaatgagggattgattggcatgatgggggaataa

SEQ ID NO: 269 - protein, 887 aa, Salmonella enterica subsp. enterica serovar Typhimurium str. 14028S; identical to SEQ ID NO: 267
  REGION 1..887: note = Salmonella enterica subsp. enterica serovar Typhimurium 14028S Cas3

SEQ ID NO: 270 - DNA, 2664 bp, Salmonella enterica subsp. enterica serovar Typhimurium str. 14028S; identical to SEQ ID NO: 268
  misc_feature 1..2664: note = Salmonella enterica subsp. enterica serovar Typhimurium 14028S Cas3 nucleotide sequence
  source 1..2664: mol_type = other DNA

SEQ ID NO: 271 - protein, 926 aa, Streptococcus salivarius
  REGION 1..926: note = Streptococcus salivarius Cas3
MKHINDNFWAKKTEENSRLLWLPLTQHLEDTKNIAGLLWEHWLSEGQKVLIENSINAKANIENQGKRLAQFLGAVHDIGKATPAFQTQKGYANSVDLDIQLLEKLERAGFSGISSLQLASPKKSHHSIAGQYLLSHYGVEEDIATIIGGHHGRPVDDLDGINSQKSYPSNYFQDEKKDSLVYQKWNSTQEAFLNWALTETGFNSVSQLPKIKQPAQVILSGLLIMSDWIASNEHFFPLLSLDETNVKSKSQRIETGFKKWKKSNLWEPETFVDLVTLYQERFGFSPRNFQLILSQTIEKTTNPGIVILEAPMGLGKTEAALAASEQLSSKKGCSGLFFGLPTQATSNGIFKRIEQWTESIKGNNSDNFSIQLVHGKAALNTDFIELPKGNTINMDDSENGSIFVNEWFSGRKTSALDDFVVGTVDQFLMVALKQKHLALRHLGFSKKVIVIDEVHAYDAYMSQYLLEAIRWMGAYGVPVIILSATLPAQQREKLIKSYMAGMGVKWRDIENIDQIKIDAYPLITYNDGPNIHQVKTFEKQEQKNIYIHRLPEEQLFDIVKEALDNGGVVGIIVNTVRKSQELARNFSDIFGDDMVDLLHSNFIATERIRKEKDLLQEIGKKAMRPPKKIIIGTQVIEQSLDIDFDVLISDLAPMDLLIQRIGRLHRHKIKRPQKHEVARFYILGTFEEFDFDEGTRLVYGDYLLARTQYFLPDEIRLPDDISPLVQKVYNSDLTITYPKPELHQKYLDAKMEHDDQIKNKERKAKSYRIANPVLKKSRVRTNSLIGWLKNLHPNDSEEKAYAQVRDIEDTVEVIALKKISDGYGLFIENKDISQNITDPIIAKKVAQNTLRLPMSLSKAYNIDQTINELERYNNSHLSQWRNSSWLKGSLGIIFDKNNEFILNGFKLLYDEKYGVTIERLDKNESV

SEQ ID NO: 272 - DNA, 2781 bp, Streptococcus salivarius
  misc_feature 1..2781: note = Streptococcus salivarius Cas3 nucleotide sequence
  source 1..2781: mol_type = other DNA
atgaaacatattaatgataatttttgggctaagaaaacagaggaaaatagtagacttctttggttaccattaactcaacacttagaagacacgaaaaatattgcaggcctcttatgggaacattggttaagtgaaggacaaaaggtattaattgaaaattctattaatgctaaagcaaatattgaaaatcaagggaaaagattggcacaattcctaggagctgttcatgatatcggtaaagcaacaccagcttttcagacgcaaaaaggttatgcaaattcagtagatttggatattcaattgttagaaaaattggaacgcgcaggtttttctggcattagttctctccaactagcctcccctaaaaagagccatcatagcattgcaggtcaatatttgttatcccattatggcgtggaggaagatattgcaacaattattggtgggcaccatggacgaccagttgatgatttagacggtataaattctcaaaagagctatccttccaattatttccaggatgaaaagaaagatagtctagtttatcagaaatggaattcaactcaagaagcttttttaaactgggctttaacagaaacagggtttaattctgtgtctcagcttccaaaaatcaaacagcctgctcaggttattctatcaggtttactcataatgtctgactggattgctagtaatgaacatttttttcctttgttaagtttggatgaaactaatgtgaaaagcaagagtcaacgtattgaaactgggtttaaaaagtggaaaaaatctaacttgtgggaacctgaaactttcgttgaccttgttactctttatcaggaaagatttggatttagtccacgaaattttcagctgatactctcacaaacaatcgaaaagacgactaatcctggaatagtgatactggaagcgccgatgggactcgggaaaacagaggcggctctagcggcatcagagcagttatctagtaaaaaaggatgtagtggattgttttttggattgcctacacaagcaacctctaatggaatttttaagaggattgaacagtggacagagagtataaagggtaacaattctgataatttttctattcagctggttcatggaaaagcagccttaaatacggattttatagagctacctaaaggaaatacaattaacatggacgactcggaaaacggtagtatttttgtcaatgagtggttttctgggagaaaaacttcagcattagatgattttgtagttggaacagtcgaccaatttttaatggtggctttaaaacaaaaacatttggccttacgacatttggggtttagtaaaaaagttatcgttattgatgaagttcacgcttatgatgcctatatgagccaatatttgttggaagccatcagatggatgggagcttatggtgttcctgtaattattttatcagcaactttacctgcccaacaaagagaaaaactcataaaaagctatatggctggaatgggagtgaaatggcgagatattgaaaatatagatcagataaaaatagacgcatatcctttaatcacttataatgacggacctaacattcatcaagttaaaacgttcgaaaagcaagaacaaaaaaatatctacattcatcgtttaccagaagaacagttatttgatattgtaaaagaagctcttgacaatggtggagtagtggggataattgtcaatacagtgagaaaatctcaagaattggcaagaaatttttcagatatttttggagatgatatggtagatttgcttcattctaatttcatagcaactgaaagaatccgaaaagaaaaggatttattgcaagaaattgggaaaaaagcaatgcgtccaccaaagaaaatcattattggtacacaggtgattgaacagtcgttagatattgattttgatgtactgataagcgatttagcgcctatggatttactcattcaacgtatcggacgactacatcgtcacaaaatcaaacgaccccaaaagcacgaagtagcaagattttatattttaggaacatttgaagagtttgattttgatgaaggaacgcgtttggtttatggggactacctattagctagaactcagtactttttaccagatgaaatacgacttcctgatgatatttcaccgcttgtccaaaaggtttataattcagacttaacaattacgtatccaaagccagaacttcatcaaaaatatttggatgctaagatggaacatgatgatcagattaaaaataaagaaagaaaggcaaagtcataccgtattgctaatccagtcttaaaaaaatcgagagttcgaactaacagtttgattggttggttaaagaacctccatccaaatgatagtgaagaaaaagcatatgctcaagttcgagatattgaagatacagttgaagtgattgctttaaaaaaaatatctgatgggtatggtttgttcatagaaaataaagatatatctcagaacattactgatcctataattgcaaaaaaggtagcacaaaatactttacgacttccgatgagtttatccaaagcctataatattgatcaaacgattaatgagcttgaaagatataacaatagccacttaagtcaatggcgaaactcatcatggttaaagggatctcttgggattatttttgataaaaacaatgagtttatactgaatggatttaaactattatatgatgaaaaatatggtgttaccatagaaaggttggataagaatgagtcggtttaa

SEQ ID NO: 273 - protein, 661 aa, Clostridium difficile R20291
  REGION 1..661: note = Clostridium difficile Cas3
MNNLYEYKAKSDGTSIDKHNEDMNYIMNQLVSIYNISNDMKNDLYEAIVCHDVGKVVKSFQDNIESSTRRVRHELLSASIKYLNRGQKLAILTHHKDIKFLEGQITNSIYEIELKELKELLDIEVEDIRPFIKEISRARNDDTRKLENILLKGYLQYCDHIASAGIKSIDKGFNSIKDFSIPKGVSYNSIQEKVLNMDKNEDIMIMAMTGLGKTATSLYWSNLVQNEYKSKRVYYILPYTASINSLYENLYNRNISVSMLHSKAPYFLNKISDEEDIKQLYQIYKKSVKQINVCTIFQLVKSVFSCKRFEMLLSQLKDSIFIVDEIHCFDTRVLCYTLEFLKYLKENLNVKICIMSASIPTCLKKLIQERLQISTIIEPDSKDLIFRHRLNRLSEGILDSIHKIENDLMQGKRVLICVNSVDLSQELYGRLQKYNPKLIHGRFNTRDREQAEKGIEESFLLIGTQSIEVSLDISYDVLYTELAPLDSLLQRFGRVNRRGDNAELSNIYIYDYDRKLNIYDEDIINRTDIVISDIIHNDNSIVDESKVPSYLDNVYLDIDMDKYNKHKVALEIIMKNMRLGVWNKSANNDMLNNDTISVVPECLLEEYKLYIDKKMYLEASSLFVNVSVKRYNYNKKMFYECGDIVVTSYSYNDKLGLIFDC

SEQ ID NO: 274 - DNA, 1986 bp, Clostridium difficile R20291
  misc_feature 1..1986: note = Clostridium difficile Cas3 nucleotide sequence
  source 1..1986: mol_type = other DNA
atgaataatttatatgaatataaagctaaatcagatgggacaagtatagataagcataatgaagatatgaattacataatgaatcaattagttagcatatataatatatctaatgatatgaaaaatgatttatatgaggcaattgtatgtcatgatgtagggaaagtagtaaaaagctttcaagataatattgaaagtagcacaagaagagttagacatgagttattatcagcaagtattaagtatttaaatagaggtcagaagttagctatattaacccaccataaagatataaagtttctagagggtcaaataacaaattctatttatgaaattgaattaaaggaattaaaggaactattagatattgaagtagaagatataagaccatttataaaggaaatatcaagagcaagaaatgatgatactagaaaacttgaaaatatattattaaaaggttacttgcaatattgtgaccatatagcttctgcgggaattaaaagtatagataaaggatttaattctattaaagattttagtataccaaagggtgtaagttataattcaatacaagaaaaagttttaaatatggataaaaatgaagatataatgataatggctatgacaggtcttggaaaaacagcaacatcattgtattggagtaacctagttcaaaatgaatataaaagtaagagagtgtattatatacttccttatacagcaagcataaattctttatatgaaaatttatataatagaaatataagcgtaagtatgttacacagtaaagctccatattttttgaataaaattagtgatgaagaagatataaaacaactttaccagatatacaaaaagagtgtaaaacaaattaatgtatgtactatatttcaattagtaaagtcagtattttcttgtaagagatttgaaatgctactatcacaattaaaagatagtatatttatagttgatgaaatacattgttttgatacaagagtattgtgttatacattggaatttttaaaatatttaaaagaaaacttaaatgtaaaaatatgtataatgagtgcaagtataccaacttgcttaaaaaagttaatacaggaaagattgcaaataagtacaattattgaaccagatagtaaagatttaatatttagacatagattgaatagattaagtgaaggaatacttgatagcatacataaaatagaaaatgatttaatgcaaggaaaaagagtattaatatgtgttaattcagtagatttatctcaagagttatatggaaggcttcaaaaatataatcctaaattaatacatggtcgatttaatactagagatagagagcaggcagaaaaagggatagaagaaagcttcttattgataggtactcaaagtatagaggtaagtttagatataagttatgatgttctttatacagagttagctcctttagattcattgttacaaaggtttggtagagtaaatagaaggggagataatgctgagttgagcaatatttatatatatgattatgatagaaagcttaatatatatgatgaagatataataaataggactgatatagtaatatcagatataatacataatgataattctatagttgatgagagtaaagttccatcttatttagataatgtctatttagatatagatatggataaatataataaacataaagttgctttagagattataatgaaaaatatgaggttaggggtatggaataaatctgctaataatgatatgttaaataatgatactattagtgttgtgcctgaatgtcttttagaagagtacaagttgtatattgataaaaaaatgtatttagaagcgagttcattatttgtaaatgtatctgtaaaaagatacaattataataaaaagatgttttatgaatgtggagatatagttgttacaagttatagttataatgataaactaggtctaatatttgattgttaa

SEQ ID NO: 275 - protein, 773 aa, Clostridium difficile 70-100-2010
  REGION 1..773: note = CRISPR-associated helicase Cas3 [Clostridium difficile 70-100-2010]
MLYAKSNPVETLREHTDELLKQMNVLRESYGKNINSLDFLEEEIFWQLLDLVIEFHDIGKAFSPFQELIKSRMDTKINEPKIVTHLENNVGHNYLSPAFIDYSYIDRKKNKELRAVLNQVIVYHHERDIFIDKDFKNLIQKILDEDLINKVYELQHEFKVRYPIKTERLSKVYLQSVEKRIDKNHKYYNLYIMLKGILHRLDHSASAHEVVECNNVINIGEQTENYLMKEFGSLREAQSFAKSNRNKNIILIASTGMGKTETALIWIDKDKAFFTLPLRVSINALFDRAKNIVGVGESNDTFLGLLHSTAIDYLEESNQENSSEIVDLAKLLSCKLTFSTIDQIFKFPFLYRGYEKVYSTLAYSKVVIDEIQAYSPEIAAVLVKGIEMIHKIGGRFMIMTATMPTIYIDELKKRGVMNSNLAELTCNTEKIRHCVSIVENSIDENLGKIIQSGMNKKVLVIVNTVKSAVEKYELIEEIVKPKGIDVNLNLLHSMYIQEDRAKLEKYIKEFANSDRNGIWITTQLVEASLDIDFDELHTENSTLDSLFQRFGRCYRSREYEENSPNIFIYTEKATGIGSIYDKDIVEKGLELLKTFINGKECVKMKEKYKVEMVKILYSKESLEGTAFEKRFTSALNILDTITPYSLGSKDAQNILRNIEGYTVIPEDIYNKIEETLIKDYEELGQELINAYSNDDRQLINKIKSKRKKARREIIKKTVNLPIYKAKQNVIDIQVKGLEDLKILLYKYDIYENKHTKQIFGKGVLISNEIDQFI

SEQ ID NO: 276 - protein, 852 aa, Clostridium difficile 70-100-2010
  REGION 1..852: note = CRISPR-associated helicase Cas3 [Clostridium difficile CD51]
MYFKKVELFDISNNINNCKNIYAHINKDRKPETLKEHSDLSYSYLMKLCVKKDLSSCLERIENKFFKKDSFLSKNFYREIILNMVYMHDIGKINSSFQFVKMQNKNFKKISLRYTKHSFISSMLYFDYYFEKLKKYDFEEKKILSLFLMINTYTISKHHGVLKSFKEFLFLFKDEFINIKENFKDLFKNNYNLELKSVPKTIEKMVRGVEAYLDDSHIKDNLAIDLYIYSKLMFSIVTSCDFYATSEYNSGNSIDDFGTIDNYNKYYDVLKKSEIYKGMKKYREYLNNNSECPYKENDINRLRTEMSIEAEDAITHNTRKRIFYLEAPTGSGKTVTSINLALKSIELNQSLKKIFYIFPFNTLVEQTKDVFINEIFNSVKDIQKDVVVINSITPIQTEDKEEDNKNVEYCVTKQEIDYDKSLLNRQFLHYPIVLTTNIGFFNYLFGVSREECFPLIHMINSVIILDEIQNYKNEIWKEIILFLEKYADILNIKFIIMSATLPRLNKLGCNDDNFAYLVKNREKFFKNHLFKDRVNISFEMLNSEINDIEEISEKVIEEAEIYNKILIEFIKKSSALKFYKNIKEKLKYKLEDVFLLTGDDNKLERKKIINKIKDMNSVILVATQVVEAGVDIDMDLGFKDISTIDSDEQFLGRINRSCKKLNSKVYFFNLDDASKIYKKDVRKERHLTLNEESNRKIILDKDFEKYYDKIIARIEENKHKHNDKNIEVFIKDIVGNLNFTEVKKWMALIPDLKEYTIFLNTIVKDESGNMIVGSDVWYEYISLLKNDNVEYSEKRVKMSEIMEKLDYFTYKVQKFDNSFNDLVGDIFYIDDGSKYFTEGKFDRSKFNQNEFL

SEQ ID NO: 277 - protein, 661 aa, Clostridium difficile F253; identical to SEQ ID NO: 273
  REGION 1..661: note = CRISPR-associated helicase Cas3 [Clostridium difficile F253]

SEQ ID NO: 278 - protein, 468 aa, Clostridium difficile F501
  REGION 1..468: note = CRISPR-associated helicase Cas3 [Clostridium difficile F501]
MVYAVPYTSIIEQNARVFRDVLGERSVLEHHANFDFDFDEEVESYKSGDAKKALRRASENWDAPIVVTTNVQFFESLYANRTSRCRKLHNIANSVIVLDEAQMVPTKQLLPCLRALIELVANYGCSVVLCTATQPAFNGMLGRKGFAVREIAPAPSELFKKLKRVSYRFDGVLGDDDLAARLADRDQSLCIVNSRKQARRLHELLDGEGSYHLTTLMHPVHRERVLNEIRQRLREGRTCRVVATSLIEAGVDVDFPVVYRALAGVDSMVQAAGRCNREGRQSAEESIVHVFEPADDYALPSDVAQKVAIARSVISEMEGAACESCDIGALEAIDAYFARLYAVREGALDASGVLRDLEGFSLKSLNIPFKRAADDFRMIEEGSRTVVIPDPEIESDILAVKTGFANRSTMRRLSRYAVGVYDGDIKALLGSGKVETLAVDLFVLVDGTCYSDQRGLDLKIEEGKGIFL

SEQ ID NO: 279 - protein, 788 aa, Clostridium difficile P28
  REGION 1..788: note = CRISPR-associated helicase Cas3 [Clostridium difficile P28]
MNILAHINSNQEMQSLQEHSEHTFTAIKEYAAARGLTNCMKLTAFLHDCGKASREFQKYITKAAMENIFLPKVNHSSAGAQILLEVCRSYSDMSECLVKLMLANAIVSHHGLCDFINVHGDNALRSRCYPKKALDMEHITAFMNDFISTEELENLFRAAHKELSVYLANFMKQKTAQDAKDYYFYIGALQRLLMSLLIHGDREDTRNFMEHTQTIVYTEDTIWQAATDKLESHLAEITANSSFNPINELRASISDQCKAFSSHSPGIYRLSCPTGSGKTLASLRYALHHAKKYHKKHIIYVAPFKTILEQNAEVMKQFFNEDLVLEHHSNIIPSQYTDYDYYSSSWNKPVILTTAVRLFDVMFKDRTTDVRRFHQLADSVLIIDEAQKIPVQTISMFNEMMNFLAYNCNTTVVLCTATQPLLETTTYPIKLASESEIVKQTKEMQEQFKRVHIEDACRRGGYSIADLSDFIFQKLQPGCSMLVIVNTKAEALNLYRACEQHHEIDGLHLYHLSTSMCPEHRHLTLEDLKEHMEQKDTVLCIATNLIEAGVDIDCDVVIRSLCGLDSILQAAGRCNRNGKNSELGTVYLINSNEEHIEKLKDVRKGQNETDILLSQLHASKEGNRVDELLTLPFIRQYYDSYLFDRRQDTEYSTKIENRKVSLFDLFSRIGSKKESDDLAHPCLGHALKSAGEKFEMIDSQSIGVLVPYKDGEKLINQLNSSISNAEKYALLDKTQRFMVNVYEHKYKELEKEDMIYQLEFNGMLVLRDGFYKKDTGLEVRKELEDMFV

SEQ ID NO: 280 - protein, 841 aa, Clostridium difficile E15
  REGION 1..841: note = CRISPR-associated helicase Cas3 [Clostridium difficile E15]
MNLEKIIKSNKYIYSHKSEDEEENILLHLDRTKCVFFQIDSKYKILNKLRKTYGNLKFKLNELDFYLSEEAINLIENMFLYSVYLHDIGKINPKYQSEKMKNNFEFLSEEEKSTLCLNKIVSTNHSYLSSIVYIDLMQEKIDESKNISTKEKIVLYYLMLVNANIISRHHSNQSNLEYYFAKLEREINNAKMANYLYFYNKKLNINYEKISKAFINIKKIKFDETSVYIWNKILNSLLISCDFIATHSFYSKKSISEFKINCIEGKENIKDIFYKNPIYKGIESYKLNNRYFEENNLPKINELRSDILIESNNNLDKNNNERIFNIESPTGSGKTINSLSCALKLIKDGSKLFYVFPVNTLAEQTEDVLNGIFKGKLNTQIINSISPLPIKSTDKKIDYNKVLLDRQILNYESILTSNITLFNLFFGCGREQSMGLFSLFDSVIILDEIQNYKNLIWKEIVEFLYKFSEIMDFKLIIMSATLPNLEELMDFEDKKFINLIENPKIYYNNKLFKDRVSIENKLLNETVDFKKLLDLIKEEVNIWNKEKKEYAKFLIEFITKKTAQEFYMYVSKKLNNYTVFELDGDDNKIKKQSIINHLKKDSKELKSNILLITTQVIEAGVDIDMDLGAKDTSFPDLDEQFIGRINRSCLKEGCKAFLFNLDMANIVYKNDYRLVMNIDKNKDNYLKCLSNKDFSCLYDKVFNKINLTKGNWLCSEIDVFYKDLKMIRNKDISKHMKLIDINSFEIFIPTIIDGVDGEEVWSEYVELVSNIDMEYAERKVKMINLKEKLEMFTFSIKSNKSNKLNAFGGFYYIKNGNKFIANDKFDSSRFKKEYMCLLNAQ

SEQ ID NO: 281 - protein, 796 aa, Peptoclostridium difficile CD105KSO7
  REGION 1..796: note = CRISPR-associated helicase Cas3 [Peptoclostridium difficile strain CD105KSO7]
MKKELLAGPCNLNINKKEQTLVEHIKDLFEVLESILDPDLYSYKDIEILKICCALHDLGKINLIVQQKIEINNKISSSFSKEEIEKLEYQKKSLEKIARHNVFSGAFLQSILEKMNLSEEDKLYIYKTIMLHHGNYIDYMKLTTTKVQEEIYKYIESGILENKDSFNLEDIENYIKYILDIEFKFNEDMLDYDYLDKVSENMVIESDYNNGQIDDSILNDRRSKHIFYKGMLNLIDHRAQSINKEIKFYNDFTDKEIDEMILIDICKNHSDLEKSNVEFNTIQKRLRELSGKNVLTVDFTNSVKTYADDRKRFKRKLFLVSNQLSLESLYIKNIFKNKNNLDRRNDDYIGLIDGDINLYSYTENNKELDFVVTSRDIDLSVNFCKPYIIATIDQLLLSMFKFPGYEMTFAAIKNSSITIDEVHLLHPKIFLILIYFMQFACKYLNVDFHLMTTILPKPYKDQMISKGIIFQEECNENITDKGEIVFIESNKEEELCEGKNVKVSFIKEKEIKLIVEEALEKKQRILIIKNTIDSANSAYEFLKENLSDKYNGIDINVLHNRFKFKDKKDKYSKILNGKGDILISTQEISLDLDFNIVISDLAHMDCLIQRMGKCNVNNKYEYGNFYILPSEDNFYDNKLKNATKDILNNILKTNSIFTMSLRKNILDYYYDNGIVKKYFEDSFSNCDKEIKNIFGIYKTHFDGLDLIFNFEPYKNIIDNEKEASKLFKSTEISCKIILEEDFYKEDRDLRNDSIQVSGFIFNRFYYLGLITPLEGYMILKSSNKFEYNSTVGLILQ

SEQ ID NO: 282 - protein, 798 aa, Clostridium difficile 1002
  REGION 1..798: note = CRISPR-associated helicase Cas3 [Clostridium difficile strain 1002]
MLLNYLESWVFTMKKEILAKSYNLITNQQEQTLVEHIENLFKVLEVISESNLYSNKDIEMLKVCCALHDLGKINLITQQKIEINNKISSSSSKEEIKKLEFEKKSLEKIARHNVFSGAFLKSILEKMNLSEEDEFYIYKNIMLHHGSYIDYMKLTTTKVQEEIYKYIDNGILENKESFNLKDIEDYISEILNIDFKFNEDVLDYDYLDKLSEKMVIESDYSNGQIDDSVLNQRRANYILYKGMLNLIDHVAQGTNKDIKFYNDFTDKEIDEMILNDIYNNHDNLENNNIEFNIVQKRLREFSGKNVLTVAFTGSGKKVADCRKNFKRKLFLVPNQFPSESFYIKNIFKNDYLGLLNGDINLYSYSENYNEQDCEVTLRDIDLSLNLCKPYLIATIDQLLLSMFKFPGYEKIFASVKNASITVDEVHLLNPKMFLILIYFIQFACKYLNVDFHLMATMLPKSYKEQMISKGIIFQEECNENITDKGEIVFIESNKEEDICEGKNVKVSFIKEKEIKSIVENALEKKQRILIIKNTIDSANSTYKLLKENLSNKYNDADINVLHDRFKFKDKEEKYNKIFDEKGDVWISTQEISLDIDFNIVISDLATMDSLIQRMSKCNSNDKCEYGNFYILPSKDEIYDDKLKNTTKSILNKILKTESIFTMSIRKNILNEYYDNSVVKKYFEDSFINCDNEIKNIFGMYKANFDGLDLIFNFEPYKHIVDNESEASKLFKATDTNCKIILEEDFYREDIDLQRDSIQVSGFIFNRLCYLKLINKLEGYMVLKSSNKLKYNSTLGLIL

SEQ ID NO: 283 - protein, 806 aa, Clostridioides difficile R9385
  REGION 1..806: note = CRISPR-associated helicase Cas3 [Clostridioides difficile strain R 9385]
MKNIMQKEILAKSYNLRTNQQEQTLVEHIKDLFEVLESILELNLYSDKDVEILKICCALHDLGKINSIMQQKMEINNKISYSCSEEERKKLESDKKSLKKIARHNIFSGAFLKDILEKMNLSEEDKLYIYKSIMLHHGNYEDYMRLSISKVQEEIYEYIEKGILEKEEFNLKDIESYINSILNVDFKFGEDVLDYDYIDKLSESMFIDSDYNNGQIEDSVLNYRKFKYILYKGMLNLIDHSASSRQKGIKFYNDFTDEEIDDMILNEIYKSQGNLEKNNIEFNTIQKRLRELSGRNVLTVAFTGSGKTAADYRKIFKRKFFLVPNKISAESFYRKNIFQNKNDLDTRSSNDYIGLLHGDINLYSENEDNGEHDFVLTLRDIDLSINFCKPCVIATVDQLLLSMFKFPGYEKIFAAVKNASITVDEVHLLEPKMFLILIYFMQFACKYLDVDFHLMTATLPKSYKEQMINKGIIFQEESNENVTDKGEIVFIESNKEEEICEGKDVKVSFIKEKEIKSIVEDALENKQKILIIKNTIDSVNRTYEFLKENLSDKYGGVDIDVLHSRFKFKDKKEKYSKILNGEGDIWISTQSVEISLDLDFNIIISDLATMDSLIQRMGRCNRNNKYEYGNFYILPSEDKIYDNKLKNTTKNILKDILKTNSIFTMGIRKTILDDYYDNSVVKKYFEENFISCDKEIKNIYGINKEIFDGLDLIFNFEPYKNIVDSKKEAAKIFRDVDVSYKIILEEDFYKEDRELQQDSIQVSGFIFNRLYYYGLISKVEGYMVLKSSSKFEYNSTVGLILKRAYV

SEQ ID NO: 284 - protein, 770 aa, Clostridium sordellii R32921
  REGION 1..770: note = CRISPR-associated helicase Cas3 [[Clostridium] sordellii strain R32921]
MIYAKSDPIETLREHTDALIEAQKLLKESYGNNINKLNFINEEEFWNLLDIIVEFHDIGKAFSPFQKLIRDNMEVEFNEDKVVTHLENNVNHNYISPAFIKYKDLGIKDKELRKVLNQAIVYHHERDIFIDEDFKSLVQKVLDEDLINKVEEIQSDFKIRYPIKTKKLSSSYLDGVEKRITNKHEYYKLYIMLKGLLHKLDHSASAHELIEVDYDKYIGKYTEEFILNEYDGLRDVQKFAKENIDKNVLLIASTGMGKTETALIWINEDKAFFTLPLRVSINALFDRVKNIKDKEENEYKYAGLLHSTSIDYLEENDYEDSKQITDLSKLMSKKLTFSTIDQVFKFPFMYKGYEKTYATLAYSKVVIDEIQAYSPEIAAVLIKGLEMIHKIGGKFMIMTATMPTIYIDEMKERGLFDDNLAIATFNTEKVRHNIVVKDESINENIKEITKAGLSKKVLIIVNTVKSAIEKYEQIEKIIEDNELDIDLNLLHSMYIQEDRSKLEKAIKDFASSEKNGIWITTQLVEASLDIDFDILHTEISTLDSLFQRFGRCNRAGKKSINRPNIFIYSKEAQGIGTIYDEEIVKKGIELLKEYTKGKESLKIKEDDKVKMVEVLYSKENLENTEFYKKFKAALDILDTMPPYSVGSKDAQKILRDIDAYTVIPRQIYDKIEDNLIDEYKYLGEELSAAYNNKDKKLISELKDKRRSIRQQITKKTVSVSAYKVRQNKLINNIDVKGLEDLKILEYEYDMNYEILKGKGVLLGKELSQFI

SEQ ID NO: 285 - protein, 674 aa, Clostridium sordellii R32668
  REGION 1..674: note = CRISPR-associated helicase Cas3 [[Clostridium] sordellii strain R32668]
MDMFYAKGNKETIEEHTYKVLERLNRVIDLYKSNIKYHELMRLAVKYHDAGKVMLSFQKKLKNEHFKNVEFIKHKDYIKHNHLSSYFVLNEEVKDLDYDELRMLYQIIYYHHQQKNSIFIKNLDEVEEIIDYISENILPHYDFNYDVEEYILDRIDFFNEYDEQLVYNYYVSRGIVKRSDWMGSANLNIETDKLDKVESVHNFMSKKKFSLNKMQQFMFNNTNNNIITIASTGMGKTEGSLLWIGDSKGLFTLPLKVSLNSLYKRSISEDILNLDKSKVGLVHSDTSFIVDDKEEIPNMKNFNKNLTFCTIDQLLPIVFKHKHFDVKLGILSHSKVVLDEVQAYNPTMLGYIVVFLKMVVAAGGQFAIVTATLPPVFKYYLEKELKQEVLTESFIHEDKNNHVVTCYDKYVEVDDIIKNYNNNKVLVVVNTVRKAKKLYEELTQRGIEANLLHSHFTVKDRKIKETDIQSQFNDGIWISTQIVEASLDIDFDILLTELSEISGLVQRMGRIYRHRKYTSDKSNILVYTKTDSIGPTKNIVDYTIYKLTKEAIQSYKDYLLTEYEKQELVKNIYSVDNLKKHNSEYLQEIRNTINNIRLLNESDIKAKDIKIRELDTVTMIPRILGTEYNRENTIVIRRDILNKLSKTKEISYDSTNNCYFMDVKYDFEHGLYLD

SEQ ID NO: 286 - protein, 847 aa, Robinsoniella peoriensis 6600698
  REGION 1..847: note = CRISPR-associated helicase Cas3 [Robinsoniella peoriensis strain 6600698]
MCLFINMEDVINADYPLYAHWKDDSDKETLVEHLQRCGKYFQMLEKEKELSIVVKRFALKLLPNDPDNIQSFIYKMFCNVVLFHDFGKINPTFQIQKMKNKKVPIKTLDGLSGSDHSLFSAVIYLDYFLEEIEKSSYSKKDKCLLTLLVWINAYVISRHHSDLEKMIDFTSKFKGKDGEIGYLLDVLTQSGLEGYAGLRSLSSDTIEKCVKKYSNVKDRMDRGQDITCFFYMRYLYSVLVACDYYATTEYMENVEIKEFGTIQCADTFQEPYERSELLQSIRNYEKERILQAEKSLVECNDINRMRSEMFLDAEEALRKNPEDTIYFLEAPTGSGKSNTAMNLGFQLLGSGKKIYYIYPFNTLVEQNRKILQEIFTDKKVQNQIVVVNSLMPITGRGNIAEDSREYYQNALLDRQFLNYPFILSTHVSFFETLFGYRKENIFSFMQLTDSIVILDEIQSYKNTIWAEIIIFLQACSELLGMKIIIMSATLPGLDILAGGEGTVTRLIEDRKKYFNHPLFQKRVTVSYELLKEKMTIDHLLEQVLEKSKPDKKVLVTFIKKDSAYEFFDSLCNYSDIQVPAYLITGDDSMYEREQILRPIREGNTGGMILVSTQVIEAGVDIDMDIGFKDISKLDSEEQFLGRINRSCKRDGIVYFFDMDQAKNIYGLDFRIDESFTLLTSEMREILKEKEFDIYYKKVLNVLKQQRNESTSSEGLDDFFYEHVKHMNSPCIADRMKLIEENKWNMSLVICRTLEIENGNVLDGWSLWERYEELLRNRTMDFSEKQLKLSDVRSKLNNFIYQVKWNPDLNYSGVLGELYCIRDGEEYFENGKLNRKKLESQGVMFVEL

SEQ ID NO: 287 - protein, 899 aa, Escherichia coli ECOR31
  REGION 1..899: note = CRISPR-associated helicase Cas3 [Escherichia coli strain ECOR31]
MRKYPLSLLKDKNIVTFFDFWGKTRRDEKEGGDDYHLLCWHSLDVAAMGYLMVKRNCFGLADYFRQLGISDKEQAAQFFAWLLCWHDIGKFARSFQQLYLHPQLKVPEGARKNYEKISHSTLGYWLWHHYLSECEELLPASSLSTRKLKRVIAMWMPMTTGHHGRPPDRIDELDNFLPEDKAAARDFLLEIKPLFPQLEIPAFWDDDEGVELIKQLSWYISATVVLADWTGSSTRFFPRVAQTMDIEDYWQKALVQAQNALTVFPPKAETAPFTGINTLFPFIENPKPLQQKVLDLDISQPGPQLFILEDVTGAGKTEAALILAHRLMAAGKAQGLFFGLPTMATANAMYDRLVKTWLSFYSPESRPSLVLAHSARTLMDRFNESLWSGDLVGSEEPDEQTFSQGCAAWFADSNKKALLAEIGVGKLDQAMMAVMPFKHNNLRLLGLSNKILLADEIHACDAYMSYILEGLIERQVRGGNSVILLSATLSQQQRDKLVAAFARGTEGQQEAPFLEKDDYPWLTHVTKSDVHSHRVATRKDVERSVSVGWLHSEQECIARIESAVSQGKCIAWIRNSVDDAIKVYRQLLARGVIPASSLSLFHSRFAFSDRQRIETETLARFGKNCSLKRSSQVIVCTQVIEQSVDIDLDEMISDLAPIDLLIQRAGRLQRHIRDINGQLKRDGKDERSPPELLILAPVWDDAPGDEWFGSAMRNSAYVYPDHGRIWLTQRVLREQGVIQMPHSARLLIESVYGEDVVMPDGFARSEQEQVGKYYCDRSMAKKFVLNFRPGYAANINDYLPEKLSTRLAEESVSLWLASCINGVVKPYASGAHAWEMSVVRVRRSWWKKHRDEFSLLEGEVLRQWCIEQRQDPEMANVILVTDDESCGYSATEGLIGKVD

SEQ ID NO: 288 - protein, 1077 aa, Escherichia coli ECOR61
  REGION 1..1077: note = CRISPR-associated helicase Cas3 [Escherichia coli strain ECOR61]
MNVLIISRCTKNARVESCRIIDQFAERTGDAAWQTVITLEGVNTLRRLLRKTARRNTAVACHWLKKNGQTELMWIVGNIRRFNAQGRVPTNRTTQISLVNKEENRWQCAESIALLAAIAGLFHDFGKSGRSFQQSLTQKNTRSYQPYRHEWISLRLFQTFVGERPDDVWLAKLGELTADDESAILERLQKDTPQFSNSPFSSLQPLAKTVGWLILSHHRMPENLSPQSEQSCKGCESWLEKQLNADWNAVNHRRDDWSQQDFAHVWQFPSGTPLQSASWREKARQIARRASNALGLKTYGQMEQLFPLHMARFCLMLADHYYSSSDAQQKWQDPDYIVWANSDRQSGTLKQRVDEHLVGVAHHAYLLGRQLMHTRASLPAIARHKGFSQRATDVNYRWQDKAWDVARALRERSREEGFFGVNMASTGCGKTFANARIMYALADEREGCRFTVALGLRTLTLQTGDALRSRLGLGEDELAVLIGSAAVNQLWQQEKIDNDCGSASQESPAEEQQFVKYEGSLHTGALEKWLKDDSKLKELVSAPILVSTIDHLISATEGVRGGKQLPAMLRLLTSDLVLDEPDDFDIADLHAVCRLMNWAGMLGTRVLLSSATLPPGLIQALFAAYLAGRKMWQASCGINGRPVNICCAWFDEKDADATQIYDGPGFRDAHAKFVARRAVMLAEKERLHFGRVASVSSASGAIQDVTESVAQTVHTQMLKLHQAHRQRHESGKTVSLGLVRFANINPLVAVTKALIAIPSPEDVCIHYCVYHSRHPLAVRSDIEKRLDRAFTRHNELDFWNNEDIADALHNRPESHHLFVVLGTSVIEVGRDWDADWGIIEPSSMRSIIQFAGRIQRHRRNVPTSENLVILRSNIKSLQKKAPAFCKPGFETKEHLLNSHDICELIPIADYRTINALPRILSANNANKLAELEHSRLSAELMSSKSKHVVAAQWWRAPLSWNGWMQRQTPFRYSPLPEAVFFLHMDDEESEARFYSRTGDNERKAQGNFRREEVRCASGVACWGVMDYQHVLLNLADKQSCEIANVGEKFAEVRVPVSEEDAVDDWRYHPWLGVFRNM

SEQ ID NO: 289 - protein, 888 aa, Escherichia coli ECOR72
  REGION 1..888: note = CRISPR-associated helicase Cas3 [Escherichia coli strain ECOR72]
MEPFKYICHYWGKSSKSLTKENDIHLLIYHCLDVAAVADCWWDQSVVLQNTFCRNEMLSKQRVKAWLLFFIALHDIGKFDIRFQYKSAESWLKLNPATPSLNGPSTQMCRKFNHGAAGLYWFNQDSLSEQSLGDFFSFFDAAPHPYESWFPWVEAVTGHHGFILHSQDQDKSRWEMPASLASYAAQDKQAREEWISVLEALFLTPAGLSINDIPPDCSSLLAGFCSLADWLGSWTTTNTFLFNEDAPSDINALRTYFQDRQQDASRVLELSGLVSNKRCYEGVHALLDNGYQPRQLQVLVDALPVAPGLTVIEAPTGSGKTETALAYAWKLIDQQIADSVIFALPTQATANAMLTRMEASASHLFSSPNLILAHGNSRFNHLFQSIKSRAITEQGQEEAWVQCCQWLSQSNKKVFLGQIGVCTIDQVLISVLPVKHRFIRGLGIGRSVLIVDEVHAYDTYMNGLLEAVLKAQADVGGSVILLSATLPMKQKQKLLDTYGLHTDPVENNSAYPLINWRGVNGAQRFDLLAHPEQLPPRFSIQPEPIYLADMLPDLTMLERMIAAANAGAQVCLICNLVDVAQVCYQRLKELNNTQVDIDLFHARFTLNDRREKENRVISDFGKNGERNVGRILVATQVVEQSLDVDFDWLITQHCPADLLFQRLGRLHRHHRKYRPAGFEIPVATILLPDGEGYGRHEHIYSNVRVMWRTQQHIEELNGASLFFPDAYRQWLDSIYDDAEMDEPEWVIKGMDKFESAECEKRFKARKVLQWAEEYSLQDNDETILAVTRDGEMSLPLLPYVQTSSGKQLLDGQVYEDLSYEQQYEALALNRVNVPFTWKRSFSEVVDEDGLLWLEGKQNQDGWFWQGNSIVITYTRDEGMTRVIPANPK

SEQ ID NO: 290 - DNA, 25 bp, Clostridium difficile 630
  misc_feature 1..25: note = C. difficile Repeat 73
  source 1..25: mol_type = other DNA
tgtttataatgtggataatatttaa

SEQ ID NO: 291 - DNA, 28 bp, Clostridium difficile 630
  misc_feature 1..28: note = C. difficile Repeat 74
  source 1..28: mol_type = other DNA
tgtgcgttagcactttaagcaacagaat

SEQ ID NO: 292 - DNA, 29 bp, Clostridium difficile 630
  misc_feature 1..29: note = C. difficile Repeat 75
  source 1..29: mol_type = other DNA
gttttagattaactatatggaatgtaaat

SEQ ID NO: 293 - DNA, 29 bp, Clostridium difficile 630
  misc_feature 1..29: note = C. difficile Repeat 76
  source 1..29: mol_type = other DNA
gttttagattaactatatggaatgtaaat

SEQ ID NO: 294 - DNA, 27 bp, Clostridium difficile 630
  misc_feature 1..27: note = C. difficile Repeat 77
  source 1..27: mol_type = other DNA
gtgcgttagcactttaagtaacggaat

SEQ ID NO: 295 - DNA, 29 bp, Clostridium difficile 630
  misc_feature 1..29: note = C. difficile Repeat 78
  source 1..29: mol_type = other DNA
gttttatattaactaagtggtatgtaaag

SEQ ID NO: 296 - DNA, 29 bp, Clostridium difficile 630
  misc_feature 1..29: note = C. difficile Repeat 79
  source 1..29: mol_type = other DNA
gttttatattaactaagtggtatgtaaat

SEQ ID NO: 297 - DNA, 29 bp, Clostridium difficile 630
  misc_feature 1..29: note = C. difficile Repeat 80
  source 1..29: mol_type = other DNA
gttttatattaactatatggaatgtaaat

SEQ ID NO: 298 - DNA, 29 bp, Clostridium difficile 630
  misc_feature 1..29: note = C. difficile Repeat 81
  source 1..29: mol_type = other DNA
gttttatattaactatgtggtatgtaaat

SEQ ID NO: 299 - DNA, 29 bp, Clostridium difficile 630
  misc_feature 1..29: note = C. difficile Repeat 82
  source 1..29: mol_type = other DNA
ctttacataccacatagttgatataaaac

SEQ ID NO: 300 - DNA, 29 bp, Clostridium difficile 630
  misc_feature 1..29: note = C. difficile Repeat 83
  source 1..29: mol_type = other DNA
atttacattccatatagttaatctaaaac

SEQ ID NO: 301 - DNA, 29 bp, Clostridium difficile 630
  misc_feature 1..29: note = C. difficile Repeat 84
  source 1..29: mol_type = other DNA
atttacattccatatagttaatataaaac

SEQ ID NO: 302 - DNA, 26 bp, Clostridium difficile 630
  misc_feature 1..26: note = C. difficile Repeat 85
  source 1..26: mol_type = other DNA
ttaccatctatttgttgccatcctgt

SEQ ID NO: 303 - DNA, 26 bp, Clostridium difficile 630
  misc_feature 1..26: note = C. difficile Repeat 86
  source 1..26: mol_type = other DNA
tcttctgatggtggtactggaggatt

SEQ ID NO: 304 - DNA, 29 bp, Clostridium difficile 630
  misc_feature 1..29: note = C. difficile Repeat 87
  source 1..29: mol_type = other DNA
atttacattccatatagttaatctaaaac

SEQ ID NO: 305 - DNA, 29 bp, Clostridium difficile 630
  misc_feature 1..29: note = C. difficile Repeat 88
  source 1..29: mol_type = other DNA
atttacattccatatagttaatctaaaac

SEQ ID NO: 306 - DNA, 29 bp, Clostridium difficile 630
  misc_feature 1..29: note = C. difficile Repeat 89
  source 1..29: mol_type = other DNA
atttacataccacttagttaatataaaac

SEQ ID NO: 307 - DNA, 25 bp, Clostridium difficile
  misc_feature 1..25: note = C. difficile Repeat 90
  source 1..25: mol_type = other DNA
tgtttataatgtggataatatttaa

SEQ ID NO: 308 - DNA, 28 bp, Clostridium difficile
  misc_feature 1..28: note = C. difficile Repeat 91
  source 1..28: mol_type = other DNA
tgtgcgttagcactttaagcaacagaat

SEQ ID NO: 309 - DNA, 29 bp, Clostridium difficile
  misc_feature 1..29: note = C. difficile Repeat 92
  source 1..29: mol_type = other DNA
gttttagattaactatatggaatgtaaat

SEQ ID NO: 310 - DNA, 29 bp, Clostridium difficile
  misc_feature 1..29: note = C. difficile Repeat 93
  source 1..29: mol_type = other DNA
gttttagattaactatatggaatgtaaat

SEQ ID NO: 311 - DNA, 27 bp, Clostridium difficile
  misc_feature 1..27: note = C. difficile Repeat 94
  source 1..27: mol_type = other DNA
gtgcgttagcactttaagtaacggaat

SEQ ID NO: 312 - DNA, 29 bp, Clostridium difficile
  misc_feature 1..29: note = C. difficile Repeat 95
  source 1..29: mol_type = other DNA
gttttatattaactaagtggtatgtaaag

SEQ ID NO: 313 - DNA, 29 bp, Clostridium difficile
  misc_feature 1..29: note = C. difficile Repeat 96
  source 1..29: mol_type = other DNA
gttttatattaactaagtggtatgtaaat

SEQ ID NO: 314 - DNA, 29 bp, Clostridium difficile
  misc_feature 1..29: note = C. difficile Repeat 97
  source 1..29: mol_type = other DNA
gttttatattaactatatggaatgtaaat

SEQ ID NO: 315 - DNA, 29 bp, Clostridium difficile
  misc_feature 1..29: note = C. difficile Repeat 98
  source 1..29: mol_type = other DNA
gttttatattaactatgtggtatgtaaat

SEQ ID NO: 316 - DNA, 29 bp, Clostridium difficile
  misc_feature 1..29: note = C. difficile Repeat 99
  source 1..29: mol_type = other DNA
ctttacataccacatagttgatataaaac

SEQ ID NO: 317 - DNA, 29 bp, Clostridium difficile
  misc_feature 1..29: note = C. difficile Repeat 100
  source 1..29: mol_type = other DNA
atttacattccatatagttaatctaaaac

SEQ ID NO: 318 - DNA, 29 bp, Clostridium difficile
  misc_feature 1..29: note = C. difficile Repeat 101
  source 1..29: mol_type = other DNA
atttacattccatatagttaatataaaac

SEQ ID NO: 319 - DNA, 26 bp, Clostridium difficile
  misc_feature 1..26: note = C. difficile Repeat 102
  source 1..26: mol_type = other DNA
ttaccatctatttgttgccatcctgt

SEQ ID NO: 320 - DNA, 26 bp, Clostridium difficile
  misc_feature 1..26: note = C. difficile Repeat 103
  source 1..26: mol_type = other DNA
tcttctgatggtggtactggaggatt

SEQ ID NO: 321 - DNA, 29 bp, Clostridium difficile
  misc_feature 1..29: note = C. difficile Repeat 104
  source 1..29: mol_type = other DNA
atttacattccatatagttaatctaaaac

SEQ ID NO: 322 - DNA, 29 bp, Clostridium difficile
  misc_feature 1..29: note = C. difficile Repeat 105
  source 1..29: mol_type = other DNA
atttacattccatatagttaatctaaaac

SEQ ID NO: 323 - DNA, 29 bp, Clostridium difficile
  misc_feature 1..29: note = C. difficile Repeat 106
  source 1..29: mol_type = other DNA
atttacataccacttagttaatataaaac

SEQ ID NO: 324 - DNA, 28 bp, Clostridium difficile
  misc_feature 1..28: note = C. difficile Repeat 107
  source 1..28: mol_type = other DNA
tgtgcgttagcactttaagcaacagaat

SEQ ID NO: 325 - DNA, 25 bp, Clostridium difficile
  misc_feature 1..25: note = C. difficile Repeat 108
  source 1..25: mol_type = other DNA
tgtttataatgtggataatatttaa

SEQ ID NO: 326 - DNA, 28 bp, Clostridium difficile
  misc_feature 1..28: note = C. difficile Repeat 109
  source 1..28: mol_type = other DNA
tgtgcgttagcactttaagcaacagaat

SEQ ID NO: 327 - DNA, 34 bp, Clostridium difficile
  misc_feature 1..34: note = C. difficile Repeat 110
  source 1..34: mol_type = other DNA
aaaatcaaacagaaaaaatatgtatggaagcagt

SEQ ID NO: 328 - DNA, 30 bp, Clostridium difficile
  misc_feature 1..30: note = C. difficile Repeat 111
  source 1..30: mol_type = other DNA
gttttagattaactatatggaatgtaaatt

SEQ ID NO: 329 - DNA, 30 bp, Clostridium difficile
  misc_feature 1..30: note = C. difficile Repeat 112
  source 1..30: mol_type = other DNA
gttgaagaataacatgagatgtttttaaat

SEQ ID NO: 330 - DNA, 29 bp, Clostridium difficile
  misc_feature 1..29: note = C. difficile Repeat 113
  source 1..29: mol_type = other DNA
gttttatattaactaagtggtatgtaaag

SEQ ID NO: 331 - DNA, 29 bp, Clostridium difficile
  misc_feature 1..29: note = C. difficile Repeat 114
  source 1..29: mol_type = other DNA
gttttatattaactaagtggtatgtaaat

SEQ ID NO: 332 - DNA, 29 bp, Clostridium difficile
  misc_feature 1..29: note = C. difficile Repeat 115
  source 1..29: mol_type = other DNA
gttttatattaactatatggaatgtaaat

SEQ ID NO: 333 - DNA, 29 bp, Clostridium difficile
  misc_feature 1..29: note = C. difficile Repeat 116
  source 1..29: mol_type = other DNA
gttttatattaactatgtggtatgtaaat

SEQ ID NO: 334 - DNA, 29 bp, Clostridium difficile
  misc_feature 1..29: note = C. difficile Repeat 117
  source 1..29: mol_type = other DNA
ctttacataccacatagttgatataaaac

SEQ ID NO: 335 - DNA, 29 bp, Clostridium difficile
  misc_feature 1..29: note = C. difficile Repeat 118
  source 1..29: mol_type = other DNA
ttttacattccatatagttaatctaaaac

SEQ ID NO: 336 - DNA, 29 bp, Clostridium difficile
  misc_feature 1..29: note = C. difficile Repeat 119
  source 1..29: mol_type = other DNA
atttacattccatatagttaatataaaac

SEQ ID NO: 337 - DNA, 26 bp, Clostridium difficile
  misc_feature 1..26: note = C. difficile Repeat 120
  source 1..26: mol_type = other DNA
ttaccatctatttgttgccatcctgt

SEQ ID NO: 338 - DNA, 29 bp, Clostridium difficile
  misc_feature 1..29: note = C. difficile Repeat 121
  source 1..29: mol_type = other DNA
atttacataccacttagttaatataaaac

SEQ ID NO: 339 - DNA, 29 bp, Clostridium difficile
  misc_feature 1..29: note = C. difficile Repeat 122
  source 1..29: mol_type = other DNA
gttttatattaactaagtggtatgtaaat

SEQ ID NO: 340 - DNA, 29 bp, Clostridium difficile
  misc_feature 1..29: note = C. difficile Repeat 123
  source 1..29: mol_type = other DNA
gttttatattaactaagtggtatgtaaat

SEQ ID NO: 341 - DNA, 29 bp, Clostridium difficile
  misc_feature 1..29: note = C. difficile Repeat 124
  source 1..29: mol_type = other DNA
gttttatattaactatatggaatgtaaat

SEQ ID NO: 342 - DNA, 29 bp, Clostridium difficile
  misc_feature 1..29: note = C. difficile Repeat 125
  source 1..29: mol_type = other DNA
gttttagattaactatatggaatgtaaat

SEQ ID NO: 343 - DNA, 29 bp, Clostridium difficile
  misc_feature 1..29: note = C. difficile Repeat 126
  source 1..29: mol_type = other DNA
gttttatattaactatatggaatgtaaat

SEQ ID NO: 344 - DNA, 28 bp, Clostridium difficile
  misc_feature 1..28: note = C. difficile Repeat 127
  source 1..28: mol_type = other DNA
gttttatatcaactatgtggtatgtaaa

SEQ ID NO: 345 - DNA, 29 bp, Clostridium difficile
  misc_feature 1..29: note = C. difficile Repeat 128
  source 1..29: mol_type = other DNA
atttacataccacttagttaatataaaac

SEQ ID NO: 346 - DNA, 29 bp, Clostridium difficile
  misc_feature 1..29: note = C. difficile Repeat 129
  source 1..29: mol_type = other DNA
atttacattccatatagttaatataaaac

SEQ ID NO: 347 - DNA, 29 bp, Clostridium difficile
  misc_feature 1..29: note = C. difficile Repeat 130
  source 1..29: mol_type = other DNA
atttacataccacttagttaatataaaac

SEQ ID NO: 348 - DNA, 29 bp, Clostridium difficile
  misc_feature 1..29: note = C. difficile Repeat 131
  source 1..29: mol_type = other DNA
ctttacataccacttagttaatataaaac

SEQ ID NO: 349 - DNA, 27 bp, Clostridium difficile
  misc_feature 1..27: note = C. difficile Repeat 132
  source 1..27: mol_type = other DNA
attccgttgcttaaagtgctaacgcac

SEQ ID NO: 350 - DNA, 27 bp, Clostridium difficile
  misc_feature 1..27: note = C. difficile Repeat 133
  source 1..27: mol_type = other DNA
attccgttgcttaaagtgctaacgcac

SEQ ID NO: 351 - DNA, 25 bp, Clostridium difficile 2007855
  misc_feature 1..25: note = C. difficile Repeat 134
  source 1..25: mol_type = other DNA
tgtttataatgtggataatatttaa

SEQ ID NO: 352 - DNA, 24 bp, Clostridium difficile 2007855
  misc_feature 1..24: note = C. difficile Repeat 135
  source 1..24: mol_type = other DNA
ttgaatggtaaaaaatattacttt

SEQ ID NO: 353 - DNA, 24 bp, Clostridium difficile 2007855
  misc_feature 1..24: note = C. difficile Repeat 136
  source 1..24: mol_type = other DNA
ttgaatggtaaaaaatattacttt

SEQ ID NO: 354 - DNA, 24 bp, Clostridium difficile 2007855
  misc_feature 1..24: note = C. difficile Repeat 137
  source 1..24: mol_type = other DNA
ttgaatggtaaaaaatattacttt

SEQ ID NO: 355 - DNA, 24 bp, Clostridium difficile 2007855
  misc_feature 1..24: note = C. difficile Repeat 138
  source 1..24: mol_type = other DNA
ttgaatggtaaaaaatattacttt

SEQ ID NO: 356 - DNA, 24 bp, Clostridium difficile 2007855
  misc_feature 1..24: note = C. difficile Repeat 139
  source 1..24: mol_type = other DNA
ttgaatggtaaaaaatattacttt

SEQ ID NO: 357 - DNA, 24 bp, Clostridium difficile 2007855
  misc_feature 1..24: note = C. difficile Repeat 140
  source 1..24: mol_type = other DNA
ttgaatggtaaaaaatattacttt

SEQ ID NO: 358 - DNA, 24 bp, Clostridium difficile 2007855
  misc_feature 1..24: note = C. difficile Repeat 141
  source 1..24: mol_type = other DNA
ttgaatggtaaaaaatattacttt

SEQ ID NO: 359 - DNA, 29 bp, Clostridium difficile 2007855
  misc_feature 1..29: note = C. difficile Repeat 142
  source 1..29: mol_type = other DNA
gttttatattaactaagtggtatgtaaag

SEQ ID NO: 360 - DNA, 29 bp, Clostridium difficile 2007855
  misc_feature 1..29: note = C. difficile Repeat 143
  source 1..29: mol_type = other DNA
gttttatattaactaagtggtatgtaaat

SEQ ID NO: 361 - DNA, 29 bp, Clostridium difficile 2007855
  misc_feature 1..29: note = C. difficile Repeat 144
  source 1..29: mol_type = other DNA
gttttatattaactatatggaatgtaaat

SEQ ID NO: 362 - DNA, 29 bp, Clostridium difficile 2007855
  misc_feature 1..29: note = C. difficile Repeat 145
  source 1..29: mol_type = other DNA
gttttagattaactatatggaatgtaaat

SEQ ID NO: 363 - DNA, 30 bp, Clostridium difficile 2007855
  misc_feature 1..30: note = C. difficile Repeat 146
  source 1..30: mol_type = other DNA
gttttatattaactatatggaatgtaaatc

SEQ ID NO: 364 - DNA, 29 bp, Clostridium difficile 2007855
  misc_feature 1..29: note = C. difficile Repeat 147
  source 1..29: mol_type = other DNA
gttttatattaactatgtggtatgtaaat

SEQ ID NO: 365 - DNA, 29 bp, Clostridium difficile 2007855
  misc_feature 1..29: note = C. difficile Repeat 148
  source 1..29: mol_type = other DNA
ctttacattccatatagttaatataaaac

SEQ ID NO: 366 - DNA, 26 bp, Clostridium difficile 2007855
  misc_feature 1..26: note = C. difficile Repeat 149
  source 1..26: mol_type = other DNA
ttaccatctatttgttgccatcctgt

SEQ ID NO: 367 - DNA, 26 bp, Clostridium difficile 2007855
  misc_feature 1..26: note = C. difficile Repeat 150
  source 1..26: mol_type = other DNA
tcttctgatggtggtactggtggatt

SEQ ID NO: 368 - DNA, 29 bp, Clostridium difficile 2007855
  misc_feature 1..29: note = C. difficile Repeat 151
  source 1..29: mol_type = other DNA
atttacataccacttagttaatataaaac

SEQ ID NO: 369 - DNA, 29 bp, Clostridium difficile 2007855
  misc_feature 1..29: note = C. difficile Repeat 152
  source 1..29: mol_type = other DNA
atttataactaacttagtgtaatttaaac

SEQ ID NO: 370 - DNA, 25 bp, Clostridium difficile 630
  misc_feature 1..25: note = C. difficile Repeat 153
  source 1..25: mol_type = other DNA
tgtttataatgtggataatatttaa

SEQ ID NO: 371 - DNA, 28 bp, Clostridium difficile 630
  misc_feature 1..28: note = C. difficile Repeat 154
  source 1..28: mol_type = other DNA
tgtgcgttagcactttaagcaacagaat

SEQ ID NO: 372 - DNA, 29 bp, Clostridium difficile 630
  misc_feature 1..29: note = C. difficile Repeat 155
  source 1..29: mol_type = other DNA
gttttagattaactatatggaatgtaaat

SEQ ID NO: 373 - DNA, 29 bp, Clostridium difficile 630
  misc_feature 1..29: note = C. difficile Repeat 156
  source 1..29: mol_type = other DNA
gttttagattaactatatggaatgtaaat

SEQ ID NO: 374 - DNA, 27 bp, Clostridium difficile 630
  misc_feature 1..27: note = C. difficile Repeat 157
  source 1..27: mol_type = other DNA
gtgcgttagcactttaagtaacggaat

SEQ ID NO: 375 - DNA, 29 bp, Clostridium difficile 630
  misc_feature 1..29: note = C. difficile Repeat 158
  source 1..29: mol_type = other DNA
gttttatattaactaagtggtatgtaaag

SEQ ID NO: 376 - DNA, 29 bp, Clostridium difficile 630
  misc_feature 1..29: note = C. difficile Repeat 159
  source 1..29: mol_type = other DNA
gttttatattaactaagtggtatgtaaat

SEQ ID NO: 377 - DNA, 29 bp, Clostridium difficile 630
  misc_feature 1..29: note = C. difficile Repeat 160
  source 1..29: mol_type = other DNA
gttttatattaactatatggaatgtaaat

SEQ ID NO: 378 - DNA, 29 bp, Clostridium difficile 630
  misc_feature 1..29: note = C. difficile Repeat 161
  source 1..29: mol_type = other DNA
gttttatattaactatgtggtatgtaaat

SEQ ID NO: 379 - DNA, 29 bp, Clostridium difficile 630
  misc_feature 1..29: note = C. difficile Repeat 162
  source 1..29: mol_type = other DNA
ctttacataccacatagttgatataaaac

SEQ ID NO: 380 - DNA, 29 bp, Clostridium difficile 630
  misc_feature 1..29: note = C. difficile Repeat 163
  source 1..29: mol_type = other DNA
atttacattccatatagttaatctaaaac

SEQ ID NO: 381 - DNA, 29 bp, Clostridium difficile 630
  misc_feature 1..29: note = C. difficile Repeat 164
  source 1..29: mol_type = other DNA
atttacattccatatagttaatataaaac

SEQ ID NO: 382 - DNA, 29 bp, Clostridium difficile 630
  misc_feature 1..29: note = C. difficile Repeat 165
  source 1..29: mol_type = other DNA
atttacattccatatagttaatctaaaac

SEQ ID NO: 383 - DNA, 29 bp, Clostridium difficile 630
  misc_feature 1..29: note = C. difficile Repeat 166
  source 1..29: mol_type = other DNA
atttacattccatatagttaatctaaaac

SEQ ID NO: 384 - DNA, 29 bp, Clostridium difficile 630
  misc_feature 1..29: note = C. difficile Repeat 167
  source 1..29: mol_type = other DNA
atttacataccacttagttaatataaaac

SEQ ID NO: 385 - DNA, 29 bp, Clostridium difficile BI1
  misc_feature 1..29: note = C. difficile Repeat 168
  source 1..29: mol_type = other DNA
attaaaccttaacactacgtgtatttaaa

SEQ ID NO: 386 - DNA, 29 bp, Clostridium difficile BI1
  misc_feature 1..29: note = C. difficile Repeat 169
  source 1..29: mol_type = other DNA
attaaaccttaacactacgtgtatttaaa

SEQ ID NO: 387 - DNA, 29 bp, Clostridium difficile BI1
  misc_feature 1..29: note = C. difficile Repeat 170
  source 1..29: mol_type = other DNA
attaaaccttaacactacgtgtatttaaa

SEQ ID NO: 388 - DNA, 29 bp, Clostridium difficile BI1
  misc_feature 1..29: note = C. difficile Repeat 171
  source 1..29: mol_type = other DNA
attaaaccttaacactacgtgtatttaaa

SEQ ID NO: 389 - DNA, 29 bp, Clostridium difficile BI1
  misc_feature 1..29: note = C. difficile Repeat 172
  source 1..29: mol_type = other DNA
attaaaccttaacactacgtgtatttaaa

SEQ ID NO: 390 - DNA, 29 bp, Clostridium difficile BI1
  misc_feature 1..29: note = C. difficile Repeat 173
  source 1..29: mol_type = other DNA
attaaaccttaacactacgtgtatttaaa

SEQ ID NO: 391 - DNA, 29 bp, Clostridium difficile BI1
  misc_feature 1..29: note = C. difficile Repeat 173
  source 1..29: mol_type = other DNA
tattaaaccttaacactatgtgtatttaa

SEQ ID NO: 392 - DNA, 23 bp, Clostridium difficile BI1
  misc_feature 1..23: note = C. difficile Repeat 174
  source 1..23: mol_type = other DNA
aaccttaacactatgtgtattta

SEQ ID NO: 393 - DNA, 23 bp, Clostridium difficile BI1
  misc_feature 1..23: note = C. difficile Repeat 175
  source 1..23: mol_type = other DNA
attaaaccttaacactatgtgta

SEQ ID NO: 394 - DNA, 23 bp, Clostridium difficile BI1
  misc_feature 1..23: note = C. difficile Repeat 176
  source 1..23: mol_type = other DNA
attaaaccttaacactatgtgta

SEQ ID NO: 395 - DNA, 23 bp, Clostridium difficile BI1
  misc_feature 1..23: note = C. difficile Repeat 177
  source 1..23: mol_type = other DNA
attaaaccttaacactatgtgta

SEQ ID NO: 396 - DNA, 31 bp, Clostridium difficile BI1
  misc_feature 1..31: note = C. difficile Repeat 178
  source 1..31: mol_type = other DNA
attaaaccttaacactatgtgtatttaaatt

SEQ ID NO: 397 - DNA, 30 bp, Clostridium difficile BI1
  misc_feature 1..30: note = C. difficile Repeat 179
  source 1..30: mol_type = other DNA
attaaaccttaacactaagtgtatttgaac

SEQ ID NO: 398 - DNA, 31 bp, Clostridium difficile BI1
  misc_feature 1..31: note = C. difficile Repeat 180
  source 1..31: mol_type = other DNA
attaaaccttaacactacatgtatttaaatc

SEQ ID NO: 399 - DNA, 27 bp, Clostridium difficile BI1
  misc_feature 1..27: note = C. difficile Repeat 181
  source 1..27: mol_type = other DNA
ttgtatagaagcagtaaaacaaaatgg

SEQ ID NO: 400 - DNA, 27 bp, Clostridium difficile BI1
  misc_feature 1..27: note = C. difficile Repeat 182
  source 1..27: mol_type = other DNA
ttgtatagaagcagtaaaacaaaatgg

SEQ ID NO: 401 - DNA, 25 bp, Clostridium difficile BI1
  misc_feature 1..25: note = C. difficile Repeat 183
  source 1..25: mol_type = other DNA
tgtttataatgtggataatatttaa

SEQ ID NO: 402 - DNA, 24 bp, Clostridium difficile BI1
  misc_feature 1..24: note = C. difficile Repeat 184
  source 1..24: mol_type = other DNA
ttgaatggtaaaaaatattacttt

SEQ ID NO: 403 - DNA, 24 bp, Clostridium difficile BI1
  misc_feature 1..24: note = C. difficile Repeat 185
  source 1..24: mol_type = other DNA
ttgaatggtaaaaaatattacttt

SEQ ID NO: 404 - DNA, 24 bp, Clostridium difficile BI1
  misc_feature 1..24: note = C. difficile Repeat 186
  source 1..24: mol_type = other DNA
ttgaatggtaaaaaatattacttt

SEQ ID NO: 405 - DNA, 24 bp, Clostridium difficile BI1
  misc_feature 1..24: note = C. difficile Repeat 187
  source 1..24: mol_type = other DNA
ttgaatggtaaaaaatattacttt

SEQ ID NO: 406 - DNA, 24 bp, Clostridium difficile BI1
  misc_feature 1..24: note = C. difficile Repeat 188
  source 1..24: mol_type = other DNA
ttgaatggtaaaaaatattacttt

SEQ ID NO: 407 - DNA, 24 bp, Clostridium difficile BI1
  misc_feature 1..24: note = C. difficile Repeat 189
  source 1..24: mol_type = other DNA
ttgaatggtaaaaaatattacttt

SEQ ID NO: 408 - DNA, 24 bp, Clostridium difficile BI1
  misc_feature 1..24: note = C. difficile Repeat 190
  source 1..24: mol_type = other DNA
ttgaatggtaaaaaatattacttt

SEQ ID NO: 409 - DNA, 29 bp, Clostridium difficile BI1
  misc_feature 1..29: note = C. difficile Repeat 191
  source 1..29: mol_type = other DNA
gttttatattaactaagtggtatgtaaag

SEQ ID NO: 410 - DNA, 29 bp, Clostridium difficile BI1
  misc_feature 1..29: note = C. difficile Repeat 192
  source 1..29: mol_type = other DNA
gttttatattaactaagtggtatgtaaat

SEQ ID NO: 411 - DNA, 29 bp, Clostridium difficile BI1
  misc_feature 1..29: note = C. difficile Repeat 193
  source 1..29: mol_type = other DNA
gttttatattaactatatggaatgtaaat

SEQ ID NO: 412 - DNA, 29 bp, Clostridium difficile BI1
  misc_feature 1..29: note = C. difficile Repeat 194
  source 1..29: mol_type = other DNA
gttttagattaactatatggaatgtaaat

SEQ ID NO: 413 - DNA, 30 bp, Clostridium difficile BI1; identical to SEQ ID NO: 363
  misc_feature 1..30: note = C. difficile Repeat 195
  source 1..30: mol_type = other DNA

SEQ ID NO: 414 - DNA, 29 bp, Clostridium difficile BI1
  misc_feature 1..29: note = C. difficile Repeat 196
  source 1..29: mol_type = other DNA
gttttatattaactatgtggtatgtaaat

SEQ ID NO: 415 - DNA, 29 bp, Clostridium difficile BI1
  misc_feature 1..29: note = C. difficile Repeat 197
  source 1..29: mol_type = other DNA
ctttacattccatatagttaatataaaac

SEQ ID NO: 416 - DNA, 26 bp, Clostridium difficile BI1
  misc_feature 1..26: note = C. difficile Repeat 198
  source 1..26: mol_type = other DNA
ttaccatctatttgttgccatcctgt

SEQ ID NO: 417 - DNA, 26 bp, Clostridium difficile BI1
  misc_feature 1..26: note = C. difficile Repeat 199
  source 1..26: mol_type = other DNA
tcttctgatggtggtactggtggatt

SEQ ID NO: 418 - DNA, 29 bp, Clostridium difficile BI1
  misc_feature 1..29: note = C. difficile Repeat 200
  source 1..29: mol_type = other DNA
atttacataccacttagttaatataaaac

SEQ ID NO: 419 - DNA, 29 bp, Clostridium difficile BI1
  misc_feature 1..29: note = C. difficile Repeat 201
  source 1..29: mol_type = other DNA
atttataactaacttagtgtaatttaaac

SEQ ID NO: 420 - DNA, 25 bp, Clostridium difficile BI1
  misc_feature 1..25: note = C. difficile Repeat 202
  source 1..25: mol_type = other DNA
tgtttataatgtggataatatttaa

SEQ ID NO: 421 - DNA, 32 bp, Clostridium difficile BI1
  misc_feature 1..32: note = C. difficile Repeat 203
  source 1..32: mol_type = other DNA
atggtaaaaaatattactttaatactaacact

SEQ ID NO: 422 - DNA, 32 bp, Clostridium difficile BI1; identical to SEQ ID NO: 421
  misc_feature 1..32: note = C. difficile Repeat 204
  source 1..32: mol_type = other DNA

SEQ ID NO: 423 - DNA, 47 bp, Clostridium difficile BI1
  misc_feature 1..47: note = C. difficile Repeat 205
  source 1..47: mol_type = other DNA
tagtaataatttatagcaagtaagaaatttaggaagtaggaagttta

SEQ ID NO: 424 - DNA, 29 bp, Clostridium difficile BI1
  misc_feature 1..29: note = C. difficile Repeat 206
  source 1..29: mol_type = other DNA
gttttatattaactatgtggtatgtaaat

SEQ ID NO: 425 - DNA, 29 bp, Clostridium difficile BI1
  misc_feature 1..29: note = C. difficile Repeat 207
  source 1..29: mol_type = other DNA
gttttagattaactatatggaatgtaaat

SEQ ID NO: 426 - DNA, 29 bp, Clostridium difficile BI1
  misc_feature 1..29: note = C. difficile Repeat 208
  source 1..29: mol_type = other DNA
gttttagattaactatatggaatgtaaat

SEQ ID NO: 427 - DNA, 29 bp, Clostridium difficile BI1
  misc_feature 1..29: note = C. difficile Repeat 209
  source 1..29: mol_type = other DNA
gttttatattaactaagtggtatgtaaat

SEQ ID NO: 428 - DNA, 29 bp, Clostridium difficile BI1
  misc_feature 1..29: note = C. difficile Repeat 210
  source 1..29: mol_type = other DNA
gttttatattaactatatggaatgtaaat

SEQ ID NO: 429 - DNA, 29 bp, Clostridium difficile BI1
  misc_feature 1..29: note = C. difficile Repeat 211
  source 1..29: mol_type = other DNA
gttttatattaactaagtggtatgtaaat

SEQ ID NO: 430 - DNA, 29 bp, Clostridium difficile BI1
  misc_feature 1..29: note = C. difficile Repeat 212
  source 1..29: mol_type = other DNA
ttttacattccatatagttaatctaaaac

SEQ ID NO: 431 - DNA, 29 bp, Clostridium difficile BI1
  misc_feature 1..29: note = C. difficile Repeat 213
  source 1..29: mol_type = other DNA
atttacattccatatagttaatataaaac

SEQ ID NO: 432 - DNA, 26 bp, Clostridium difficile BI1
  misc_feature 1..26: note = C. difficile Repeat 214
  source 1..26: mol_type = other DNA
ttaccatctatttgttgccatcctgt

SEQ ID NO: 433 - DNA, 29 bp, Clostridium difficile BI1
  misc_feature 1..29: note = C. difficile Repeat 215
  source 1..29: mol_type = other DNA
atttacataccacttagttaatataaaac

SEQ ID NO: 434 - DNA, 29 bp, Clostridium difficile BI1
  misc_feature 1..29: note = C. difficile Repeat 216
  source 1..29: mol_type = other DNA
atttacataccacttagttaatataaaac

SEQ ID NO: 435 - DNA, 25 bp, Clostridium difficile CD196
  misc_feature 1..25: note = C. difficile Repeat 217
  source 1..25: mol_type = other DNA
tgtttataatgtggataatatttaa

SEQ ID NO: 436 - DNA, 23 bp, Clostridium difficile CD196
  misc_feature 1..23: note = C. difficile Repeat 218
  source 1..23: mol_type = other DNA
tttaatgaagatggtattatgca

SEQ ID NO: 437 - DNA, 24 bp, Clostridium difficile CD196
  misc_feature 1..24: note = C. difficile Repeat 219
  source 1..24: mol_type = other DNA
ttgaatggtaaaaaatattacttt

SEQ ID NO: 438 - DNA, 24 bp, Clostridium difficile CD196
  misc_feature 1..24: note = C. difficile Repeat 220
  source 1..24: mol_type = other DNA
ttgaatggtaaaaaatattacttt

SEQ ID NO: 439 - DNA, 24 bp, Clostridium difficile CD196
  misc_feature 1..24: note = C. difficile Repeat 221
  source 1..24: mol_type = other DNA
ttgaatggtaaaaaatattacttt

SEQ ID NO: 440 - DNA, 24 bp, Clostridium difficile CD196
  misc_feature 1..24: note = C. difficile Repeat 222
  source 1..24: mol_type = other DNA
ttgaatggtaaaaaatattacttt

SEQ ID NO: 441 - DNA, 24 bp, Clostridium difficile CD196
  misc_feature 1..24: note = C. difficile Repeat 223
  source 1..24: mol_type = other DNA
ttgaatggtaaaaaatattacttt

SEQ ID NO: 442 - DNA, 24 bp, Clostridium difficile CD196
  misc_feature 1..24: note = C. difficile Repeat 224
  source 1..24: mol_type = other DNA
ttgaatggtaaaaaatattacttt

SEQ ID NO: 443 - DNA, 24 bp, Clostridium difficile CD196
  misc_feature 1..24: note = C. difficile Repeat 225
  source 1..24: mol_type = other DNA
ttgaatggtaaaaaatattacttt

SEQ ID NO: 444 - DNA, 29 bp, Clostridium difficile CD196
  misc_feature 1..29: note = C. difficile Repeat 226
  source 1..29: mol_type = other DNA
gttttatattaactaagtggtatgtaaag

SEQ ID NO: 445 - DNA, 29 bp, Clostridium difficile CD196
  misc_feature 1..29: note = C. difficile Repeat 227
  source 1..29: mol_type = other DNA
gttttatattaactaagtggtatgtaaat

SEQ ID NO: 446 - DNA, 29 bp, Clostridium difficile CD196
  misc_feature 1..29: note = C. difficile Repeat 228
  source 1..29: mol_type = other DNA
gttttatattaactatatggaatgtaaat

SEQ ID NO: 447 - DNA, 29 bp, Clostridium difficile CD196
  misc_feature 1..29: note = C. difficile Repeat 229
  source 1..29: mol_type = other DNA
gttttagattaactatatggaatgtaaat

SEQ ID NO: 448 - DNA, 30 bp, Clostridium difficile CD196; identical to SEQ ID NO: 363
  misc_feature 1..30: note = C. difficile Repeat 230
  source 1..30: mol_type = other DNA

SEQ ID NO: 449 - DNA, 29 bp, Clostridium difficile CD196
  misc_feature 1..29: note = C. difficile Repeat 231
  source 1..29: mol_type = other DNA
gttttatattaactatgtggtatgtaaat

SEQ ID NO: 450 - DNA, 29 bp, Clostridium difficile CD196
  misc_feature 1..29: note = C. difficile Repeat 232
  source 1..29: mol_type = other DNA
ctttacattccatatagttaatataaaac

SEQ ID NO: 451 - DNA, 29 bp, Clostridium difficile CD196
  misc_feature 1..29: note = C. difficile Repeat 233
  source 1..29: mol_type = other DNA
atttacataccacttagttaatataaaac

SEQ ID NO: 452 - DNA, 29 bp, Clostridium difficile CD196
  misc_feature 1..29: note = C. difficile Repeat 234
  source 1..29: mol_type = other DNA
atttataactaacttagtgtaatttaaac

SEQ ID NO: 453 - DNA, 31 bp, Clostridium difficile CF5
  misc_feature 1..31: note = C. difficile Repeat 235
  source 1..31: mol_type = other DNA
gttggcgctgtgcgttagcactttaagcaac

SEQ ID NO: 454 - DNA, 27 bp, Clostridium difficile CF5
  misc_feature 1..27: note = C. difficile Repeat 236
  source 1..27: mol_type = other DNA
attgatggtaaaaaatattactttaat

SEQ ID NO: 455 - DNA, 27 bp, Clostridium difficile CF5
  misc_feature 1..27: note = C. difficile Repeat 237
  source 1..27: mol_type = other DNA
attgatggtaaaaaatattactttaat

SEQ ID NO: 456 - DNA, 27 bp, Clostridium difficile CF5
  misc_feature 1..27: note = C. difficile Repeat 238
  source 1..27: mol_type = other DNA
attgatggtaaaaaatattactttaat

SEQ ID NO: 457 - DNA, 30 bp, Clostridium difficile CF5
  misc_feature 1..30: note = C. difficile Repeat 239
  source 1..30: mol_type = other DNA
gttttatattaactaagtggtatgtaaata

SEQ ID NO: 458 - DNA, 29 bp, Clostridium difficile CF5
  misc_feature 1..29: note = C. difficile Repeat 240
  source 1..29: mol_type = other DNA
gttttatattaactatatggaatgtaaat

SEQ ID NO: 459 - DNA, 29 bp, Clostridium difficile CF5
  misc_feature 1..29: note = C. difficile Repeat 241
  source 1..29: mol_type = other DNA
gttttagattaactatatggaatgtaaat

SEQ ID NO: 460 - DNA, 29 bp, Clostridium difficile CF5
  misc_feature 1..29: note = C. difficile Repeat 242
  source 1..29: mol_type = other DNA
gttttagattaactatatggaatgtaaat

SEQ ID NO: 461 - DNA, 28 bp, Clostridium difficile CF5
  misc_feature 1..28: note = C. difficile Repeat 243
  source 1..28: mol_type = other DNA
ttttatattaactatgtggtatgtaaat

SEQ ID NO: 462 - DNA, 29 bp, Clostridium difficile CF5
  misc_feature 1..29: note = C. difficile Repeat 244
  source 1..29: mol_type = other DNA
gttttatattaactatgtggtatgtaaat

SEQ ID NO: 463 - DNA, 29 bp, Clostridium difficile CF5
  misc_feature 1..29: note = C. difficile Repeat 245
  source 1..29: mol_type = other DNA
atttacattccatatagttaatataaaac

SEQ ID NO: 464 - DNA, 26 bp, Clostridium difficile CF5
  misc_feature 1..26: note = C. difficile Repeat 246
  source 1..26: mol_type = other DNA
ttaccatctatttgttgccatcctgt

SEQ ID NO: 465 - DNA, 26 bp, Clostridium difficile CF5
  misc_feature 1..26: note = C. difficile Repeat 247
  source 1..26: mol_type = other DNA
tttcttttacagcttctaaacatata

SEQ ID NO: 466 - DNA, 26 bp, Clostridium difficile CF5
  misc_feature 1..26: note = C. difficile Repeat 248
  source 1..26: mol_type = other DNA
tttcttttacagcttctaaacatata

SEQ ID NO: 467 - DNA, 26 bp, Clostridium difficile CF5
  misc_feature 1..26: note = C. difficile Repeat 249
  source 1..26: mol_type = other DNA
tttcttttacagcttctaaacatata

SEQ ID NO: 468 - DNA, 26 bp, Clostridium difficile CF5
  misc_feature 1..26: note = C. difficile Repeat 250
  source 1..26: mol_type = other DNA
tcttctgatggtggtattggtggatt

SEQ ID NO: 469 - DNA, 25 bp, Clostridium difficile M120
  misc_feature 1..25: note = C. difficile Repeat 251
  source 1..25: mol_type = other DNA
tgtttataatgtggataatatttaa

SEQ ID NO: 470 - DNA, 29 bp, Clostridium difficile M120
  misc_feature 1..29: note = C. difficile Repeat 252
  source 1..29: mol_type = other DNA
gttttatattaactaagtggtatgtaaag

SEQ ID NO: 471 - DNA, 33 bp, Clostridium difficile M120
  misc_feature 1..33: note = C. difficile Repeat 253
  source 1..33: mol_type = other DNA
ttatattaacataactatattttacttgataaa

SEQ ID NO: 472 - DNA, 29 bp, Clostridium difficile M120
  misc_feature 1..29: note = C. difficile Repeat 254
  source 1..29: mol_type = other DNA
gttttatattaactatgtggtatgtaaat

SEQ ID NO: 473 - DNA, 29 bp, Clostridium difficile M120
  misc_feature 1..29: note = C. difficile Repeat 255
  source 1..29: mol_type = other DNA
ctttacataccacatagttaatataaaac

SEQ ID NO: 474 - DNA, 29 bp, Clostridium difficile M120
  misc_feature 1..29: note = C. difficile Repeat 256
  source 1..29: mol_type = other DNA
atttacataccacttagttaatataaaac

SEQ ID NO: 475 - DNA, 30 bp, Clostridium difficile M120
  misc_feature 1..30: note = C. difficile Repeat 257
  source 1..30: mol_type = other DNA
atttaaatacatctcatgttactgtttaac

SEQ ID NO: 476 - DNA, 29 bp, Clostridium difficile M120
  misc_feature 1..29: note = C. difficile Repeat 258
  source 1..29: mol_type = other DNA
ctttacataccacttagttaatataaaac

SEQ ID NO: 477 - DNA, 27 bp, Clostridium difficile M68
  misc_feature 1..27: note = C. difficile Repeat 259
  source 1..27: mol_type = other DNA
attgatggtaaaaaatattactttaat

SEQ ID NO: 478 - DNA, 27 bp, Clostridium difficile M68
  misc_feature 1..27: note = C. difficile Repeat 260
  source 1..27: mol_type = other DNA
attgatggtaaaaaatattactttaat

SEQ ID NO: 479 - DNA, 27 bp, Clostridium difficile M68
  misc_feature 1..27: note = C. difficile Repeat 261
  source 1..27: mol_type = other DNA
attgatggtaaaaaatattactttaat

SEQ ID NO: 480 - DNA, 30 bp, Clostridium difficile M68; identical to SEQ ID NO: 457
  misc_feature 1..30: note = C. difficile Repeat 262
  source 1..30: mol_type = other DNA

SEQ ID NO: 481 - DNA, 29 bp, Clostridium difficile M68
  misc_feature 1..29: note = C. difficile Repeat 263
  source 1..29: mol_type = other DNA
gttttatattaactatatggaatgtaaat

SEQ ID NO: 482 - DNA, 29 bp, Clostridium difficile M68
  misc_feature 1..29: note = C. difficile Repeat 264
  source 1..29: mol_type = other DNA
gttttatattaactatatggaatgtaaat

SEQ ID NO: 483 - DNA, 28 bp, Clostridium difficile M68
  misc_feature 1..28: note = C. difficile Repeat 265
  source 1..28: mol_type = other DNA
gttttagattaactatatggaatgtaaa

SEQ ID NO: 484 - DNA, 28 bp, Clostridium difficile M68
  misc_feature 1..28: note = C. difficile Repeat 266
  source 1..28: mol_type = other DNA
ttttatattaactatgtggtatgtaaat

SEQ ID NO: 485 - DNA, 29 bp, Clostridium difficile M68
  misc_feature 1..29: note = C. difficile Repeat 267
  source 1..29: mol_type = other DNA
gttttatattaactatgtggtatgtaaat

SEQ ID NO: 486 - DNA, 29 bp, Clostridium difficile M68
  misc_feature 1..29: note = C. difficile Repeat 268
  source 1..29: mol_type = other DNA
atttacattccatatagttaatataaaac

SEQ ID NO: 487 - DNA, 26 bp, Clostridium difficile M68
  misc_feature 1..26: note = C. difficile Repeat 269
  source 1..26: mol_type = other DNA
ttaccatctatttgttgccatcctgt

SEQ ID NO: 488 - DNA, 26 bp, Clostridium difficile M68
  misc_feature 1..26: note = C. difficile Repeat 270
  source 1..26: mol_type = other DNA
tttcttttacagcttctaaacatata

SEQ ID NO: 489 - DNA, 26 bp, Clostridium difficile M68
  misc_feature 1..26: note = C. difficile Repeat 271
  source 1..26: mol_type = other DNA
tttcttttacagcttctaaacatata

SEQ ID NO: 490 - DNA, 27 bp, Clostridium difficile M68
  misc_feature 1..27: note = C. difficile Repeat 272
  source 1..27: mol_type = other DNA
attccgttgcttaaagtgctaacgcac

SEQ ID NO: 491 - DNA, 31 bp, Clostridium difficile M68
  misc_feature 1..31: note = C. difficile Repeat 273
  source 1..31: mol_type = other DNA
gttggcgctgtgcgttagtactttaagcaac

SEQ ID NO: 492 - DNA, 31 bp, Clostridium difficile M68; identical to SEQ ID NO: 453
  misc_feature 1..31: note = C. difficile Repeat 274
  source 1..31: mol_type = other DNA

SEQ ID NO: 493 - DNA, 31 bp, Clostridium difficile M68; identical to SEQ ID NO: 453
  misc_feature 1..31: note = C. difficile Repeat 275
  source 1..31: mol_type = other DNA

SEQ ID NO: 494 - DNA, 31 bp, Clostridium difficile M68; identical to SEQ ID NO: 453
  misc_feature 1..31: note = C. difficile Repeat 276
  source 1..31: mol_type = other DNA

SEQ ID NO: 495 - DNA, 27 bp, Clostridium difficile M68
  misc_feature 1..27: note = C. difficile Repeat 277
  source 1..27: mol_type = other DNA
attccgttgcttaaagtgctaacgcac

SEQ ID NO: 496 - DNA, 25 bp, Clostridium difficile R20291
  misc_feature 1..25: note = C. difficile Repeat 278
  source 1..25: mol_type = other DNA
tgtttataatgtggataatatttaa

SEQ ID NO: 497 - DNA, 23 bp, Clostridium difficile R20291
  misc_feature 1..23: note = C. difficile Repeat 279
  source 1..23: mol_type = other DNA
tttaatgaagatggtattatgca

SEQ ID NO: 498 - DNA, 24 bp, Clostridium difficile R20291
  misc_feature 1..24: note = C. difficile Repeat 280
  source 1..24: mol_type = other DNA
ttgaatggtaaaaaatattacttt

SEQ ID NO: 499 - DNA, 24 bp, Clostridium difficile R20291
  misc_feature 1..24: note = C. difficile Repeat 281
  source 1..24: mol_type = other DNA
ttgaatggtaaaaaatattacttt

SEQ ID NO: 500 - DNA, 24 bp, Clostridium difficile R20291
  misc_feature 1..24: note = C. difficile Repeat 282
  source 1..24: mol_type = other DNA
ttgaatggtaaaaaatattacttt

SEQ ID NO: 501 - DNA, 24 bp, Clostridium difficile R20291
  misc_feature 1..24: note = C. difficile Repeat 283
  source 1..24: mol_type = other DNA
ttgaatggtaaaaaatattacttt

SEQ ID NO: 502 - DNA, 24 bp, Clostridium difficile R20291
  misc_feature 1..24: note = C. difficile Repeat 284
  source 1..24: mol_type = other DNA
ttgaatggtaaaaaatattacttt

SEQ ID NO: 503 - DNA, 24 bp, Clostridium difficile R20291
  misc_feature 1..24: note = C. difficile Repeat 285
  source 1..24: mol_type = other DNA
ttgaatggtaaaaaatattacttt

SEQ ID NO: 504 - DNA, 24 bp, Clostridium difficile R20291
  misc_feature 1..24: note = C. difficile Repeat 286
  source 1..24: mol_type = other DNA
ttgaatggtaaaaaatattacttt

SEQ ID NO: 505 - DNA, 29 bp, Clostridium difficile R20291
  misc_feature 1..29: note = C. difficile Repeat 287
  source 1..29: mol_type = other DNA
gttttatattaactaagtggtatgtaaag

SEQ ID NO: 506 - DNA, 29 bp, Clostridium difficile R20291
  misc_feature 1..29: note = C. difficile Repeat 288
  source 1..29: mol_type = other DNA
gttttatattaactaagtggtatgtaaat

SEQ ID NO: 507 - DNA, 29 bp, Clostridium difficile R20291
  misc_feature 1..29: note = C. difficile Repeat 289
  source 1..29: mol_type = other DNA
gttttatattaactatatggaatgtaaat

SEQ ID NO: 508 - DNA, 29 bp, Clostridium difficile R20291
  misc_feature 1..29: note = C. difficile Repeat 290
  source 1..29: mol_type = other DNA
gttttagattaactatatggaatgtaaat

SEQ ID NO: 509 - DNA, 30 bp, Clostridium difficile R20291; identical to SEQ ID NO: 363
  misc_feature 1..30: note = C. difficile Repeat 291
  source 1..30: mol_type = other DNA

SEQ ID NO: 510 - DNA, 29 bp, Clostridium difficile R20291
  misc_feature 1..29: note = C. difficile Repeat 292
  source 1..29: mol_type = other DNA
gttttatattaactatgtggtatgtaaat

SEQ ID NO: 511 - DNA, 29 bp, Clostridium difficile R20291
  misc_feature 1..29: note = C. difficile Repeat 293
  source 1..29: mol_type = other DNA
ctttacattccatatagttaatataaaac

SEQ ID NO: 512 - DNA, 29 bp, Clostridium difficile R20291
  misc_feature 1..29: note = C. difficile Repeat 294
  source 1..29: mol_type = other DNA
atttacataccacttagttaatataaaac

SEQ ID NO: 513 - DNA, 29 bp, Clostridium difficile R20291
  misc_feature 1..29: note = C. difficile Repeat 295
  source 1..29: mol_type = other DNA
atttataactaacttagtgtaatttaaac

SEQ ID NO: 514 - DNA, 42 bp, Escherichia coli 042
  misc_feature 1..42: note = E. coli Repeat 5
  source 1..42: mol_type = other DNA
tgccggatgcggcgtgaacgccttatccggcctacgagtggc

SEQ ID NO: 515 - DNA, 47 bp, Escherichia coli 042
  misc_feature 1..47: note = E. coli Repeat 6
  source 1..47: mol_type = other DNA
gccggatgcggcgtgaacgccttatccggcctacaaaagaaatgcag

SEQ ID NO: 516 - DNA, 28 bp, Escherichia coli 042
  misc_feature 1..28: note = E. coli Repeat 7
  source 1..28: mol_type = other DNA
gttcactgccgtacaggcagcttagaaa

SEQ ID NO: 517 - DNA, 39 bp, Escherichia coli 042
  misc_feature 1..39: note = E. coli Repeat 8
  source 1..39: mol_type = other DNA
tttgtaggcctgataagacgcgccagcgtcgcatcaggc

SEQ ID NO: 518 - DNA, 29 bp, Escherichia coli 042
  misc_feature 1..29: note = E. coli Repeat 9
  source 1..29: mol_type = other DNA
cggtttatccccgctgacgcggggaacac

SEQ ID NO: 519 - DNA, 39 bp, Escherichia coli 1303; identical to SEQ ID NO: 517
  misc_feature 1..39: note = E. coli Repeat 10
  source 1..39: mol_type = other DNA

SEQ ID NO: 520 - DNA, 29 bp, Escherichia coli 1303
  misc_feature 1..29: note = E. coli Repeat 11
  source 1..29: mol_type = other DNA
cggtttatccccgctggcgcggggaacac

SEQ ID NO: 521 - DNA, 29 bp, Escherichia coli 1303
  misc_feature 1..29: note = E. coli Repeat 12
  source 1..29: mol_type = other DNA
cggtttatccccgctggcgcggggaacac

SEQ ID NO: 522 - DNA, 43 bp, Escherichia coli 536
  misc_feature 1..43: note = E. coli Repeat 13
  source 1..43: mol_type = other DNA
gccggatgcggcgtgaacgccttatccggcctacgaatggcgc

SEQ ID NO: 523 - DNA, 47 bp, Escherichia coli 536; identical to SEQ ID NO: 515
  misc_feature 1..47: note = E. coli Repeat 14
  source 1..47: mol_type = other DNA

SEQ ID NO: 524 - DNA, 28 bp, Escherichia coli 536
  misc_feature 1..28: note = E. coli Repeat 15
  source 1..28: mol_type = other DNA
gttcactgccgtacaggcagcttagaaa

SEQ ID NO: 525 - DNA, 33 bp, Escherichia coli 536
  misc_feature 1..33: note = E. coli Repeat 16
  source 1..33: mol_type = other DNA
tttgtaggccggataagcgaagcgcatccggca

SEQ ID NO: 526 - DNA, 38 bp, Escherichia coli 536
  misc_feature 1..38: note = E. coli Repeat 17
  source 1..38: mol_type = other DNA
cgcctgatgcgacgctgtcgcgtcttatcaggcctaca

SEQ ID NO: 527 - DNA, 44 bp, Escherichia coli 536
  misc_feature 1..44: note = E. coli Repeat 18
  source 1..44: mol_type = other DNA
tgtgtaggtcggataaggcgttcacgccgcatccgacaataaca

SEQ ID NO: 528 - DNA, 29 bp, Escherichia coli 55989
  misc_feature 1..29: note = E. coli Repeat 19
  source 1..29: mol_type = other DNA
cggtttatccccgctggcgcggggaacac

SEQ ID NO: 529 - DNA, 29 bp, Escherichia coli 55989
  misc_feature 1..29: note = E. coli Repeat 20
  source 1..29: mol_type = other DNA
cggtttatccccgctggcgcggggaactc

SEQ ID NO: 530 - DNA, 30 bp, Escherichia coli ACN001
  misc_feature 1..30: note = E. coli Repeat 21
  source 1..30: mol_type = other DNA
cggtttatccccgctggcgcggggaacaca

SEQ ID NO: 531 - DNA, 29 bp, Escherichia coli ACN001
  misc_feature 1..29: note = E. coli Repeat 22
  source 1..29: mol_type = other DNA
cggtttatccccgctggcgcggggaactc

SEQ ID NO: 532 - DNA, 49 bp, Escherichia coli ACN001
  misc_feature 1..49: note = E. coli Repeat 23
  source 1..49: mol_type = other DNA
tctgtgtcggtcggataaggcgttcacgccgcatccgacaataacaaca

SEQ ID NO: 533 - DNA, 37 bp, Escherichia coli APEC IMT5155
  misc_feature 1..37: note = E. coli Repeat 24
  source 1..37: mol_type = other DNA
gcctgatgcgacgctgtcgcgtcttatcaggcctaca

SEQ ID NO: 534 - DNA, 44 bp, Escherichia coli APEC IMT5155
  misc_feature 1..44: note = E. coli Repeat 25
  source 1..44: mol_type = other DNA
tgtgtaggtcggataaggcgttcacgtcgcatccgacaataaca

SEQ ID NO: 535 - DNA, 47 bp, Escherichia coli APEC IMT5155; identical to SEQ ID NO: 515
  misc_feature 1..47: note = E. coli Repeat 26
  source 1..47: mol_type = other DNA

SEQ ID NO: 536 - DNA, 28 bp, Escherichia coli APEC IMT5155
  misc_feature 1..28: note = E. coli Repeat 27
  source 1..28: mol_type = other DNA
gttcactgccgtacaggcagcttagaaa

SEQ ID NO: 537 - DNA, 28 bp, Escherichia coli APEC IMT5155
  misc_feature 1..28: note = E. coli Repeat 27
  source 1..28: mol_type = other DNA
gttcactgccgtacaggcagcttagaaa

SEQ ID NO: 538 - DNA, 47 bp, Escherichia coli APEC O1; identical to SEQ ID NO: 515
  misc_feature 1..47: note = E. coli Repeat 28
  source 1..47: mol_type = other DNA

SEQ ID NO: 539 - DNA, 28 bp, Escherichia coli APEC O1
  misc_feature 1..28: note = E. coli Repeat 29
  source 1..28: mol_type = other DNA
gttcactgccgtacaggcagcttagaaa

SEQ ID NO: 540 - DNA, 28 bp, Escherichia coli APEC O1
  misc_feature 1..28: note = E. coli Repeat 30
  source 1..28: mol_type = other DNA
gttcactgccgtacaggcagcttagaaa

SEQ ID NO: 541 - DNA, 37 bp, Escherichia coli APEC O1; identical to SEQ ID NO: 533
  misc_feature 1..37: note = E. coli Repeat 31
  source 1..37: mol_type = other DNA

SEQ ID NO: 542 - DNA, 44 bp, Escherichia coli APEC O1; identical to SEQ ID NO: 534
  misc_feature 1..44: note = E. coli Repeat 32
  source 1..44: mol_type = other DNA

SEQ ID NO: 543 - DNA, 49 bp, Escherichia coli APEC O78; identical to SEQ ID NO: 532
  misc_feature 1..49: note = E. coli Repeat 33
  source 1..49: mol_type = other DNA

SEQ ID NO: 544 - DNA, 30 bp, Escherichia coli APEC O78; identical to SEQ ID NO: 530
  misc_feature 1..30: note = E. coli Repeat 34
  source 1..30: mol_type = other DNA

SEQ ID NO: 545 - DNA, 29 bp, Escherichia coli APEC O78
  misc_feature 1..29: note = E. coli Repeat 35
  source 1..29: mol_type = other DNA
cggtttatccccgctggcgcggggaactc

SEQ ID NO: 546 - DNA, 43 bp, Escherichia coli B
  misc_feature 1..43: note = E. coli Repeat 36
  source 1..43: mol_type = other DNA
atgcctgatgcgacgcttgccgcgtcttatcaggcctacaaaa

SEQ ID NO: 547 - DNA, 50 bp, Escherichia coli B
  misc_feature 1..50: note = E. coli Repeat 37
  source 1..50: mol_type = other DNA
ctacggctcggtttgtaggcctgataagacgcgccagcgtcgcatcaggc

SEQ ID NO: 548 - DNA, 45 bp, Escherichia coli B
  misc_feature 1..45: note = E. coli Repeat 38
  source 1..45: mol_type = other DNA
cacaatgcctgatgcgacgctggagcgtcttatcatgcctacaaa

SEQ ID NO: 549 - DNA, 29 bp, Escherichia coli B
  misc_feature 1..29: note = E. coli Repeat 39
  source 1..29: mol_type = other DNA
cggtttatccccgctggcgcggggaacac

SEQ ID NO: 550 - DNA, 29 bp, Escherichia coli B
  misc_feature 1..29: note = E. coli Repeat 40
  source 1..29: mol_type = other DNA
cggtttatccccgctggcgcggggaacac

SEQ ID NO: 551 - DNA, 43 bp, Escherichia coli B; identical to SEQ ID NO: 546
  misc_feature 1..43: note = E. coli Repeat 41
  source 1..43: mol_type = other DNA

SEQ ID NO: 552 - DNA, 50 bp, Escherichia coli B; identical to SEQ ID NO: 547
  misc_feature 1..50: note = E. coli Repeat 42
  source 1..50: mol_type = other DNA

SEQ ID NO: 553 - DNA, 45 bp, Escherichia coli B; identical to SEQ ID NO: 548
  misc_feature 1..45: note = E. coli Repeat 43
  source 1..45: mol_type = other DNA

SEQ ID NO: 554 - DNA, 29 bp, Escherichia coli B
  misc_feature 1..29: note = E. coli Repeat 44
  source 1..29: mol_type = other DNA
cggtttatccccgctggcgcggggaacac

SEQ ID NO: 555 - DNA, 29 bp, Escherichia coli B
  misc_feature 1..29: note = E. coli Repeat 45
  source 1..29: mol_type = other DNA
cggtttatccccgctggcgcggggaacac

SEQ ID NO: 556 - DNA, 43 bp, Escherichia coli B str. REL606; identical to SEQ ID NO: 546
  misc_feature 1..43: note = E. coli Repeat 46
  source 1..43: mol_type = other DNA

SEQ ID NO: 557 - DNA, 50 bp, Escherichia coli B str. REL606; identical to SEQ ID NO: 547
  misc_feature 1..50: note = E. coli Repeat 47
  source 1..50: mol_type = other DNA

SEQ ID NO: 558 - DNA, 45 bp, Escherichia coli B str. REL606; identical to SEQ ID NO: 548
  misc_feature 1..45: note = E. coli Repeat 48
  source 1..45: mol_type = other DNA

SEQ ID NO: 559 - DNA, 29 bp, Escherichia coli B str. REL606
  misc_feature 1..29: note = E. coli Repeat 49
  source 1..29: mol_type = other DNA
cggtttatccccgctggcgcggggaacac

SEQ ID NO: 560 - DNA, 29 bp, Escherichia coli B str. REL606
  misc_feature 1..29: note = E. coli Repeat 50
  source 1..29: mol_type = other DNA
cggtttatccccgctggcgcggggaacac

SEQ ID NO: 561 - DNA, 43 bp, Escherichia coli BL21; identical to SEQ ID NO: 546
  misc_feature 1..43: note = E. coli Repeat 51
  source 1..43: mol_type = other DNA

SEQ ID NO: 562 - DNA, 50 bp, Escherichia coli BL21; identical to SEQ ID NO: 547
  misc_feature 1..50: note = E. coli Repeat 52
  source 1..50: mol_type = other DNA

SEQ ID NO: 563 - DNA, 45 bp, Escherichia coli BL21; identical to SEQ ID NO: 548
  misc_feature 1..45: note = E. coli Repeat 53
  source 1..45: mol_type = other DNA

SEQ ID NO: 564 - DNA, 29 bp, Escherichia coli BL21
  misc_feature 1..29: note = E. coli Repeat 54
  source 1..29: mol_type = other DNA
cggtttatccccgctggcgcggggaacac

SEQ ID NO: 565 - DNA, 29 bp, Escherichia coli BL21
  misc_feature 1..29: note = E. coli Repeat 55
  source 1..29: mol_type = other DNA
cggtttatccccgctggcgcggggaacac

SEQ ID NO: 566 - DNA, 29 bp, Escherichia coli BL21
  misc_feature 1..29: note = E. coli Repeat 56
  source 1..29: mol_type = other DNA
gtgttccccgcgccagcggggataaaccg

SEQ ID NO: 567 - DNA, 29 bp, Escherichia coli BL21
  misc_feature 1..29: note = E. coli Repeat 57
  source 1..29: mol_type = other DNA
gtgttccccgcgccagcggggataaaccg

SEQ ID NO: 568 - DNA, 43 bp, Escherichia coli BL21
  misc_feature 1..43: note = E. coli Repeat 58
  source 1..43: mol_type = other DNA
ttttgcaggcctgataagacgcggcaagcgtcgcatcaggcat

SEQ ID NO: 569 - DNA, 45 bp, Escherichia coli BL21
  misc_feature 1..45: note = E. coli Repeat 59
  source 1..45: mol_type = other DNA
taaaccgtaggcctgataagacgcgcaaagcgtcgcatcaggcat

SEQ ID NO: 570 - DNA, 43 bp, Escherichia coli BL21; identical to SEQ ID NO: 546
  misc_feature 1..43: note = E. coli Repeat 60
  source 1..43: mol_type = other DNA

SEQ ID NO: 571 - DNA, 50 bp, Escherichia coli BL21; identical to SEQ ID NO: 547
  misc_feature 1..50: note = E. coli Repeat 61
  source 1..50: mol_type = other DNA

SEQ ID NO: 572 - DNA, 45 bp, Escherichia coli BL21; identical to SEQ ID NO: 548
  misc_feature 1..45: note = E. coli Repeat 62
  source 1..45: mol_type = other DNA

SEQ ID NO: 573 - DNA, 29 bp, Escherichia coli BL21
  misc_feature 1..29: note = E. coli Repeat 63
  source 1..29: mol_type = other DNA
cggtttatccccgctggcgcggggaacac

SEQ ID NO: 574 - DNA, 29 bp, Escherichia coli BL21
  misc_feature 1..29: note = E. coli Repeat 64
  source 1..29: mol_type = other DNA
cggtttatccccgctggcgcggggaacac

SEQ ID NO: 575 - DNA, 43 bp, Escherichia coli BW25113; identical to SEQ ID NO: 546
  misc_feature 1..43: note = E. coli Repeat 65
  source 1..43: mol_type = other DNA

SEQ ID NO: 576 - DNA, 39 bp, Escherichia coli BW25113; identical to SEQ ID NO: 517
  misc_feature 1..39: note = E. coli Repeat 66
  source 1..39: mol_type = other DNA

SEQ ID NO: 577 - DNA, 29 bp, Escherichia coli BW25113
  misc_feature 1..29: note = E. coli Repeat 67
  source 1..29: mol_type = other DNA
cggtttatccccgctggcgcggggaactc

SEQ ID NO: 578 - DNA, 28 bp, Escherichia coli BW25113
  misc_feature 1..28: note = E. coli Repeat 68
  source 1..28: mol_type = other DNA
ggtttatccccgctggcgcggggaacac

SEQ ID NO: 579 - DNA, 43 bp, Escherichia coli BW2952; identical to SEQ ID NO: 546
  misc_feature 1..43: note = E. coli Repeat 69
  source 1..43: mol_type = other DNA

SEQ ID NO: 580 - DNA, 39 bp, Escherichia coli BW2952; identical to SEQ ID NO: 517
  misc_feature 1..39: note = E. coli Repeat 70
  source 1..39: mol_type = other DNA

SEQ ID NO: 581 - DNA, 29 bp, Escherichia coli BW2952
  misc_feature 1..29: note = E. coli Repeat 71
  source 1..29: mol_type = other DNA
cggtttatccccgctggcgcggggaactc

SEQ ID NO: 582 - DNA, 28 bp, Escherichia coli BW2952
  misc_feature 1..28: note = E. coli Repeat 72
  source 1..28: mol_type = other DNA
ggtttatccccgctggcgcggggaacac

SEQ ID NO: 583 - DNA, 29 bp, Escherichia coli C str. ATTC 8739
  misc_feature 1..29: note = E. coli Repeat 73
  source 1..29: mol_type = other DNA
gagttccccgcgccagcggggataaaccg

SEQ ID NO: 584 - DNA, 29 bp, Escherichia coli C str. ATTC 8739
  misc_feature 1..29: note = E. coli Repeat 74
  source 1..29: mol_type = other DNA
gagttccccgcgccagcggggataaaccg

SEQ ID NO: 585 - DNA, 29 bp, Escherichia coli C str. ATTC 8739
  misc_feature 1..29: note = E. coli Repeat 75
  source 1..29: mol_type = other DNA
gagttccccgcgccagcggggataaaccg

SEQ ID NO: 586 - DNA, 28 bp, Escherichia coli C str. ATTC 8739
  misc_feature 1..28: note = E. coli Repeat 76
  source 1..28: mol_type = other DNA
tttctaagctgcctgtacggcagtgaac

SEQ ID NO: 587 - DNA, 43 bp, Escherichia coli C str. ATTC 8739
  misc_feature 1..43: note = E. coli Repeat 77
  source 1..43: mol_type = other DNA
ttttgtaggcctgataagacgcgacaagcgtcgcatcaggcat

SEQ ID NO: 588 - DNA, 45 bp, Escherichia coli C str. ATTC 8739; identical to SEQ ID NO: 569
  misc_feature 1..45: note = E. coli Repeat 78
  source 1..45: mol_type = other DNA

SEQ ID NO: 589 - DNA, 41 bp, Escherichia coli DH1
  misc_feature 1..41: note = E. coli Repeat 79
  source 1..41: mol_type = other DNA
cacgccgcatccgccagtggcgcggtgcagatgccggatgc

SEQ ID NO: 590 - DNA, 28 bp, Escherichia coli DH1
  misc_feature 1..28: note = E. coli Repeat 80
  source 1..28: mol_type = other DNA
gtgttccccgcgccagcggggataaacc

SEQ ID NO: 591 - DNA, 29 bp, Escherichia coli DH1
  misc_feature 1..29: note = E. coli Repeat 81
  source 1..29: mol_type = other DNA
gagttccccgcgccagcggggataaaccg

SEQ ID NO: 592 - DNA, 43 bp, Escherichia coli DH1; identical to SEQ ID NO: 568
  misc_feature 1..43: note = E. coli Repeat 82
  source 1..43: mol_type = other DNA

SEQ ID NO: 593 - DNA, 41 bp, Escherichia coli DH1
  misc_feature 1..41: note = E. coli Repeat 83
  source 1..41: mol_type = other DNA
ccgtaggcctgataagacgcgcaaagcgtcgcatcaggcat

SEQ ID NO: 594 - DNA, 43 bp, Escherichia coli DH1; identical to SEQ ID NO: 546
  misc_feature 1..43: note = E. coli Repeat 84
  source 1..43: mol_type = other DNA

SEQ ID NO: 595 - DNA, 39 bp, Escherichia coli DH1; identical to SEQ ID NO: 517
  misc_feature 1..39: note = E. coli Repeat 85
  source 1..39: mol_type = other DNA

SEQ ID NO: 596 - DNA, 29 bp, Escherichia coli DH1
  misc_feature 1..29: note = E. coli Repeat 86
  source 1..29: mol_type = other DNA
cggtttatccccgctggcgcggggaactc

SEQ ID NO: 597 - DNA, 28 bp, Escherichia coli DH1
  misc_feature 1..28: note = E. coli Repeat 87
  source 1..28: mol_type = other DNA
ggtttatccccgctggcgcggggaacac

SEQ ID NO: 598 - DNA, 29 bp, Escherichia coli E24377A
  misc_feature 1..29: note = E. coli Repeat 88
  source 1..29: mol_type = other DNA
gttcactgccgtacaggcagcttagaaat

SEQ ID NO: 599 - DNA, 29 bp, Escherichia coli E24377A
  misc_feature 1..29: note = E. coli Repeat 89
  source 1..29: mol_type = other DNA
cggtttatccccgctggcgcggggaacac

SEQ ID NO: 600 - DNA, 29 bp, Escherichia coli E24377A
  misc_feature 1..29: note = E. coli Repeat 90
  source 1..29: mol_type = other DNA
cggtttatccccgctggcgcggggaacac

SEQ ID NO: 601 - DNA, 29 bp, Escherichia coli ECC-1470
  misc_feature 1..29: note = E. coli Repeat 91
  source 1..29: mol_type = other DNA
gttcactgccgtacaggcagcttagaaat

SEQ ID NO: 602 - DNA, 29 bp, Escherichia coli ECC-1470
  misc_feature 1..29: note = E. coli Repeat 92
  source 1..29: mol_type = other DNA
cggtttatccccgctggcgcggggaacac

SEQ ID NO: 603 - DNA, 29 bp, Escherichia coli ECC-1470
  misc_feature 1..29: note = E. coli Repeat 93
  source 1..29: mol_type = other DNA
cggtttatccccgctggcgcggggaacac

SEQ ID NO: 604 - DNA, 43 bp, Escherichia coli ED1a; identical to SEQ ID NO: 522
  misc_feature 1..43: note = E. coli Repeat 94
  source 1..43: mol_type = other DNA

SEQ ID NO: 605 - DNA, 28 bp, Escherichia coli ED1a
  misc_feature 1..28: note = E. coli Repeat 95
  source 1..28: mol_type = other DNA
gttcactgccgtacaggcagcttagaaa

SEQ ID NO: 606 - DNA, 28 bp, Escherichia coli ED1a
  misc_feature 1..28: note = E. coli Repeat 96
  source 1..28: mol_type = other DNA
gttcactgccgtacaggcagcttagaaa

SEQ ID NO: 607 - DNA, 33 bp, Escherichia coli ED1a; identical to SEQ ID NO: 525
  misc_feature 1..33: note = E. coli Repeat 97
  source 1..33: mol_type = other DNA

SEQ ID NO: 608 - DNA, 46 bp, Escherichia coli ED1a
  misc_feature 1..46: note = E. coli Repeat 98
  source 1..46: mol_type = other DNA
tgtgtaggtcggataaggcgttcacgtcgcatccgacaataacaac

SEQ ID NO: 609 - DNA, 43 bp, Escherichia coli ER2796; identical to SEQ ID NO: 546
  misc_feature 1..43: note = E. coli Repeat 99
  source 1..43: mol_type = other DNA

SEQ ID NO: 610 - DNA, 39 bp, Escherichia coli ER2796; identical to SEQ ID NO: 517
  misc_feature 1..39: note = E. coli Repeat 100
  source 1..39: mol_type = other DNA

SEQ ID NO: 611 - DNA, 29 bp, Escherichia coli ER2796
  misc_feature 1..29: note = E. coli Repeat 101
  source 1..29: mol_type = other DNA
cggtttatccccgctggcgcggggaactc

SEQ ID NO: 612 - DNA, 28 bp, Escherichia coli ER2796
  misc_feature 1..28: note = E. coli Repeat 102
  source 1..28: mol_type = other DNA
ggtttatccccgctggcgcggggaacac

SEQ ID NO: 613 - DNA, 43 bp, Escherichia coli ETEC H10407; identical to SEQ ID NO: 546
  misc_feature 1..43: note = E. coli Repeat 103
  source 1..43: mol_type = other DNA

SEQ ID NO: 614 - DNA, 39 bp, Escherichia coli ETEC H10407
  misc_feature 1..39: note = E. coli Repeat 104
  source 1..39: mol_type = other DNA
atgctgccaacttactgatttagtgtatgatggtgtttt

SEQ ID NO: 615 - DNA, 39 bp, Escherichia coli ETEC H10407; identical to SEQ ID NO: 517
  misc_feature 1..39: note = E. coli Repeat 105
  source 1..39: mol_type = other DNA

SEQ ID NO: 616 - DNA, 45 bp, Escherichia coli ETEC H10407; identical to SEQ ID NO: 548
  misc_feature 1..45: note = E. coli Repeat 106
  source 1..45: mol_type = other DNA

SEQ ID NO: 617 - DNA, 30 bp, Escherichia coli ETEC H10407
  misc_feature 1..30: note = E. coli Repeat 107
  source 1..30: mol_type = other DNA
acggtttatccccgctggcgcggggaactc

SEQ ID NO: 618 - DNA, 29 bp, Escherichia coli ETEC H10407
  misc_feature 1..29: note = E. coli Repeat 108
  source 1..29: mol_type = other DNA
cggtttatccccgctggcgcggggaacac

SEQ ID NO: 619 - DNA, 28 bp, Escherichia coli
  misc_feature 1..28: note = E. coli Repeat 109
  source 1..28: mol_type = other DNA
tttctaagctgcctgtacggcagtgaac

SEQ ID NO: 620 - DNA, 43 bp, Escherichia coli; identical to SEQ ID NO: 587
  misc_feature 1..43: note = E. coli Repeat 110
  source 1..43: mol_type = other DNA

SEQ ID NO: 621 - DNA, 40 bp, Escherichia coli
  misc_feature 1..40: note = E. coli Repeat 111
  source 1..40: mol_type = other DNA
gctggagagcaaccgtaggccggataagatgcgccagcat

SEQ ID NO: 622 - DNA, 29 bp, Escherichia coli
  misc_feature 1..29: note = E. coli Repeat 112
  source 1..29: mol_type = other DNA
gtgttccccgcgccagcggggataaaccg

SEQ ID NO: 623 - DNA, 29 bp, Escherichia coli
  misc_feature 1..29: note = E. coli Repeat 113
  source 1..29: mol_type = other DNA
gtgttccccgcgccagcggggataaaccg

SEQ ID NO: 624 - DNA, 39 bp, Escherichia coli; identical to SEQ ID NO: 517
  misc_feature 1..39: note = E. coli Repeat 114
  source 1..39: mol_type = other DNA

SEQ ID NO: 625 - DNA, 29 bp, Escherichia coli
  misc_feature 1..29: note = E. coli Repeat 115
  source 1..29: mol_type = other DNA
gtgttccccgcgccagcggggataaaccg

SEQ ID NO: 626 - DNA, 29 bp, Escherichia coli
  misc_feature 1..29: note = E. coli Repeat 116
  source 1..29: mol_type = other DNA
gtgttccccgcgccagcggggataaaccg

SEQ ID NO: 627 - DNA, 28 bp, Escherichia coli
  misc_feature 1..28: note = E. coli Repeat 117
  source 1..28: mol_type = other DNA
tttctaagctgcctgtacggcagtgaac

SEQ ID NO: 628 - DNA, 43 bp, Escherichia coli; identical to SEQ ID NO: 587
  misc_feature 1..43: note = E. coli Repeat 118
  source 1..43: mol_type = other DNA

SEQ ID NO: 629 - DNA, 40 bp, Escherichia coli; identical to SEQ ID NO: 621
  misc_feature 1..40: note = E. coli Repeat 119
  source 1..40: mol_type = other DNA

SEQ ID NO: 630 - DNA, 29 bp, Escherichia coli
  misc_feature 1..29: note = E. coli Repeat 120
  source 1..29: mol_type = other DNA
gtgttccccgcgccagcggggataaaccg

SEQ ID NO: 631 - DNA, 29 bp, Escherichia coli
  misc_feature 1..29: note = E. coli Repeat 121
  source 1..29: mol_type = other DNA
gtgttccccgcgccagcggggataaaccg

SEQ ID NO: 632 - DNA, 28 bp, Escherichia coli
  misc_feature 1..28: note = E. coli Repeat 122
  source 1..28: mol_type = other DNA
tttctaagctgcctgtacggcagtgaac

SEQ ID NO: 633 - DNA, 43 bp, Escherichia coli; identical to SEQ ID NO: 587
  misc_feature 1..43: note = E. coli Repeat 123
  source 1..43: mol_type = other DNA

SEQ ID NO: 634 - DNA, 40 bp, Escherichia coli; identical to SEQ ID NO: 621
  misc_feature 1..40: note = E. coli Repeat 124
  source 1..40: mol_type = other DNA

SEQ ID NO: 635 - DNA, 26 bp, Escherichia coli
  misc_feature 1..26: note = E. coli Repeat 125
  source 1..26: mol_type = other DNA
cggtttatccccgctggccggggaac

SEQ ID NO: 636 - DNA, 29 bp, Escherichia coli
  misc_feature 1..29: note = E. coli Repeat 126
  source 1..29: mol_type = other DNA
cggtttatccccgctggcgcggggaactc

SEQ ID NO: 637 - DNA, 26 bp, Escherichia coli
  misc_feature 1..26: note = E. coli Repeat 127
  source 1..26: mol_type = other DNA
cggtttatccccgctggccggggaac

SEQ ID NO: 638 - DNA, 29 bp, Escherichia coli
  misc_feature 1..29: note = E. coli Repeat 128
  source 1..29: mol_type = other DNA
cggtttatccccgctggcgcggggaactc

SEQ ID NO: 639 - DNA, 26 bp, Escherichia coli
  misc_feature 1..26: note = E. coli Repeat 129
  source 1..26: mol_type = other DNA
cggtttatccccgctggccggggaac

SEQ ID NO: 640 - DNA, 29 bp, Escherichia coli
  misc_feature 1..29: note = E. coli Repeat 130
  source 1..29: mol_type = other DNA
cggtttatccccgctggcgcggggaactc

SEQ ID NO: 641 - DNA, 28 bp, Escherichia coli
  misc_feature 1..28: note = E. coli Repeat 131
  source 1..28: mol_type = other DNA
gttcactgccgtacaggcagcttagaaa

SEQ ID NO: 642 - DNA, 29 bp, Escherichia coli
  misc_feature 1..29: note = E. coli Repeat 132
  source 1..29: mol_type = other DNA
cggtttatccccgctggcgcggggaactc

SEQ ID NO: 643 - DNA, 29 bp, Escherichia coli
  misc_feature 1..29: note = E. coli Repeat 133
  source 1..29: mol_type = other DNA
cggtttatccccgctggcgcggggaacac

SEQ ID NO: 644 - DNA, 54 bp, Escherichia coli
  misc_feature 1..54: note = E. coli Repeat 134
  source 1..54: mol_type = other DNA
ctaacgtgcaggttttgtaggtcggataaggcgttcacgccgcatccgacacgg

SEQ ID NO: 645 - DNA, 29 bp, Escherichia coli
  misc_feature 1..29: note = E. coli Repeat 135
  source 1..29: mol_type = other DNA
gttcactgccgtacaggcagcttagaaat

SEQ ID NO: 646 - DNA, 29 bp, Escherichia coli
  misc_feature 1..29: note = E. coli Repeat 136
  source 1..29: mol_type = other DNA
cggtttatccccgctggcgcggggaacac

SEQ ID NO: 647 - DNA, 29 bp, Escherichia coli
  misc_feature 1..29: note = E. coli Repeat 137
  source 1..29: mol_type = other DNA
cggtttatccccgctggcgcggggaacac

SEQ ID NO: 648 - DNA, 29 bp, Escherichia coli
  misc_feature 1..29: note = E. coli Repeat 138
  source 1..29: mol_type = other DNA
cggtttatccccgctggcgcggggaacac

SEQ ID NO: 649 - DNA, 29 bp, Escherichia coli
  misc_feature 1..29: note = E. coli Repeat 139
  source 1..29: mol_type = other DNA
cggtttatccccgctggcgcggggaacac

SEQ ID NO: 650 - DNA, 43 bp, Escherichia coli; identical to SEQ ID NO: 546
  misc_feature 1..43: note = E. coli Repeat 140
  source 1..43: mol_type = other DNA

SEQ ID NO: 651 - DNA, 39 bp, Escherichia coli; identical to SEQ ID NO: 517
  misc_feature 1..39: note = E. coli Repeat 141
  source 1..39: mol_type = other DNA

SEQ ID NO: 652 - DNA, 29 bp, Escherichia coli
  misc_feature 1..29: note = E. coli Repeat 142
  source 1..29: mol_type = other DNA
cggtttatccccgctggcgcggggaactc

SEQ ID NO: 653 - DNA, 28 bp, Escherichia coli
  misc_feature 1..28: note = E. coli Repeat 143
  source 1..28: mol_type = other DNA
ggtttatccccgctggcgcggggaacac

SEQ ID NO: 654 - DNA, 43 bp, Escherichia coli; identical to SEQ ID NO: 546
  misc_feature 1..43: note = E. coli Repeat 144
  source 1..43: mol_type = other DNA

SEQ ID NO: 655 - DNA, 50 bp, Escherichia coli; identical to SEQ ID NO: 547
  misc_feature 1..50: note = E. coli Repeat 145
  source 1..50: mol_type = other DNA

SEQ ID NO: 656 - DNA, 45 bp, Escherichia coli; identical to SEQ ID NO: 548
  misc_feature 1..45: note = E. coli Repeat 146
  source 1..45: mol_type = other DNA

SEQ ID NO: 657 - DNA, 29 bp, Escherichia coli
  misc_feature 1..29: note = E. coli Repeat 147
  source 1..29: mol_type = other DNA
cggtttatccccgctggcgcggggaacac

SEQ ID NO: 658 - DNA, 29 bp, Escherichia coli
  misc_feature 1..29: note = E. coli Repeat 148
  source 1..29: mol_type = other DNA
cggtttatccccgctggcgcggggaacac

SEQ ID NO: 659 - DNA, 43 bp, Escherichia coli; identical to SEQ ID NO: 546
  misc_feature 1..43: note = E. coli Repeat 149
  source 1..43: mol_type = other DNA

SEQ ID NO: 660 - DNA, 50 bp, Escherichia coli; identical to SEQ ID NO: 547
  misc_feature 1..50: note = E. coli Repeat 150
  source 1..50: mol_type = other DNA

SEQ ID NO: 661 - DNA, 45 bp, Escherichia coli; identical to SEQ ID NO: 548
  misc_feature 1..45: note = E. coli Repeat 151
  source 1..45: mol_type = other DNA

SEQ ID NO: 662 - DNA, 29 bp, Escherichia coli
  misc_feature 1..29: note = E. coli Repeat 152
  source 1..29: mol_type = other DNA
cggtttatccccgctggcgcggggaacac

SEQ ID NO: 663 - DNA, 29 bp, Escherichia coli
  misc_feature 1..29: note = E. coli Repeat 153
  source 1..29: mol_type = other DNA
cggtttatccccgctggcgcggggaacac

SEQ ID NO: 664 - DNA, 28 bp, Escherichia coli LF82
  misc_feature 1..28: note = E. coli Repeat 154
  source 1..28: mol_type = other DNA
gttcactgccgtacaggcagcttagaaa

SEQ ID NO: 665 - DNA, 28 bp, Escherichia coli LF82
  misc_feature 1..28: note = E. coli Repeat 155
  source 1..28: mol_type = other DNA
gttcactgccgtacaggcagcttagaaa

SEQ ID NO: 666 - DNA, 33 bp, Escherichia coli LF82; identical to SEQ ID NO: 525
  misc_feature 1..33: note = E. coli Repeat 156
  source 1..33: mol_type = other DNA

SEQ ID NO: 667 - DNA, 44 bp, Escherichia coli LF82; identical to SEQ ID NO: 534
  misc_feature 1..44: note = E. coli Repeat 157
  source 1..44: mol_type = other DNA

SEQ ID NO: 668 - DNA, 30 bp, Escherichia coli LY180
  misc_feature 1..30: note = E. coli Repeat 158
  source 1..30: mol_type = other DNA
cgatgtaacaacgcgcacagatcagtcccc

SEQ ID NO: 669 - DNA, 29 bp, Escherichia coli LY180
  misc_feature 1..29: note = E. coli Repeat 159
  source 1..29: mol_type = other DNA
cggtttatccccgctggcgcggggaacac

SEQ ID NO: 670 - DNA, 29 bp, Escherichia coli LY180
  misc_feature 1..29: note = E. coli Repeat 160
  source 1..29: mol_type = other DNA
cggtttatccccgctggcgcggggaactc

SEQ ID NO: 671 - DNA, 29 bp, Escherichia coli O104:H4
  misc_feature 1..29: note = E. coli Repeat 161
  source 1..29: mol_type = other DNA
gagttccccgcgccagcggggataaaccg

SEQ ID NO: 672 - DNA, 29 bp, Escherichia coli O104:H4
  misc_feature 1..29: note = E. coli Repeat 162
  source 1..29: mol_type = other DNA
gtgttccccgcgccagcggggataaaccg

SEQ ID NO: 673 - DNA, 45 bp, Escherichia coli O104:H4
  misc_feature 1..45: note = E. coli Repeat 163
  source 1..45: mol_type = other DNA
ggataagacgcgccagcgtcgcatccgacattttgggcacagtag

SEQ ID NO: 674 - DNA, 29 bp, Escherichia coli O111:H str. 1128
  misc_feature 1..29: note = E. coli Repeat 164
  source 1..29: mol_type = other DNA
cggtttatccccgctggcgcggggaacac

SEQ ID NO: 675 - DNA, 29 bp, Escherichia coli O111:H str. 1128
  misc_feature 1..29: note = E. coli Repeat 165
  source 1..29: mol_type = other DNA
cggtttatccccgctggcgcggggaacac

SEQ ID NO: 676 - DNA, 24 bp, Escherichia coli O111:H str. 1128
  misc_feature 1..24: note = E. coli Repeat 166
  source 1..24: mol_type = other DNA
tgcgccagcatcgcatccggcatc

SEQ ID NO: 677 - DNA, 29 bp, Escherichia coli O157:H7
  misc_feature 1..29: note = E. coli Repeat 167
  source 1..29: mol_type = other DNA
cggtttatccccgctggcgcggggaacac

SEQ ID NO: 678 - DNA, 29 bp, Escherichia coli O157:H7
  misc_feature 1..29: note = E. coli Repeat 168
  source 1..29: mol_type = other DNA
cggtttatccccgctggcgcggggaactc

SEQ ID NO: 679 - DNA, 39 bp, Escherichia coli P12b
  misc_feature 1..39: note = E. coli Repeat 169
  source 1..39: mol_type = other DNA
gtaggcctgataagacgcgccagcgtcgcatcaggcgtt

SEQ ID NO: 680 - DNA, 41 bp, Escherichia coli P12b
  misc_feature 1..41: note = E. coli Repeat 170
  source 1..41: mol_type = other DNA
tgcctacaaacctgtgccggatcggtaggccggataaggcg

SEQ ID NO: 681 - DNA, 41 bp, Escherichia coli P12b
  misc_feature 1..41: note = E. coli Repeat 171
  source 1..41: mol_type = other DNA
tgcctgatgcgacgctggcgcgtcttatcaggcctacaaga

SEQ ID NO: 682 - DNA, 39 bp, Escherichia coli P12b; identical to SEQ ID NO: 517
  misc_feature 1..39: note = E. coli Repeat 172
  source 1..39: mol_type = other DNA

SEQ ID NO: 683 - DNA, 29 bp, Escherichia coli P12b
  misc_feature 1..29: note = E. coli Repeat 173
  source 1..29: mol_type = other DNA
cggtttatccccgctggcgcggggaacac

SEQ ID NO: 684 - DNA, 29 bp, Escherichia coli P12b
  misc_feature 1..29: note = E. coli Repeat 174
  source 1..29: mol_type = other DNA
cggtttatccccgctggcgcggggaacac

SEQ ID NO: 685 - DNA, 29 bp, Escherichia coli PCN033
  misc_feature 1..29: note = E. coli Repeat 175
  source 1..29: mol_type = other DNA
cggtttatccccgctcgcgcgggaaactc

SEQ ID NO: 686 - DNA, 28 bp, Escherichia coli PCN061
  misc_feature 1..28: note = E. coli Repeat 176
  source 1..28: mol_type = other DNA
gttcactgccgtacaggcagcttagaaa

SEQ ID NO: 687 - DNA, 39 bp, Escherichia coli PCN061; identical to SEQ ID NO: 517
  misc_feature 1..39: note = E. coli Repeat 177
  source 1..39: mol_type = other DNA

SEQ ID NO: 688 - DNA, 29 bp, Escherichia coli PCN061
  misc_feature 1..29: note = E. coli Repeat 178
  source 1..29: mol_type = other DNA
cggtttatccccgctggcgcggggaacac

SEQ ID NO: 689 - DNA, 30 bp, Escherichia coli PCN061
  misc_feature 1..30: note = E. coli Repeat 179
  source 1..30: mol_type = other DNA
ggtttatccccgctggcgcggggaacactc

SEQ ID NO: 690 - DNA, 29 bp, Escherichia coli SECEC SMS-3-5
  misc_feature 1..29: note = E. coli Repeat 180
  source 1..29: mol_type = other DNA
cggtttatccccgctggcgcagggaacac

SEQ ID NO: 691 - DNA, 43 bp, Escherichia coli K-12 substr. MC4100; identical to SEQ ID NO: 546
  misc_feature 1..43: note = E. coli Repeat 181
  source 1..43: mol_type = other DNA

SEQ ID NO: 692 - DNA, 39 bp, Escherichia coli K-12 substr. MC4100; identical to SEQ ID NO: 517
  misc_feature 1..39: note = E. coli Repeat 182
  source 1..39: mol_type = other DNA

SEQ ID NO: 693 - DNA, 41 bp, Escherichia coli K-12 substr. MC4100; identical to SEQ ID NO: 589
  misc_feature 1..41: note = E. coli Repeat 183
  source 1..41: mol_type = other DNA

SEQ ID NO: 694 - DNA, 28 bp, Escherichia coli K-12 substr. MC4100
  misc_feature 1..28: note = E. coli Repeat 184
  source 1..28: mol_type = other DNA
gtgttccccgcgccagcggggataaacc

SEQ ID NO: 695 - DNA, 29 bp, Escherichia coli K-12 substr. MC4100
  misc_feature 1..29: note = E. coli Repeat 185
  source 1..29: mol_type = other DNA
gagttccccgcgccagcggggataaaccg

SEQ ID NO: 696 - DNA, 28 bp, Escherichia coli UM146
  misc_feature 1..28: note = E. coli Repeat 186
  source 1..28: mol_type = other DNA
tttctaagctgcctgtacggcagtgaac

SEQ ID NO: 697 - DNA, 28 bp, Escherichia coli UM146
  misc_feature 1..28: note = E. coli Repeat 187
  source 1..28: mol_type = other DNA
tttctaagctgcctgtacggcagtgaac

SEQ ID NO: 698 - DNA, 37 bp, Escherichia coli UM146; identical to SEQ ID NO: 533
  misc_feature 1..37: note = E. coli Repeat 188
  source 1..37: mol_type = other DNA

SEQ ID NO: 699 - DNA, 44 bp, Escherichia coli UM146; identical to SEQ ID NO: 534
  misc_feature 1..44: note = E. coli Repeat 189
  source 1..44: mol_type = other DNA

SEQ ID NO: 700 - DNA, 41 bp, Escherichia coli UMN026
  misc_feature 1..41: note = E. coli Repeat 190
  source 1..41: mol_type = other DNA
tgcctgatgcgacgctggcgcgtcttatcatgcctacaaac

SEQ ID NO: 701 - DNA, 47 bp, Escherichia coli UMN026; identical to SEQ ID NO: 515
  misc_feature 1..47: note = E. coli Repeat 191
  source 1..47: mol_type = other DNA

SEQ ID NO: 702 - DNA, 28 bp, Escherichia coli UMN026
  misc_feature 1..28: note = E. coli Repeat 192
  source 1..28: mol_type = other DNA
gttcactgccgtacaggcagcttagaaa

SEQ ID NO: 703 - DNA, 39 bp, Escherichia coli UMN026; identical to SEQ ID NO: 517
  misc_feature 1..39: note = E. coli Repeat 193
  source 1..39: mol_type = other DNA

SEQ ID NO: 704 - DNA, 29 bp, Escherichia coli UMN026
  misc_feature 1..29: note = E. coli Repeat 194
  source 1..29: mol_type = other DNA
cggtttatccccgctggcgcggggaacac

SEQ ID NO: 705 - DNA, 29 bp, Escherichia coli UMN026
  misc_feature 1..29: note = E. coli Repeat 195
  source 1..29: mol_type = other DNA
cggtttatccccgctggcgcggggaactc

SEQ ID NO: 706 - DNA, 39 bp, Escherichia coli UMN026
  misc_feature 1..39: note = E. coli Repeat 196
  source 1..39: mol_type = other DNA
gtgctgtgtaggtcggataaggcgttcatgccgcatccg

SEQ ID NO: 707 - DNA, 54 bp, Escherichia coli UMN026; identical to SEQ ID NO: 644
  misc_feature 1..54: note = E. coli Repeat 197
  source 1..54: mol_type = other DNA

SEQ ID NO: 708 - DNA, 39 bp, Escherichia coli UMNF18; identical to SEQ ID NO: 517
  misc_feature 1..39: note = E. coli Repeat 198
  source 1..39: mol_type = other DNA

SEQ ID NO: 709 - DNA, 29 bp, Escherichia coli UMNF18
  misc_feature 1..29: note = E. coli Repeat 199
  source 1..29: mol_type = other DNA
cggtttatccccgctggcgcggggaacac

SEQ ID NO: 710 - DNA, 29 bp, Escherichia coli UMNF18
  misc_feature 1..29: note = E. coli Repeat 200
  source 1..29: mol_type = other DNA
cggtttatccccgctggcgcggggaacac

SEQ ID NO: 711 - DNA, 29 bp, Escherichia coli UMNF18
  misc_feature 1..29: note = E. coli Repeat 201
  source 1..29: mol_type = other DNA
cggtttatccccgctggcgcggggaacac

SEQ ID NO: 712 - DNA, 39 bp, Escherichia coli UMNK88; identical to SEQ ID NO: 517
  misc_feature 1..39: note = E. coli Repeat 202
  source 1..39: mol_type = other DNA

SEQ ID NO: 713 - DNA, 45 bp, Escherichia coli UMNK88; identical to SEQ ID NO: 548
  misc_feature 1..45: note = E. coli Repeat 203
  source 1..45: mol_type = other DNA

SEQ ID NO: 714 - DNA, 29 bp, Escherichia coli UMNK88
  misc_feature 1..29: note = E. coli Repeat 203
  source 1..29: mol_type = other DNA
cggtttatccccgctggcgcggggaactc

SEQ ID NO: 715 - DNA, 28 bp, Escherichia coli UMNK88
  misc_feature 1..28: note = E. coli Repeat 204
  source 1..28: mol_type = other DNA
ggtttatccccgctggcgcggggaacac

SEQ ID NO: 716 - DNA, 47 bp, Escherichia coli UTI89; identical to SEQ ID NO: 515
  misc_feature 1..47: note = E. coli Repeat 205
  source 1..47: mol_type = other DNA

SEQ ID NO: 717 - DNA, 28 bp, Escherichia coli UTI89
  misc_feature 1..28: note = E. coli Repeat 206
  source 1..28: mol_type = other DNA
gttcactgccgtacaggcagcttagaaa

SEQ ID NO: 718 - DNA, 28 bp, Escherichia coli UTI89
  misc_feature 1..28: note = E. coli Repeat 207
  source 1..28: mol_type = other DNA
gttcactgccgtacaggcagcttagaaa

SEQ ID NO: 719 - DNA, 37 bp, Escherichia coli UTI89; identical to SEQ ID NO: 533
  misc_feature 1..37: note = E. coli Repeat 208
  source 1..37: mol_type = other DNA

SEQ ID NO: 720 - DNA, 44 bp, Escherichia coli UTI89; identical to SEQ ID NO: 534
  misc_feature 1..44: note = E. coli Repeat 209
  source 1..44: mol_type = other DNA

SEQ ID NO: 721 - DNA, 39 bp, Escherichia coli VR50; identical to SEQ ID NO: 517
  misc_feature 1..39: note = E. coli Repeat 210
  source 1..39: mol_type = other DNA

SEQ ID NO: 722 - DNA, 29 bp, Escherichia coli VR50
  misc_feature 1..29: note = E. coli Repeat 211
  source 1..29: mol_type = other DNA
cggtttatccccgctggcgcggggaactc

SEQ ID NO: 723 - DNA, 28 bp, Escherichia coli VR50
  misc_feature 1..28: note = E. coli Repeat 212
  source 1..28: mol_type = other DNA
ggtttatccccgctggcgcggggaacac

SEQ ID NO: 724 - DNA, 30 bp, Escherichia coli W; identical to SEQ ID NO: 668
  misc_feature 1..30: note = E. coli Repeat 213
  source 1..30: mol_type = other DNA

SEQ ID NO: 725 - DNA, 29 bp, Escherichia coli W
  misc_feature 1..29: note = E. coli Repeat 214
  source 1..29: mol_type = other DNA
cggtttatccccgctggcgcggggaacac

SEQ ID NO: 726 - DNA, 29 bp, Escherichia coli W
  misc_feature 1..29: note = E. coli Repeat 215
  source 1..29: mol_type = other DNA
cggtttatccccgctggcgcggggaactc

SEQ ID NO: 727 - DNA, 30 bp, Escherichia coli W; identical to SEQ ID NO: 668
  misc_feature 1..30: note = E. coli Repeat 216
  source 1..30: mol_type = other DNA

SEQ ID NO: 728 - DNA, 29 bp, Escherichia coli W
  misc_feature 1..29: note = E. coli Repeat 217
  source 1..29: mol_type = other DNA
cggtttatccccgctggcgcggggaacac

SEQ ID NO: 729 - DNA, 29 bp, Escherichia coli W
  misc_feature 1..29: note = E. coli Repeat 218
  source 1..29: mol_type = other DNA
cggtttatccccgctggcgcggggaactc

SEQ ID NO: 730 - DNA, 29 bp, Escherichia coli Xuzhou21
  misc_feature 1..29: note = E. coli Repeat 219
  source 1..29: mol_type = other DNA
cggtttatccccgctggcgcggggaacac

SEQ ID NO: 731 - DNA, 28 bp, Escherichia coli Xuzhou21
  misc_feature 1..28: note = E. coli Repeat 220
  source 1..28: mol_type = other DNA
ggtttatccccactggcgcggggaactc

SEQ ID NO: 732 - skipped

SEQ ID NO: 733 - DNA, 37 bp, Clostridium difficile
  misc_feature 1..37: note = tcdA TA2
  source 1..37: mol_type = other DNA
acaccttaacccagccatagagtctgataataacttc

SEQ ID NO: 734 - DNA, 37 bp, Clostridium difficile
  misc_feature 1..37: note = tcdB TB2
  source 1..37: mol_type = other DNA
gacttatttgagtctatagagaaacctagttcagtaa

SEQ ID NO: 735 - DNA, 37 bp, Clostridium difficile
  misc_feature 1..37: note = rRNA-1 TRR1
  source 1..37: mol_type = other DNA
tcgacgacttcttccaaaaggttagataatcggcttc

SEQ ID NO: 736 - DNA, 37 bp, Clostridium difficile
  misc_feature 1..37: note = rRNA-2 TRR2
  source 1..37: mol_type = other DNA
gtacaggatggacccgcgtctgattagctagttggta

SEQ ID NO: 737 - DNA, 37 bp, Clostridium difficile
  misc_feature 1..37: note = gyrA TAR1
  source 1..37: mol_type = other DNA
tcctcatggagatactgctgtttattatgctatggta

SEQ ID NO: 738 - DNA, 2322 bp, Clostridium difficile
  misc_feature 1..2322: note = Cas sequence
  source 1..2322: mol_type = other DNA
tcaaataaattggtctatttcattacttataagcacacctttaccaaatatctgttttgtatgcttattttcgtatatatcatatttatataaaagtatttttaaatcttcaagacctttcacctgtatgtcaattacattttgtttagctttatatattggtaaatttacagtttttttaattatctctcttcttgctttttttctcttagactttattttatttatcaattgtctatcatcattactatatgcatttataagctcttgtcccaactcttcataatctttgattaaagtttcttcaattttattatatatatcctctggaattactgtatatccttcaatatttctaagtatattttgtgcatctttagaacctaaactatatggcgttatagtatctaaaatatttaaagcactggtaaatctcttttcaaaagctgtaccttctagactttctttagagtatagtatcttaaccatttctaccttatatttttctttcatcttcacacattcttttccatttataaaagttttcagtagctcaagtcctttttctacaatatccttatcataaatactacctattcctgtagctttttctgtatatataaatatatttgggctattttcttcatactcacgacttctataacatctaccaaatcgttgaaatagactgtcaagtgttgaattttctgtatgaagctcatcaaaatcaatatcaagggatgcttccactaattgtgtagtaatccaaataccattactatcactatctgcaaattcttttatatatttttctaattttgctctatcttcttgtatatacatagaatgtaaaagatttaagttgacatctattccttttggcttaactatttcttctattaactcatatttttctacagcacttttaactgtatttactattacaagaacttttttattcattccactttgtattattttacctaagttttcatctattgaattttctacaatagacacacaatgtcttattttttctgtattacatgtcaattcagctaagttactattcattacacctcttttttttaattcatctatatatatggttggcatagtagctgtcattatcataaatctgccacctatcttatgtatcatttctataccttttaccaatacagctgctatttctggtgaatatgcttgtatctcatctattactacttttgaatatgctaatgttgagtacactttttcataccctctatacaaaaaaggaaatttaaatatttggtctattgtagaaaatgtcagtttgcaagataataactttgctaaatctacaatctcacttgaattttcttgattactttcttctagataatctattgctgttgaatgtaacaaacctaagaatgtatcatttgattctccaactccaactatattttttgctctatcaaataatgcatttatacttactcttaatggaagtgtaaaaaatgccttgtctttatctatccaaattaaggcagtttctgtttttcccattcctgtaggtgcaatcagtattatattcttatttctattagatttagcaaatgattgagcctctctcaaactaccaaactctttcattaaataattttctgtctgttctcctatatttataacattattgcattccacaacttcatgagcagaagcactgtggtctaatctatgtagtattccttttaacataatatataaattatagtacttgtgatttttatctattcttttttctacactttgtagatatactttactcaatttttctgtttttattggatatctaactttaaattcatgctgtagttcataaactttatttattaaatcttcatctaatattttttgtattaaatttttaaaatctttatctataaagatatctctttcatgatgatatacaataacttgatttaatactgctctaagttctttattttttttcctgtctatataactataatcaataaatgcaggagaaagataattatggcctacattattttctaaatgagttactattttaggttcatttattttagtatccattctgctttttattaactcttgaaacggtgaaaatgcttttccaatatcatgaaattctataacaaagtcaagtaattgccaaaatatctcctcttctagaaaatctaagctatttatattttttccataactttctcttaatacattcatttgttttaaaagttcatcagtatgttctctaagtgtttccactggattagatttagcatataacat